European Patent Application EP 4 194 558 A1, published June 14, 2023. Title: HUMAN CYTOMEGALOVIRUS COMPRISING EXOGENOUS ANTIGENS. Applicant: UNIV OREGON HEALTH & SCIENCE. The sequence listing filed with the application follows.

SEQUENCE LISTING (7 sequences)

SEQ ID NO: 1 - DNA, 244443 bp, Human cytomegalovirus
  source 1..244443: mol_type = genomic DNA
ggtggtgttgcctgcggcggggacgggggttgcgctgggatcgggggtggcgccggggacggggggctttcgcagcggggaacacacaccgcctatttaacctccacccgctacaacacacacatgccgcacaatcatgccagccacagacacaaacagcacccacaccacgccgcttcacccagaggaccaacacacgttacccgtacaccacagtaacacacaaccgcaagtccaaacctcggacaaacgcgccgccgaagaccaccgcacgcagatggagctcgacgccgcggactacgctgcttgctcacaggcccgccaacacctctacggtcaaacacaaccccaactacacgcataccccaacgccaacccacaggaaagcgctcattttttcacagagaatcaacatcaagtcacgcatctacttcacaacattggcgagggcgcagcgctcggctaccccgtcccccgcgcggaaatccgccgtggcggtggcgactgggccgacagcgcaagcgacttcgacgccgactgctggtgcatgtggggacgcttcggaaccatgggccgccaacctgtcgtgaccttactgttggcgcgccaacgcgacggcctcgctgactggaacgtcgtacgctgccgcggcacaggctttcgcgcacacgattccgaggacggcgtctctgtctggcgtcagcacctggtttttttactcggaggccacggccgccgtgtacagttagaacgtccatccgcgggagaagcccaagctcgaggcctattgccacgcatccggatcacccccctctccacatctccacgcccaaaaccaccccagcccaccacatccaccgcctcgcacccacatgctacggctcggccagatcacacgctctttcctgtcccttccacaccctcaaccacggttcacaatccccgaaactacgccgtccaacttcacgccgaaacgacccgcacatggcgctgggcacgacgcggtgaacgtggcgcgtggatgccggccgagacatttacgtgtcccaaggataaacgtccctggtagacggggtagggggatctaccagcccagggctcgcgtatttcgccgccacgctgcttcaccgatatccaataaacccatcccctcgccacgacgtctccgcgtatctttgtagcctcaggaatccgtccccacgtccacccatcccgagcactccacacgctataacagaccacggacacggcaaatgcatgcaaacttctcatttattgtgtctactactctgtgttgctacagggggtgaaggcaaagaaaaaaaaaaggaacaaaataatagattagcagaaggaataatccgtgcgaccgagcttgtgcttcttttcttataaggaggcaaatatactagggaaaacataagaataggaagaaaccgaggtttgggagaaaagctgagataaaatagcgcattttccatacagaggttgttgtttttgtggatcctaagaggtttcaagtgcgaatcttaaagttctcacgagaatattgtcttcaagaatcgacaactgtggtccaagatttttttttggtctttttaggttctgcgagggacatcacgatggatcgttgcgatgaagtcacgcgtacgcctctggtgtggcgcggtgtcgtgacaggagagtgtgttttcagtgcagagctgtcttgattcctatatccgagtatctgttttctcgtaaggacggtaatcttctttggtgtaagtacatctaaaagctgcaaactatattttaagggctgtctctaggtgtactttgatgctggagtttttcgctgtgttgatgtgaataaatctactactactattatatgcagaaagagtgattatgccgagacaagattgcattggctgaactgtttcaaaaacgcctacactctacttatccgtaaacctaaggtaatactatgtgtaagttgttttttttttctttttgtagtaaaatggtgatacgtgcaattaaaactgtattccatgtttccatcctttcatttcaactttaaaggcggctttgagagcgaagaagtgcgaggataaaaatggatgactccttcgtgtccagggagtcgactactgcaacgctgattgattaaaagatggtctccgatgatgatgttgttattgatcgaatcatggtgcagaacggcgacggagaggagcgtgtccgccgccgggaaggtggtctctttctcttttcttttttcaagaaatcttccatgtgtttatcgtagtgatcgaaatcgactgatctcgggttctttttgttggtttcttttcggttaatcatgtattgttttctttttttacagaaagatacttttttcatgagcaattcctcgcccggcgccggcatgccgaggtggggccactgcgatcagcggcatgccgacgccgacccggggatcttggattcaccgttttctctcttctctctctacatacagaccgggtggcaggagcggtaaggaatcatcgtcgtctttcattcttcgatgattatggtaatactaaatcttatctaggagcatatacatctaagattggagtactagtagtcgtttgtggtttctatttttttttatatttatctatgacagtttttctgtttttcgttttgataataatataataaaaactcatggacgtgaaatctggcttggttgtggtgatttcattctcattattgttgttttctttccgtcttgcggatgaagatgttgcgatgcggttgttgttggtgttgctatacaccgagagagatgatctttttgttcttctggttcatttcctatgattgtttggctgctgaccgacgcgtcaggatgtgcagggcatgcggggaatcaggaccggacacgggataatttcatctacctatacggagatcgcggtcctcgccatgaggatcgcgacaggcgcgtcgagggggcaggaacacccttgcggattgacattcttggtggtgtttcgttgttgtcggtagttgttgttgacgatgaggataaataaaaatgaccttgtttttgttctgttttctcttgttgggaatcgtcgactttgaattcttcgagttatcggaaagctgaggtacccaaatgtctgtagcttttttctttttaccctcttgtttatcatctgcgattcgtggtaggtaggagagggaaatgataatccgagattaaggaaaggagaagataaaataaaaaaaaaataaaacagaagccgaccggccgccgacccgttccccaggaccagcctacgaggaacggataacgcggtggcgacggcagcggtggtggcgctgggggtggcggtagtggtactgctgatggtagtcgggacggaggagagacgatgcatacatacacgcgtgcatgctgcatgggtggatggtccgaccgggagacgcggaagagaaactcacataaaaaggtgacaaaaagagcggttgaaaaaagaaaacgagattcgaccagacagaagaggaggaccggggcttggcgacccttccacgactgctgttgtcatctcggctcctccgtcttctcccggccacgggcggctaagtcaccgccgttctccccatccgtccgagcgccgaccgaccagccggccgattcgcccgccggggcttctggagaacgccggggcagcagcgatctggagaagccgctaaacccctgcgtttttatatggtagctctgccgagcgcgggctgacgcgttaagtaagcggaaagacgtgtgtgacgaaaaggggtcccatggtatttcacgtgacgatgaggagatgcggtttggagcacatacggtttagaaaaagggagttgtcgtgacaagggctgagggacctctgtctccatgtgtgtataaaaagcaaggcacgttcataatgtaaaaaagaacacgttgtaaacaagctattgctgtatcattcggctgactatgcttcattcggactgattttcttttcctaacggcgtaacttaaagtgattaacgtatgatatttgttccccagagttatactatagtcatcatcctaaaattcagatataaatgaacacatgtcgtatgagattattaagaaaccgaaaccacccatagttcaccatcctcttcatcattcagccgatgacccactccgtacaacgactcagtctgcttcgtcatattgcaaagcacaagcgacgtatgtgaacaacttgaaacacagactgtgttattaatgaccgttgtaccattactagtcacattgcataaagatcctccgccgtcgtcccatcttttccactcggtggaaaaccggtcgctatcatcaactatggtgagattttcaccctgcgtggtattcagtttcttcatattcataccttggattccattattaaaccccaatattaagcacgttattagtaccccccccccccaccaaggaatgtgactggaccggttcctagcagctctgggagccatgttcaggttgaaccacagctacagcgaaaccgagtccagtgaccggtaaccacgtccagcccctgcgtatgtaccagtccaagcacgtccggtcattgttctacacaggaaatctaactaggtcaacgtaattttattccaccgttacgcagaatactaacaaaaaactacacaaatgtaacggattacacataatttattacgtgaaaactgtaagaaagccaattcaccaagcgatacatttatttgacttccaagtgccacacatcaccactatattcatccatgttttcaccgaaccaacgagacagatcgaagaagccagaatcttccgactttaaattacataaatccaacgtattatgaccacagctcgacacacaaatagttgcgttactattcacagtggcattacctatacccgtaacgttgcacaaccactgatcaccattgtcaccaaaaacggttttccacttagttgtcaacggatctttcctatgcgtaatggtaaaattactaccagtcgtcgcttttagctcattacgagtattatccgcatccacatatatcaacgtcatagctaggcacgctataagtaccccccccccacaatggaatgttgccaaaccggttctttcccgttatagccatagcgttcccaggcaaaagcaaacgccgaacctaatgcagtaaaaagcgcttgcagccagaaccagcttatgtaccagccacgataacatccggtcactgtttccacaggaaaccctaccagggtagagccccgcttgttttttcctgtctatcttgtttagcaactcgtaaactgtcagtctagccacgtccgtttagatcaaaagtcacgtatactgcgacgttgtttccacccgtttccccgtcccgccgtttccgaacaacccacccgggttcagacaaccgaccaccaacagaaatatacacacagaccaccgggagttcagttaaagatttcatcaggtttattttggctgctgctagtcttttgcttcttagaaaaaaaatacccatatagagaaataatgatagtttgacaacacatatggcagggatttcttcttcatcaataagatatgcaattcccccagggagagactttcaacaattgaatttacaaaaacaaaattacatcaggagaaagagaggatacattaataaatatattatatctggtgtatatactgaatgctgctggttcataaggtaacgatgctactttttttaattccaagatggtttttctttgttagtcttttgttgacttgctggttcctaaaagttctcaaaaacgattgtgtgaagattttatgacgttggttgactagttcatgagattctgctgtacgtgtgatggttattcgctggttcgttctaagatgagtatcgtactgtgtctgcgatggtcgtctcttactggcattctctcggctgcctcttgctttcatgattgaaaaggaaaaaaggactccgagggcgcggtcatcttttacttttcggttttttcgttggcgggtcagaggtagtcagatcatgagactgtcgtggtcgatgaaactgtgtctgctcaagtgacgtccatttcttgtacggagaaaaaagtcatcgggataaataaggctatacaaggcgttgtcaagcgtgcggctctaaacaaattaagcgatacaaaattacagtaatacgaataataagttaccccctccccctgtggtccccccgagacgagagccacccatcgtgtactctcgcaccacccacgaccacagagggagacgggacgaagagacgacgcagagcgccatctccttctggaggccggcggcgttaactgctacagctgcggcggcgacaacagctgcgatttgtcggccgacatgccgatggtatgggcggcggcggcagtggccgcggcagcggggaggagaggagagagaagaggagcggggcgtccgaaggcgaggatggcatggtctcgccggagcgcccggcttttatggaacgctcgcgtccggtcgggcagcgcccacaggaagatgagtcaaaacttttaaaccatcctgagacccgagtagcggtttacaggccgcacgccagtcttagctaaaaacagcggacagtcccacgctgtttctgttgtggctctctccagtttcctcatcgccgtcccgatctccgtcgtcatcggaagaataccacccgctctcatgcggcagtcgatcgacctcgacgaacgagacgcggcgacgcctctctacggccgactggttgtggtggtgaaagaagagcaccagcaatcccaggaggagcaacaagccctcacatgtccaggaggtcggggagagggcctgtcggagatggccgtgaggcatcacgtacggcagctgaggagaaacggagaagaaaggaaaattaccgtcaggggccggggttcttattagagaaacagcacgtaggtcaggatccagatgctaatggcaatcatgatgacgatgatcatgcaggccaagacgcggcgcaccaatgccgaatccaatagccgccgtgcctccggttggtggccggcggcatctagagacatgatttgggggggaccggcggcgcgaaaagacagggagatggacagtgtcacggtgttttgttatgattaggacatggggaccggaagccgagacagagtactacagggtgttgaagggtaacgtgagggagatcatgtcatgggcgggctgaagaccgtgcggggaggattggcgtgtgcggtgcttgtggaacacggtgttttaatatgtatccgcgtgtaatgcacgcggtgtgctttttagcactcggcttgataagctacgtggccgtttgcgccgaaaacacggttaccaccaactgtctcgtgaaaacagaaaatacccacctaacatgtaagtgcaatccgaatagcacatctaccaatggcagcaagtgccacgcgatgtgcaaatgccgggtcacagaacccattaccatgctaggcgcatactcggcctggggcgcgggctcgttcgtggccacgctgatagtcctgctggtggtcttcttcgtaatttacgcgcgcgaggaggagaaaaacaacacgggcaccgaggtagatcaatgtctggcctatcggagcctgacacgcaaaaagctggaacaacacgcggctaaaaagcagaacatctacgaacggattccataccggccctccagacagaacgacaactccccgttgatcgaaccgacgggcacagacgacgaagaggacgaggacgacgacgtctgataaggaaggcgagaacgtgttttgcaccatgcagacctacagcacccccctcacgcttgtcatagtcacgtcgctgtttttgttcacaactcagggaaatttatcgaacgccgtcgaaccaaccaaaaaacccctaaagctcgccaactaccgtgccacctgcgaggaccgtacacgcacgctggttaccaggcttaacactagtcatcacagcgtagtctggcaacgttatgatatctacagcagatacatgcgtcgtatgccgccactttgcatcattacagacgcctataaagaaaccacgcatcagggtggcgcaactttcacgtgcacgcgccaaaatctcacgctgtacaatcttacgattaaagatacgggagtctatcttctacaggatcagtgtaccggcgatgtcgaggctttctacctcatcatccacccacgtagcttctgccgagctttggaaacgcgtcgatgcttttatccgggaccagggagagttgtggttacggattcccaagaggcagaccgagcaattatctcggatttaaaacgccagtggtccggcctctcactccattgcgcctgggtttcgggactgatgatctttgttggcgcactggtcatctgcttcctgcgatcacaacgaatcggggaacaggacgctgaacagctgcggacggacctggatacggaacctttgttgttgacggtggacggagatttggaataaaagatgcgcgtcaaccgtcaaagacgcaacaaccttacgtaccgacaaacggtatatgtaattctgaccttctacattgtacataggggcatatgtaacagcaccgataccaacaattctacatctacttcaaatagcaccgtctctgatactaatgtatattctactccaaatcctcccagtgtatcttctacaactcttgatacatctaccgactcacagatatcaatcgcctcaaacaccatatccagcactacaaatacattgaccgcatattctataactacgttaaacacctcgacttcatcttcaactcttactgctgtctctagtacccatacaagatcctcaatactctccaacaacgcatcatacaccacatcattggataatacaactacagacataacgtccagcgaaagttcaatcaacgtgtcgacagtttacaacaccacgtacattcctgtaacatcgcttgctattaattgtactgctacaattaacggaacaaataattctagttcaaaaacttgccaacaagacattgaaacaatacctgtgaaatcaactccactaacggcagaagaaggaacaaatattacaatacatggcaatgacacgtgggattgtcccgacgtggtttggtatcgacattataattggtctacacatggacaccacatttatcccaatacacattacaaaactttgatacatcgacgcaagatcctaacgtcacatcctatatgttattctgatcgctcatcacctaccgcgtatcatgatctatgccgttcatgtaataaaacagaactacgcctttacgatttaaacaccaccaattctggtagatatagccgacggtgttacaaacagtaccatcaccagggaccacacgaggatgaaaatttcggactaactgtaaatcccaggaacaacactgacaattataccatcccagtatgtcccagatacgtagaaacacaatcacaggaagatgaacaagacgacgattatacactaagcactaccataaataataatcttatgcgcaaaacaggtcactatgacatctcacatggcacgcacactacatgggctcttatactaatttgcatagcctgcatgcttcttttttttgttcgacgagccctcaataaaaaatatcgtccactacgagatgatattagtgaatctagccttgttgtgcaatatcatcctgaacatgaagactaacgtttccggacatgcaacacataaaattaagtaacatatctaccatgaagtacagcaaatatctactaatgtctatccatccaacagtgataccatgcactggcatcttgcgattacatggacggtaatcatatccacgttttcggaatgttgtaaccaaacttgtccgtgttcctgcgtttgtgtcaattctacaacagtcaacatatccacaaatgaaacaacgtctaaagccatcactccaactgctacgacaaataccgcaaaaacaacgtcaagccttgttattactacaccgtcatcagtaacgattagcaaagccgtgtctactgcagcttcatcaaccatactatctcaaaccaatcgcagtcatacaagtaatgtcatcacaaccccaaaaacgcggtttgaatataatatcacgggatatgttggccaagaagtgactttcaacttcagtggatcattttggagctacattgaatggttccggtacagttctccaggctggctttattcctcggaaccaatatgcaccgttaccaacagttatcatcatactttccctcgtggtaccttatgtttcgattgtaacatgacaaaatttgttatttacgatctaacgttaaacgattctggaaagtacgttgtcaagagaacacgtcatgacaatcaatacgaagaagcatgctacaatctcacggtaatttatgccaacacgacagccatagttaccaacaggacgtgtgatagaagacaaacaaaaaatacagacactactaaccatggaatcgggaaacatattattgaaactattaaaaaagccaacattcccctggggattcatgctgtgtgggcgggcatagtggtatcagtggcactcatagcactatatatgggtaaccgtcgtaggcccaggaaaccgcgttataccagacttcctaaatacgacccggatgagttttggactaaaacctgatatgcacatcaataaacttttttgtatctttagttattaatgtctgtgtgtttattcagaataactcatttataatataagacggaatattcatatacattaaaaacatgggtgtacaatataacactaaactgttattagccgtattagcaattatcccagctggcattctagtacaggcaatttcacatgagcaaaaaacatcctaccggcaacttttgctgcaaagtgaacgtgtgcaaatacccatcacaacagtcgagggagatacaatttgctttaacgttagtaacaacccctgcaacttttccagttattggaatcacaataattgtgaactttgcggttggacaccgtttttctttgaatatgctggatatactgaaaacacgtcgtgtcacccacgatttacctgtattcatgatactaaaggtctaaaactatacaatgtaaccatgaatgactcgggaatttatacacaacacgtttatcactgtgatattccatgtaacatcagcgatgatcgtaaatataacgtagatgacattgataactgcaacgctactataaatgtaaccgactatattattaccgtgttgtcttcacgttattctaaacgcaccgattaccacgtagatacttacattggttatgcaaccactgtggtgacaatagtatttatctgtgttttaacttgcattaacgtctcagcaactctaaggcacagactacgaactagaaacaacgttaacagcataacgtgattacaaagtatcaacgctagtttatccaagagaaactttcatgaaggatcgcaataaagcattgctatgtatcatctttattttaatcatgtacctcatttatatttattttaaacgtcgttgtattcctactccgtccccagacaaagcggatctgcgagtggaatttccctcattacccccgtgtgtcggcatacagtgcgctgcataagaacacgcatgacacatagcgtacctctggacggtacagtatatgataacatgattcaaggaaagtatggattcctaccgacatgttatgacagaacacacaggttttctgcgtgttttataaaagagcgtctcgaagcagcttgagccacactacggtccagataacgagcgttgcaaaaaatatgccgcgcagtagtcgaaagccgtactgagcgtgcgaagcgggtagggtgccgaacgacggatatgcgccgttgtcatcttcgactataaggatcgcgaccgagtcttcgggcatggtaaaagccacacggtgtggttgatatgtagcgtatccggtttggaatcgttcggctccggctcaggggatagtgaggaattctcaggggacgatatgggacccaatgactggataaaagaagggtttttcccagtaagatgatccccgtatcacatgaggtctggatatatataaatgaggagtgaaataggcaaagggtatcagacaccagcctcgtcatgcagccgttggttctctcagcggaggaactatcgtctctgctaatttgcaaatacatcccaccttaagcgacgagtccataaagcaccgttgtccgggtacggtgaaagtgacccggattgtagcacgtcccttttttgtttttgcatcgtttatcgtcaccactagtgcaatattttgatcgtaaggctgaaagagtattgttatgatgcttagaacgtggagattattacagatggtactgcttgccacgtactgttattatgtttttgcgaattgttcaatcagcacgacgactgctcctgtggaatggaagtctcccaaccgtcagattcccaagaatattacctgcgctaattactcagggaccgtcggcggtaacgttacttttcagggtctcaagaataaaacggaagactttttatcttggctactcgggtctggctataagtccatttgctcgttcttcccacaactccctggtgattctaatgagcagcattacagatatgaagtaaccaacctcacgtacaattgtacctatgaccgcctaacgttactgaatctgacaatggaaaacagcaggaattactatttcagaagagaagatgcgaattccaccttctactactcttgttacaatctgaccgtgtcctagagaacgcacgtgaagttccacagagccgcgtggctgtagctattgtttacgttgcttttgaaatgttaagcgtccctacggcgctaacatgtttctaggctactctgactgtgtagatcccggctttgctgtatatcgtgtatctagatcacgcttgaagctcgtgttgtcttttgtgtggttggtcggtttgcgtctccatgattgtgccacgttcgaatcctgctgttacgacatcaccgaggcggagagtaacaaggctatatcaagggacgaagcagtattcacctccagcgtgagcacccgcacaccgtccctggcgatcgcgccgcctcctgaccgatcgatgctgttatcacgggaggaagaactcgttccgtggagtcgtctcatcatcactaagcagttctacggaggcctgattttccacaccacctgggttaccggcttcgttttgctaggactcttgacgcttttcgccagcctgtttcgtgtgccgcaatccatctgtcgtttctgcatagaccgtctccgggacatcgcccgtcctttgaaataccgctatcaacgtctcgtcgccaccgtgtagctagttagccagctgtgtatagtttgttgtgttttgcttttgcgtatttgttttcagtcagagagtctgaaacggggtgggagggacttttgcgggtaatgcatgctaaaataaacgggtgggctggggtgtgcttggtaactcactgtttgaatacgcgctcacgcacatatgtagcactcaacatgttagcttttgcccgcacgccccggggcgtgccgagctgcctttttaataaagtctgggtttccagatacgcgctggttctgattttgatgatttgtgcctctgaaagctctacgagctgggccgtgacatccaatcgactgcctaactgtagcacggtaactacaacagcgggtcaagacgctgaattgcacggtccggcaccgttaagctgtaatgtgacccagtggggacgttacgagaatgaaagcacacccgtattatggtgcactttatggggatcacgcatgcgagtctcattaggacaccgtgtagcgtttggctgttcttggaaaacattttttatttataacgtttctgaaagtagcggtggcacttactatcaaaaaggttacaactgcaccgacaaacatataacactatcttgtttcaacctaacggtggttcctcgagcggttcaaagcacaaccaccgtaatgacacccacggtggttacaaactccacattcagtgtgtcacttattgcgttgagactgacgacaaattccagcgcggttggacacgctagttatcaacgacaacagcgtgttgaaaacgggacgttatccaagaacataactaacttggcattcacctatggcagctggggcgttgcgatgctgctgtttgccgccgtgatggtgctcgttgatttgggtttgcctcaatcggcttggcgacgctggcaaagccacgtggacgatgaagaacgtggtttgttaatataggaagtaaaaggcactgttttagcatgactgtttccaaaccgtaacgtggtaaataaatcatggcttccgacgtgggttctcatcctctgacagttacacgattccgctgcagagtgcatcatgtgtacaataaactgttgattttagctttgtttgcccccgtgattctggaatccgtcatctacgtgtccgggccacagggagggaacgttaccctgatatccaacttcacttcaaacatcagcgtacggtggtttcgctgggacggcaacgatagccatctcatttgcttttacaaacgtggagagggtctttctacgccctatgtgggtttaagcttaagttgtgcggctaaccagatcaccatcttcaacctcacgttaaacgactccggtcgttacggagcagaaggttttacgagaagcggcgaaaatgaaacgtttctgtggtataatttgaccgtgaaacccaaacctttggaaactactccagctagtaacgtaacaaccatcgtcacgacgacatcgacggtgaccggcgcgaaaagtaacgttacggggaacgccagtttagcaccacaactacgtgccgtcgctggattctccaatcagacgcctttggaaaacaacacgcacatggccttggtaggtgttgtcgtgtttctagccctaatagttgtttgtattatggggtggtggaagttgttgtgtagtaaaccagagttatagtaatgtgttttttatcagggagaaggttttgtaccaacaatgactacatcggggctatctgtgtcggaaaattatgacggaaattatggactcacggaaaccgccaatacaacgcgtacaaatagcagtgactgggtaacgttaggaaccagtacgccactgttgggaagcacggagactgcgatcaatttcggcaacgcaactacggttattccacaacctgtggaacacccggctggagaagtacagtaccaaagaacgacaacgcattactcttggatgctgattatcgttatcattttcatcatttttattatcatctgtctacgagcacctcgaaaagtttatgatcgttggaaagacagcagagagtacggacaagtgtttatgacggatacagaactgtaatatactatgatgtctaagaagtgtttgcggttatttccatggatgacaattttgttttgcataccaaaagcacaacattggaactatatgacaataccatgcgttcttaaaattggacgcggcggtcaaaatatgagtttgcctccccttaacaattcattgtacggaaacgatatttttcaatggtatacagacagaccgacagtcaccaacacgttatgtctttatcaaaacaatgagtactacacacaatccaatgaagatatttcaaacatcaaatggcaatgtacaaaaaaccatacgttaattcttattaacctaaccgcaacatatagtaggaactattactttcaatctcttaaaactcttgggcaaggaataccgagaccgagcagcttatgttataatgttagtgtacaccttacccaccaaacacattgtcatacaaccacattatccctgtatccacctacacctgtacacaattcattaacaatatcaccgtcattagcttcaaccaactttacacatgttgcggtccatcatgccgcaggtaacgttgaagcacaacacaacactgccactccacatacaacgtggatcatacccctggttatcattataacaatcatcattttaatttgtttcaaatttccccagaaagcttggaataaattcacacaataccgatacaacagtatgctcgccgccgcttaaagaatcaccgtcgaggaaactaaaagctatgtacgtttatttttcagctcactgtttgaataccgtaaacataatgacgtacatatacgtggttatacaacaggtgtttgtgttatgcggcgactgattaaccatatcgtgaaccatgatcttttccgatggtctgtcgtgaccgcaatgatattttacaagtattccgaaacctgtatggaggtcactgtcagagtaggtgatccagttaccctcggtagtggacatggttatcatccaggacaaaaagtacactggtataaccagtcatgcgtcggcatcagcaacggcgaaaatacgcatcctatctgcacctacgaccctcctaaacctggtagacaaaagacaatgaaaaccactccgttgccatcaccactgttgtatgaatgtcacaattccacattaagcattcttcatgtaaacgtctcagatcccagaaactattgcaggcgaaaatgtccaccaaagggtaactgtgagtttcccacatgttttacattatcgctgatttctagaacgacaaccaccagaagacccggacaaaaaactacgctgtcgcgattaaaaactacgccaaataaacatacgcagcacaaaagatccacgcgaagaacgtcacttaaagattacaatgtaacgggtctgccgaaaggctttgcggactcgtttaccggtaacgtagaggcacatagagccaaagatgccgcacacagcgcatggattctcattgtcatcatcattatcatagtcgtcattctgtttttcttcaagattcctcaaagactccgagagaaatgggacaccaagggatacctttacaaagggaccgatggcctgcccactacggactaattatcgtgagcggacggatatgtccggtttcaaactcactgtttgaatatagggacagtccctacggaacctgagaacatgtggaaatcacctgtggtagaatgctgctcaggtacattacctttcatcgcgaaaaggtactttacctaacggctgcatgcatctttggtgtctacatcagcctccatgatgcctgcataccggtggttggcaagataggtaccaacgttacgttgaacgcggtagatgttctttcccctcgcgatcaagttcgttggtcatacggtccaggcgggcaaggctacatgttatgcattttcactggcacatcaacaacaacgtttaacagcacgcgctttaatttttcatgtctgagtaattacagcctcctcctcattaacgttaccgcgcagtatagtactacctatcgtactatgacatcgctagacgattggcgtcaccaaaaacataaccatggttttcgatggactttagacacatgttacaatctgacagtgaacgaaaacggtacattccccactaccaccaccaaaaagcccactacgactacgagaacgacaactaccacaacacaaaaaacaaccaccacgagaacaaccaccaccgccaagaagacgacgataagcactacccatcataaacactccagtcccaaaaaatccaccacccctaacagtcacgtagaacatcacgttggttttgaagccacagcagcggaaacaccgttacaaccaagcccacagcaccaacacgtggctacacacgccctctgggttttagcggtcgtaatcgttattatcatcattatcattttctactttcgaataccgcaaaagctgtggctgctctggcagcatgacaagcacggcatcgtgctcatcccccaaaccgatctgtgagcaagtcgcgtaggaaacgattgcatgaaatcactgtgaaacgccaactccgtgccaactggcacggcggacaggcctttgacgtatttgaagccaggcgcgctcttgataccgaaaggatccgagggggctttccaaagccgacgtccctgattcccttcataaagctgttgaccggccctagaaagaccaagagcatgctgtgggcccactgcggtcgcttcttgcgttatcatctgctcccgctgctgctgtgtagactgccattcttactcctttttcagcggccgcagtgggcccacggcttggacattgtcgaggaggacgagtggctacgggagatacaaggagcgacgtaccagctgtccatagtgcgccaagctatgcagcacgccggattccaagtcagagcggcgtcggtcatgacacggcgaaacgccgttgacctggaccgaccgccgctttggtcgggatcgctcccgcatttgcccgtctacgatgtgcgttccccgcggccgttgagaccgccgtcatcacagcatcacgccgtatcacccgaactgccgtcgcgaaacgggatacgttggcagtaccaagagttgcagtatatggtggaagaacaacggcggcgaaatcagtcgcgtaatgcgattccgagaccctcgttcccccccccggatccaccatcgcagccggcagaggatgcacgagacgcggacgcagaacgtgccgaatcaccacatagtgcagaaagcaccgtcaggcacgacgcgagtgagaacgcagtgcggcaacggcgcgaaagacggcgctataacgctctgacggtccgcagccgggactcgctgctcctgacgcgaatacgcttctccaaccaacggtgtttcggacgcgggcgtttgagacatcccgcgggaagtggtcccaacaccggcggaccgcgacccggcggtgcgggactccgtcaactacgccaacaactgacggtccgctggcagctgttccgcctacggtgccacggttggacacagcaagtctctagccagatcagaacccgctgggaggaaagcaacgtcgtgagccagacggccacgcgagtacgtacgtggtttgtggaaagaaccacgttttggcgtcgcacgtggattccgggacagaacccggcggccgaagcgcaagaactggccgtcataccgctggcacccacggtgctccagcagaacgaggaaccacgtcaacagcttacgggagaggagacaagaaattcaacgcacactcaacgtgaagaagtggaggacgtttcgagagaggacgcgagagaagggaatgatgggagccgagcaagtggaaacgacgagagaaggaataatgcgggaagatatgatgatcacgaggttcaagagccgcaggtcacttatccagcgggacaaggagaactgaacaggaggtcacaggaggagaacgaggaaggtggaccgtgtgaatcgccgccaatgacgacaaatacgctgaccgtggcctgtccgccccgcgaacccccgcatcgtgccctgtttcgtctatgcttaggactgtgggtctcgagctacctggttcgacggcccatgacgatttagaatacaccgagccattcctttatttcccccccccccatccccggtcgcttatgcgtgtcaaacactaccaataaagataatctgccaatagcaccttatatataatatgtggtcgcgtgtggtctttttaaggagccctgaaacacagacaggtatgggcggtggccggctgccgccgctgtggctgccgctactgatcgcctggagcgagtggggcaactgctgcctcgatgcgcctccggtggtgcgttcgccctgtctgcagccggtgcgcgaccgcaaccgcgagcggaacccgggctcaccgcagttgctgccttacggcgaccgtctggaggtggcctgcatcttccccgcgcacgactggccagaggtctctatccgagtccacctctgctactggcccgagatcgtgcgttcgctggtggtggacgcacgcagcggtcaggtgttacacaacgacgccagctgttacatcgccggcgggcgctggcgttttgaggacggcggcgcggcgcagcggctgagcctctcgtttcgtctcatcaccgagaccgcgggcacctacacctgcgtgctgggcaacgagacccacagcctggcgaccgagaccacggcgctggtggccgacgtgcacgacctgcgccactcggaccgctcctgcgacctggctttcggatcgcgctcacagacgcggtacctgtggacgcccgatccctccaggttgcgcagtataaactgcggttgggagggtgaacggcaccgcgtagtccactacatccccggcacctcgggtctgctgccctcgtgcgaggaggacgagcgcgaactgtgcgtgcccttcatcagccatagcatcgccgacaacaactgcagccgccggcatcgagtagacggcgctaggcggcgctatcatctgcggagggattactggctgacggatccgaagatcgggctgctggccgcgggatcggtggccctgacctccctctgccacctgctgtgctactggtgttccgaatcgtaccggcgcctgaacaccgaagaggaaaacgaggcggcggaggaaactgccgcgggagaagcctctgcggtagcggcggcggccgtctctgaggaagagcagcagcgggagtaaacggggagagccatgaagcggatgattcgcagtcacggcaggaaaacggaatgtcagatgacgggcgccggcgagcgacgcggctccgccgtcggtgcgctcatctgcgacagcggtacccgacgcggcagcggcgccaacgaacgccgcgactccgacgtcggtcccatcgcccacagtagcggtaccagacgcggttcggcaaatgaaacgtccgcctgtacgcggaccgatcaccagaaggcggacattgggctgtggttcatgtttctgttttttggactgtgttcgtggttagcgatgcggtatcgcgcacaataaattttgaatccatatcaaggaacgcgtgttttgtattttattgggaatattggcggggataaaccggtttcggatgtttacccttaatcttaccggggacctcgttgtcctctcccccttcttcctcggacaccgggcttcatgctgacgtaggtaccgactggggtcaaaagcctgggtacttatggggagcgcgcacaaaggaccgtcaggcgccggcatggagcgtcgccgaggtacggtaccgctgggatgggtgttttttattctttgcttatctgcctcttccccgtgtgctgttgacctgggtagcaagtcctcaaactctacctgccgcttgaatgtgacggagttggcctcgatccgtcctggggaaacgtggacgttacacggaatgtgtatctctatctgctactacgagaatgtgaccgaggacgagatcatcggcgtggcttttacttggcagcataacgagtctgtggttgacctgtggttgtaccagaacgatacggtgatccgcaatttcagcgacatcaccaccaacatcttgcaagacggactgaaaatgcgaaccgtccctgtgactaaactgtacaccagccgcatggtcactaatcttaccgtgggccgttatgactgtttacgctgcgagaacggtacgatgaaaataatcgagcgcctccacgtccgattgggctcgctatatccgagaccgcccggatccgggctcgccaaacacccctccgtaagagccgacgaggaactgtccgcgaccttggcgagagacatcgtgttggtctcggccatcactctgttcttcttcttgctggccctacggatcccccagcgactgtgtcagcggctgcgcattcgcctgccgcatcgataccagcggttacgcaccgaggactgaacggataaccgcaaaggccacgtgcaacgttcacgctgctataagaaggccatgtcccccgtggacgggtctctttgacacgagcgcggcacgccgttgccacgagcatggatcacgcgctcctcacacacttcgtcggccggccccgtcactgtcggttggaaatgttgattctggacgaacaggtgtctaagagatcctgggacaccacggtttaccacaggcgccgcaaacatctacctcgacgtcgcgctccgtgcggcccccagaggcccgccgagattcccaaaagaagaaaaaaggcggccgtccttctgttttggcacgatttgtgctggctgtttcgacgacttttctttcctcgggaggactcggagccactgatgtcggatccggcacggtctcccgaagaggaggagtaaacaacacacggctaagaggatacatcatcaaagaagataggaggggtcaaaacgcggactgaaagtatataacgccgatcatgtccgaggaactgttaataaaacgccatgatgacaatgtggtgtctgacgttgtttgtgctgtggatgttgagagtggtgggaatgcacgtgttgcgttacgggtacacggggattttcgatgatacatcgcatatgacgttgaccgttgtggggatttttgacgggcaacacttttttacctatcacgttaattccagcgataaagcgtcaagtcgggccaacggtaccatttcttggatggctaacgtctcggcggcctaccccacctacctggacggggaaagagccaaaggtgaccttatttttaaccaaaccgagcaaaacctgttagagctggaaattgcgttgggttaccggtcacagagcgtgctgacgtggacgcacgagtgtaataccacggaaaacggtagttttgtagccggttacgagggatttgggtgggacggggaaactttaatggagctcaaggataacctgacactatggacgggccccaattacgaaattagttggttgaagcaaaacaaaacgtacatcgacggtaaaattaaaaacatcagcgagggggatactacaatacaaaggaactatctcaagggtaattgcactcaatggtccgtcatttatagcgggtttcaaacccccgtcacccacccagtggtaaagggcggtgtccgaaaccagaatgacaacagagctgaagcattctgtacatcttacgggttctttccaggggaaattaatattacttttatccattacggtaataaggcgcccgatgatagcgagcctcaatgcaatccgctacttcccaccttcgatgggactttccatcagggatgttacgtagccatcttttgcaatcaaaactacacctgccgcgttacacacggtaattggacggtggaaatccccatcagcgttacctcacctgacgacagttcctcgggggaggtccctgatcacccgacagctaacaaacgctataacaccatgaccatcagcagtgtcctcctagccctgcttttatgcgctttgctattcgcgttcctgcactactttaccaccttgaaacaatacctacgtaacctggcctttgcgtggcgctatcgcaaggtccggtcgtcatgaccagcaacgccctgtatgagctgtttcgacgtcggttaccgcgtgcccccgtcaacacggtcatgtttctcacgcgacgcactcgtgatgggttctgcggtcggttgacgtccatcgccacgaattcccactacactatgttcgtgttagatcacggatccgtgcgcatcgagcgaccgagtcagtcagaagtggattgcgccagtttaatggaaacgctgaagcggattcggttacgaaattcgtgggtagcgtcagaagacgagctagatgtgagtcgcagggacgcgtgacacgaaacgcgttcaggattaacgtaggttttcgaaataacctacgtccgtgagtgacgcggtttcgtgttgaaacccgcgcccgcttctcacggtggtttatgatgaaaccggcgttgcggatccacgcgggttcctcattcaacctgcgaaaagaggaagttgcggtaaaaccacgtcaataaagacgtcaatgacacctcaatgttgcgttggaacggtctttatatatacaaacgccgttatgatcagtgtccggcaagatgctcgggatacgggctatgctggtgatgctggattactactggatacagttgataacgaacaatggcactcgaagcaacaataccgataccatctttgtatctctccttaccgggcccaacggagttactcgcacagccatcggaggtctgtattcaaactacaccaacttaactggagcatttggcttcacttcaacaaatatgtcagcaaccaactcttccgctgaggataattggagcgtaaccaacctgacggagagttgcatcaaccgcggtgagtcctatgtgactaccatctggcttctggactgcactaaaaacgatacttattggtactatggaaatgcctacaatcatacatgtgaaggtacaatttcgggatatctcctgggcatgtgcaagctatggaaaagttgggtcaataatattacttcttataacactgtcagagtcgaatcgctgggaaatgaaacacggtgcatgctgctccctagacagtatactctcaacgccacggtggaatggtacaacaaatctgaaggtgacgtaccagaagaattcatggactatgttatcctgacccccttggctgtgcttacatgcggactgcaggaagcttatatactcgacaaaggtcgtagatacatgtatttgttttccgtgtcctgcgtgggaatcacaggtaccgtatctattatactcgtctccctatcgctgctcatcctcatctgttactatcgctgtggccggcttctgatatgcccacgcggctttgaactcttgccagaattcactgaggaagaggaggaaaaagaaaaattgttaacgcataatgacattgaagtccaagtgcctattcgcacgcggcgactactcgtcccttggatccgggagagcaaaatgtgggtactaccacccccgttgcctccacgacctccccacttaatagaattcccgccgtctcctccgtcatcgcctgggcccatgcacatggtggtctgcatgccagcatgacgaactttggactctgagccccaagcggtacgaactacatattttccataaatctacactgaacttgagcacaaagatactgacaatagactggatatacagacttttatatgatccctgtacagatgtaaataaaatgcttttatttaaaactggtcccaatgttcttcgggaatcatggggtggggacgggggacgcggtagggagcaaaaccgggtacatgggggggaacatcgtccaacagtagcaccagcggattgggtaggggttgctgcggaggtcggtcgatgacgatgtcgatctccatcggcagatccggcaacatctcttcatctccctcaccgaccagcactcggcgctgttctggatgtatatgattctggaaaagcctccgacgagctcgcggcgcgtagaaagccaagcggcgcaagggccggcgagcccgaaagtccatgcgcacagatggcatgagtccttgagtgacggtggtgagctggggaacagggctacctcccatcgcgacggtgacagtggatccatgagagaggcgccgcacgctgcatggctaaataccgtgaatcccctgacgtcgtctttcgtcccgaacgcgtcatgttgggggcgaggcgtaaaccgtcgaggttgaaaaaccgcgtatctgcgacccgtccggactacgttgttttttagaagcggccacatgacctcgagatgtcgtcacccaaggtatttaacggcacacagccagacgcgttcgtcagcagcgacgccgacaagacctcagcatggctcggaggctatggatcttgagcttactagccgtgaccttgacggtggctttggcggcaccttctcagaaatcgaagcgcaggtaaacggaatctggggaattcaacacaggtaagaaatataaaaaaataacgtgattgtgaacgcggttatcgtgtttttgcagcgtgacggtggaacaacccagtaccagcactaactccgatggtaataccacccccagcaagaacgtaactctcagtcagggggggtccaccaccgacggagatgaagattactccgggggagactatgacgttttgattacggatacagatggaggtaaccatcagcaaccacaagagaagaccgacgaacacaagggagaacacaccaaagaaaatgaaaagacccagtagcagcagcagatcccaagggttaaagaccatgttgactattttgttttttattaaaaagctgtaaggttttgctctaaaaacaccccgcctccggtcttttttcttttgtattcggcacgcgaaacacggtttcttcccatagcctgtctaactagccttcccgtgagagtttatgaacatgtatctcaccagaatgctagtttgtagaggctatgcgggatgctgcggcggcgcgaccttccctctccacccagccccgtcaaaacacacgcgactcgagcggttcgtatgaaaaataaaaaacagctttttatttacaggaacggggaaaaaaaaggcacacggtccgtgggagacgcgggttcacgcgtcgtcaaaaagttggtggtccactccgtaaggacaggtaggcttatttagcttccgcatgctcctggttccgtaataaatgccgttttcgtggcagcgtgtcatgccgcgagtcacaaactccatcaaactgtcggccacgatgcaaacgtgctgattgttggcagcaaagacgcgcatacagtcgtccacgaagaggttgatcacgtcgtaggggctcaccaaccagcctaaaggttccacgtggttactgccgaccatgaccctccagtcgttaatctcgctccagtcgtacagccgaatcgtggagacgcgaatgacgctgtaatcacccatgaccatgagtcggccgcgatacgtagcacgccactgcgcgaacgcgtggatgtgcatgcagccggccagcgctctaagcgaggcggtgtgcggcagctcctctgggacggtgatgaagttgcagcgtcgcaaaccgatgttgagaaattcagtgatgctctcggccacaaaggtcaacgagtcagagtagatgtggtcggtccacaggtacatggcgcccgaggcgcccaggtacagttcagacggcacgttgtgatcgcccttgtgtttaagaaagttgtaggtgcagatgctgccgacgaaacgcagcggctcggggcagcagaggtagctggccagacgctgtgcatcccgtccttcgtcgcgcaccaagcgccagcgacgccggataacgaggcagcggtctttgggccagaccagggccacgcgttgcccgggtttccacggtcgcgacgtcttaggaggcctccagcggtcgagcagattgagaaaacagtccttgattaccgacatcgcggtcgcgcgtcggtggacaaaaagaaatcgggccgatccagaaaaaaaaaaaacgacagcgaaacaccgccgtgctcgagcgaagggtggcggagggccagaagaggcggccttgacgacgttggcagcgaaaaaattggcacgcgagtcaaacgggaagtagcgtcggtgttttatgccccaagcagcgtcgtcgtcactcgtggcgtcacagtcaacggtgctgacgtcctttggggcagtcgggcacgcgatcgtagatgccgttgtggccgctgaaacgtcggttttcaaacagcaggttaagtcccagacacatgaacgtgttcagattatctcccacccggatgtagcggtcgtcgcgcacgtcgcaggcgtagacggccccggtataggcgacgacgatggggataaggtcgacgggccagcgcaggtgaggaaagggcgcgttctcgcccttgaggctgacggttcccaggccgagaacgcgcattccgaaagcggttttgatgttgcgcagcaagtgaccgccttccacgctgttttcgaaacacctgaggttgcatagacgcagttccgttcccggcgggaacgtcaatggcatgaactgcccgtggtggcggatgatgaatcgtgccatggtatccaaaccgaggctccaggcgcgcaacagcgggcgaaagtagcgcttaaccaacgacgaggtcaggtagcgcatgcagtgcagggtttcgacggcgcgcagcccgacgcgcgcaaactccatgaggttgcgggccaggtagtagacggcggtgtcctcgcgtacatagcaaaagacatagccctcgtccgagatgaggcacacggcggtcttcttctgctgatccggcgacaacacggcctcgttcacgaagcgacccacgaaggccaggcgcgtctcgcagcacaggtagtgactccaagctttcacgtcctccggtttgaagtcctcgtccgtctcgatctcctgcagcactaggttccagcccggcggccagaccacgggcaacacctggcctgcgttgatgcgcacgtaagcttccagacagcccaggccgaactcggccgtgagcgccaggctagccagatcgctcatgtgacgcgccgagtcggtgggcgagcccgggggcccgtcgcacaccacgctccgtcttcttgtcctcaccgcggccagcgtggcgaggacactttccgcgcccgaggctgtatcttcggtttgcccgccggagccggccctcactatataacgtcccgcccgggtctcctccatgtatgcaggtaagcaactgagccgaacgcacctcagcagacgagaggatgtcgtcgcggcgtcgcagctcgtcacgtcgctctggcgaaccctcgacggtgatttatatcccctcgagcaacgaggacacgccggcggatgaggaggcggaggacagcgttttcacgagcacgcgggcgcgcagcgccacggaagatctggatcgcatggaggccggtttgtcgccctacagcgtctcctcggacgctccgtcgtccttcgagctcgtgcgcgagaccggcggcaccggcgccgccaagaaaccgagcgaaaagaaacgatcgtcgtcacgtcggcaaccgcagatcgcagcgggcgcgcctcggggctcgccggcgacacccaaggccggcaagtcgcctaaagtctcgcgaccgcctagtgtgccctcgctgcccgagaacggcgccggcggcggtggcgacgataacagcagcagcggcggtagcagcagtcgcaccaccagtaacagtagcagaagcaccagtcccgtggcgccaggtgagccgtccgctgccgagggcgatgagttttccttctgtgacagcgacatcgaagactttgagcgcgaatgttaccgggtcagcgtggccgacaatctgggcttcgagcccagcgtggtcgcgccgcagcacgtcgagtatctcaaattcgtgctgcaagactttgacgtgcagcacctccgccgcctcaacgaatgcatacccatgccggccttcgcgctcaccagcctcgtcgaccccgtcttaaacaacgtagcgcctggcgagcgcgatctcacgcgtcggataatcacgcacgcggtgatcatcaactattactacgtggcgcaaaagaaagcgcgccacatggtggaggccatacggaccaccgtgcgggacgacacggtacgccgggtagccgcgcaggtcaacaaccagagccgttcggggcgtgcggccgcgctagcgcttcactttctcacgtcacgaaaaggagtgacggacggtcagtacgccacgtctctgcggcggctggacgaagagctgcggcatcgcggcacgcccgaatcgccgcggctcaccgaggtctaccagacgctacgcgattacaacgtgctcttctataccgcccactacacctcgcgcggcgcgctctacctctatcggcaaaacctgcagcggctcaacgaaaaccaccggggcatgctccggctgctttcggtcgaagagatatgcgaagagcacacgctcaacgatctggcgttcctagtaggcgtcgagcttatgatcacgcactttcaacgcaccattcgcgtgctgcgctgctatctccagcaccagctgcagagcatctcggagctgtgttacctcatctatgtacaactgccgtcgctgcgcgaagactacgcgcagcttagtgacgtgctctactgggccgtcagtcaaaactacgactacgcgctctacgcgagcacgccggcgttgtttgactttttacgcgtcgtgcgtcagcaggacgccttcatttgcaccgactacgtgtactgcgccctgcgtctgctggcctgtcccgacagacctattatcggtgacaccggcggcagcagtagctcccaacgcctcgtaggcgagtttatggtgcgcgatccgctgttgcgcgacccgcgcgccacccacctgcgccagaaactcatcacccgcgacatatgcgtggcgcggttgcaagcgcagccctcgagtcgacacattccggtcgaacacacgggtgtctcctccgtcaccctgctcaagatctttagccaggtcccccccgacgaacgcgaagaagacacgttacgcgagatggctcttaaagcgtttatggaagcgaacggtaatcaccccgaacaaatctgccgatccccaccacccccgctgccaccgcgcgactatcctcaacgcgacgagcgggaccgtcaccgtcgcgaccgccgcgacagcggggaatactgttgctgatggtgggacgaaacagcagggcggaacagtttatgatagaaagtcacaggaaagtatgtgttgttttttttttaatgtaccaagaataaaaagtgcgtctacgaccaaagcggtgtgtggacgctcgtcctctgtcttctccggtttttttttatgtgtgtgtttttcttttccttcctattttgttacggcaacagcgctgatggcacgttgccggcttcgaacatcgcgtcggtgatttcttgcttgcccggcgtcacacggtgacgcagcagcgcgcggctcacgtagcaggccgactcgcggatgacctggccgtcggcgtcgcgtcgcaggcccgagcggttgccgtgacgcagtcggccctgcgcggcgcgctccacgtcttcaaagtagctgtgtagcaggccgcgctccagcagctgcggcagcgagtcggcggcgcgcaccacaaagttctcacggctgatctcgtagcacagcacgctgccgtcggctgccacgccggccacgctgcggtcccaactgaagaggttggcgagtccgatggtgccgatgacgcgcaactgaccctgggtcaccaccagcagcttccagtattctacgtcgcgcggggtgaggatggtctcctccacgtcgcagacaaacaacgtgtagccgcgcggatagggcagatccaggtggcgaccgcgctggcggcgcataaaatcgtctaaattcaaaccgccgtcgggtgcgcgcctgctcgtcatcgccgcgcctcgtcggtcgatgaccccacggtgcttataacgcgccgccgcggcttcatgtggcgtgacctccgacctcgtgaggccgaaaacggcgtacatgaagacgctcaaacttttgaatgtgggcccggtagcgcaccgagggccccggggcggcgacgacggcgggtccgagttccagcggggccttgcggcggcagcggttggcgtggttgctcagctcggcgtccgagagcgccgagctgaactgcggcagccgcgtgcgatcctgcggcgcgtccccgtgtcgcagcgagtgccagagcaggcgctggacgcgcgccgtctcgggcgtcggcggcgcgcgacagccccggcgcagcttgaaaacgtgcaggcacagcagctcgcgcttgatgcgcagcgacacgctgcggtagtcgggaatccgctgcaccagctcgagaaagtcgcagaaggtctccacgaacgtgtcctcggtgaagcgaatgcgcttcagatcgtggacgtgtttgcgaaaccgcgacagttctcgacgttgcacggggttctgagcgagtcccttgcgcagcagcgcagcctcgcctttaaacagcctgatgagccgctgcacgtccccgctcaacatacgtatacacgccgtgtactcgtgacgtatactggcgcgcagcagccgaatgatacgcagggccagcacggcgttggaggccaggtacatggcgtagccgcgacgcgggttggcacaggcccagcccgcggggagcagaaagtagtcgtcgaccagcgtctgcgaccagtcggcgaagcccaggtcacgtgatacgctgtcctggacgcgggccacgtcgccggctgtgaggtggcggatcgccggcaggtgaaacgcgcccaggtgtcgattgcgctccagcctcagctcggcgtgctccaaacgggaatggtgggacgccaccgcggagggcgacaaagaggagtggtcgccgccgccgtagttaccgttgtgattaccgccgtcgtcgcgcccgtcgccgcactcgcaaaaggccgcgtagaggtccttcaacgccgcttcggctcgcgccataaacgtggcgtggaaaaaaacggcggcgcggtgcgtccggtacttgacgggcaacccgcggcacagggccgccggcaggcagcggccgatgagttcgcgctcctcgggctccagaaacaggcacagggtgccgtccaggcgcaggtacagctcctcggtcatcgagcatagctgccgcaagtaatgggtgcgcgtcccaaaggtcttgtaatcgagcaacgtgcacaccacgtattgccccgtggccacggccagagcgatgcgtttggcggcgcgactgatctctggcaagtactgcgcctcgtgcaccagacggcggaaagcgccggcgttgagccagcgaaaatgctgcggatcgggcggcaagggcacgcctcgaagcgcggcccagacagcgaggtccgactcgagcgtcagaccgcggatgtcgtacttgccgtgcgccgtagcgcaggctgaatggaccagacagctgcggcgaatgtacaccatggcgtgcttgggatgtttgggcgccggcgttttctttttctgaccgccggcggccgccagatcctcgggcgtgcgacacaacaggccggcgcgcacagcctcctgtcgattacgaatcggcgtcaggtaggcgcgcaggaactggtgacaaaactcctcatcatcacgacagtcgtcgagatactcgtacgtggtgagcggatcgcgaaataggcgctcgtcaccgtcgtcatggtcttctttagcctgctcctccggctgctgggttggcggtggaggcggcggctgatccacggggttcatgactgagaggaagaagaaggtggcggcgaagcgacgcggagcgacggcggtaaagccagacaccggctatatagctagtcatcacagtctcctccttcacgacgcccccgtgccgctcacgctatccagcacgctacggcccgaaaacacgtactcgctgacgtcgtacgcgggcgatgtatggctgctcaccggtttcgcggcgacggttgcgctcgagtccaacggcgagaagcaaaaacgccgtgggcaacgaaaccagaaggagccctgacggataaaaccgcgcagcgtctcggccaacttaaccagcatcgtaccgtacagcagtacgtgaatgccgccgtgcgcgtccataaatacggctttgtttacgggttccatccatccgatgactacaaagtgagcctgttctagcacgccgatcacaaaattgttggcctcgtcggcctcggccacattccacgagccgaaagtgaaagtacaagcgggcgagccgcccaggcggattttgctaccggcgtggagctgacatacgcgcagcagattggcgcggtcgtgcagtatctgggagagttcgtacatgcccgcgaaggtgtgcttaaaccacgcgccctctacgatttcatccacgtaatcgcgctcaaagaagctatacacggcaaagaggccgttctcaaaaaactcgccgaacgagagccccagcacgtacaccttgtcctcgccgggcaggtacgcaaaggcgtgcccgtgcccggagacccagatctcgggcgccgtgtttgcgtccggcacgcattcgtacacactgacgaggccgataaagtacaagcggccagcctggcgcaggcacgagaagcgccggtaggtcttgtgatcgcgcaccaccccaaagtactgagtgtcgcccagcatgatgccgtgcagcggcggccagcacagcgggagccaacgacccgccgtggcgcgcacgtagcgctgcaggtgaaccccgctcgcacgctcgcgcggcttcgggcgcttgtgggtccaggcatcacgcagaccgcgccagatgctgctgaacttgggctgcccgcgcagatagagcgacgagagcgagtcaaagtagcccacgacgagcctgtcgggagacacaagagcgcgaaaatcaaacctagagcgacgacggtgaaaaaaccgattataagcgcgtgtctcaaacacgctactttcggttataaaaacaccgtcgccctatttctgggcgtgtgtacactgatgactcacctacgctttttgaacggcagtctcagctcgggattggcctcgtacagcgagctgcggtccacggggccgatgctctcgtagcgaaagtcgtcgatgagcagcgccagccccacgcgcacgaagcccctgaggtcgcgcgccagccgcaccaacttatcctgccccaccagcgccgcgtacacggtacccgtgtcgccgcagagaatccgcacgcggtgaaagaaggtcttgtcctcggcgccctcgatctcgcccagcggcatgacgggctcgcgcgtgtacaacgaacgttgaaagcggcgcagcatcgaggccgagagccccagatcgcgcgccgtgcgcagcaccagggaatgcttctcgggccagatgagggtcagctgcgcctcgcgatgcgcctctacgtaggcgcagcgagcggcggtgtcctcgcaagccagcaactcgcggaaagccagcagcgaacgtaggtagcggccgcgagcggaggcgcgcgagcggcggcacagctcggcccgatgatcgggatgcaccaagggcacgttgggttgcagacgcgcgcagatggattcgtgcaccgggtcgcagcggatcatgcccttggcaaaaaatccggccagatccgaggccaactcgtacaggcagtcctcttgcgcgtcgtaggcgaacacggcgccgtacgcgtccacgaacacctggtaccggcaggtggcgtgcgagaccgtgccaatgagatgcagagctcggaattcgccgaaaaagtcgttctggcagtgctccagatcgatctcggtcagcgagtgcggcgaatgctcgcccccgaccacgtagatgcactgcgagggccagcccagcgacacgcacgagccctcgaagcgccgcaagtaacgccgcaggccctcatagtcgcgtcgcacgcacaggtcggccaagtcgcgcgtgcaaaagacctcgggtaccaagcagcgtttgcgacgcggccgacgcgcgtgcccgggcagaggaggaaggcgcgacggcggcgacgacgaggaggaagacgccgtggccgccgagcagcccttgcgacggccggacatgccggcagtccgcgacgatccacaggagacaaaaaagcagaagcagcagtagcctcggcgacccgctccaccccgtcctccacacgctcagccgcgactgaacgccggggcgcgccgctacttgggtttttatagccatctgccccccgtctcgggcacccgggagcgatctacggagacctgacagcagttgggcaacacaagatagggaaatacaaagacacttttaataaaaaacgagactactttgtgtgtgtgctccgtaaactgtttattctccccctccgcttcgctctggatgggctccgggcccgtcaacacgcgactcgcgcggcaaaaggcacgctgttgacggcgcgagagcccgtcgtgatagtccatcatgccccggagatcgtgcacaaagcagctgtcgccgcgcagaaaccgacgcagcgtctccacgtgctgcagctgccggcgcgtatcaggagccgtcatcgctgatgtcgtcatcgccctgacaggcgcgtagatggctccgcgagatcacgcgcgttttcaaccgccgtgacacatcaggtccatcttgagctggcgccgggcctcgcgcaggtgtcgcacgcgttgtgagcgggaggcgagttcggcttcttgctcgaactcctgctgctcactgtccgagagggtgcgataaaaggcggcaaagtcctccaagtcggctacatgcgccctgggtctgacgctccaaagcgtacgcagtctgatgaagcggacccatcgagcgtcacggcacgccgtcttgaacgcggggcccgggaagaggttcttctccccggcgcgctcgggccggcgaggccgacgcggtttatatacaccgtctcggacggcgggacgccgagcccgcgccgcggccgctcatccggagacggcggaaaccgcggcgccggaggaaacggggaccggcaacgacggcggtggcggcgaccagattatgggggaaaaacccacgcttgtaaccctgttgaccgtcgccgtgtcgtcgccgccaccgtcgtcgccgctgccgcttgtcagcttcacggagctgctgttaccgccgccgtccgtcgccgccgccgcggtggcggcgacagcgacgagcgaggtgggcgagaaaaccgcggagcaagaggtagcggctgcgggtccggagaccgggaatgagagaagagaaaacagggagaacgaaggaggggagacgaggacgacagacaccaccgcggtcaaaaggtcgcacgacggtatccctcgccaactagcagagcgcctgcggctgtgccgccacatggaccccgagcaggactatcgtctgccggcgcaggacgtggtgacctcgtggatcgaagcgctacgcgacgcggaccgcgataactacggtcgctgcgtgcgccacgctaagattcaccgttcggcctcgcacctgacggcctacgaatcgtacttggtgtccatcaccgagcagtacaacacggcctcgaacgtgacggagaaagcttcgtacgtgcagggctgcatctttctctcgtttcccgtcatttacaacaacacgcagggctgcggctacaagtacgactggtccaacgtggtgacgcccaaggcggcgtacgccgagcttttctttctgctctgctccaccagcgagagctccgtggtgctgcaaccgctcatcaccaagggcgggctctgctcgtccatggcggtttacgacgaggaaaccatgcggcagtcgcaggcggtgcagatcggttttctgcacacacaactggtcatggtgcccttcgtgccgcacgcctgcccgcattacgccgtgcctttcacgacgccgggaaagccgggctgcggcggtgctccgagcggcgttgcggggttggaggaggcggcgccctttggacgggtcagcgtcacgcggcatggcgcgacgctgctgtgtcgcgtggaccatctgacctggatcagtaagcgcgtaaccacgtacggacacaaaaaaattacgcgctacctcgcgcagttccgcggcacgatggacgacgacgaggcggcgctacccggtgaggacgaagcgtggatcgcgtccaaaaacgtgcagtacgaattcatgggtctcattttcaccgtcaacgtggattcactatgcgtggacgcggaacagcgccaactgctgggcaccgtggccacctccttctgtcaccgcgtctcggacaagatcacggcgcgcaacatgccgcgcgccttttccttctacctgctgacgagcgcgcagcgcgggtacgacctgcgatttagccgcaacccgtcactcttttttagcggcgacgcgctcaactgtccgcttctcaatgagcccaacgtgttttcgctcacggtgcacgcgccttacgatatccacttcggggtgcaaccgcggcagacggtggagttggacttgcgctacgtgcagatcacagaccggtgtttcttggtggccaacttgccacacgaggacgccttttacacggggctcagcgtgtggcgcggtggcgagccgctcaaagtcacgctgtggacgcgcacgcgttccatcgtgatcccgcagggcacccccatcgccacgttgtatcaaatcaccgagggcgacggtaacgtgtactcgtacaaccaccacacggtgtttcggcagatgcacgccgccggagcaaccacgttctttctgggcgacatgcaattgcccgcggacaactttctcacgtctccccatccctgaccctccgtccgtcctcctttcccgacacgtcactatccgatggtttcattaaaaagtacgtctgcgtgtgtgtttcttaattattcctccgtgttcttaatcttctcgatcttttggaggatgttctgcacggcgtccgacggcgttttggcgccccccatgccggcagaacccggttgcggccccgtaccgctcttctggggcgacgataggtcgaaagccaccgttttcatgcccgtcgtgctcttgacgggggaacctacggcggcggttcccgtcgagcggcgtgattgcaaagccgcgctcgcccccggtttcaggatggagggagaggccacaggcggcgcattcgatacgctgcttttggccgtagacgacggtgggtaaacggtggttaccgcgggatacgtcggcgtggtcgaggcggcccggctggtgccggacaggcgacccggcgcgctaccgctcacggggaccgagggcggtcgacctaccaccgctttgccgcccaaagtaggtttcaaggaaggaacaacaccgacacggccgccccggcctttcaccggagacgggggggcactcttggccggggacggagaggctgacgaaagcatggacagcggcgatgtggcgggggacacgacatcatcctccgtgggcgacaaaacggacgccgaagctgacggctgtcgagccgaagcggaagaggttcccgcgccagaagtcacgttccttgatgacgtcgttttagacgaagccggttgaggttgcaacagcgtggcgggtaccgtcgacggcgtgcccgacacctgtttctctagccttccctgaaccggtgtcgacgtcaccgtctgcgctcgggcggacgcgtgcggcgtcgcgactcgcttgcccagcaccggtttctggctcgtggatgtcgtcgtcattggagacgataacttagctttacgtattctggacggcgtcgactgctcgggcgtctgactgggaggcgaaatgacgtcgttgtaatcggacgacggtgttgtgtgtcccaggctgacgacggagccggtgtccgaggagtcgtcgtcttcctcctcgctgtcttcgaccggtgactctgcagtttggtcccttaaagcccaaacctcatcagcggcgttctgagacgctgtttgtgtcaccgcggcgcgtggagtcgacggcctccgaggggtggtggacacggtgttttgagaagccgtggaagtcgtaggcatcctgaagggattgtgagccaggtgaggattcttgagggcccacgcgcgttcgcgcggccagttggcggggttcatatccccgggcaacggcgccgtcggagcccagggcgagttaccgttgaccggggtttgggtacccgcgaaggtaggtgtcggggccggagcgggggccgtggaaggattgacaggcgtcggcgtgaggatggcagtgccggcgccagcagggacgttaactccggcgccgaacgtcaacgtcggttgctcgaacttgtacgcggtggtgacgggcggtttggcactcgtctcggtatccgtgatgtccaccagcgtgtcggtgaaacgcggatcttgacggttggggggatagccatccgagctgtcggaatcctcgtcgcccgagaaaagatcccctctggtctccgtgagcggcctcacgtcccacgcgctgtcccgacggacccttcccgggctggccttggtcacctgcggggagacgagactgaaagccgcgtgacgctgttgttgctgcgggatgttcaagggaccgctggtcggtttctgactgcccgaggataacaggccgctgaaaacgctggaaacaccgccaccactagcgacgcccttgccgctagttcccggtttcttgatgggcgtaaagatgtttttctcgtcatcgtcatcgtcgtcgtcctcatcggcactggagccaaagagcctccgggaggcgctcggtttacgtgccgggggcggtggttgctgttgacgttgctgcaggttctgctgcctctcctcccaagccttcagctgctgtttctcacgctgcaccacctcgtcgtccacccgtttctgccgctcgcgacgcttttcctcttcgtcgtaatagccgacggccgccgaacgggcggcgtgggcgtcggcggccggtgccagagaaccatgggcctcgaagcggaacggtttgtgtcccttccagggactggcgatccagctccagccgtccagcggctgcgtggggacatgtttcttgggtaccgacgagaaggccgaaccgccgccgagcgagaggagattggcgtcatcatcaaactccaacgacggcgagcgcgcgcccaaaaaggtgtgcgccgactgcgggaagctgtccacgtagatgtcaaagtcctcgatgagcagctccagcagcgtgtcggccgagtcgccgttttccacggcgtgcttgaggatattgcgacagtagttggaatcaaaggaaaggcacatacgcagctccttgaccagcagcttgcagcgctcctgaatgcgcgccagacatttgcgctccagctcctcccaagacctacgcacgttcatgatgagacggcccgtgtacacgagcttgttgacggcgttgaccagcgccgtgttggcgtgccggtccaggttaaggtcgagcggtttcacacagaacatgttacggcgcacaccctccaggttttcttcaatgcgctgcacctccgtatccttgaggtgcacaaaggcgatgggttccgtctggccgatggctgtgaccagcgtctcgcgcaccgacatcttggccagaatgaccgcgcttacgagcgcgcgctcgacgatctcggcatcgtggcgcacgtccgtatcgaattcggtatggtctagcacagccaggtgatcgcgcgccttaccacgatcaccgaacgggtaagtgtagccgcgacgcgccacggccgcgcaacgcacctcgaactcctcgagcaccgaggagaggtcggggttgtggaaacgcagctcgcggtagtatcccaaccaaagcatgagctcgttgaacagcaccgtacgccggtgcaggcgtttttcgccacattttttcaggatcttggggtgtgcctcgagatccacgtcgggcttttgcgtgagatggcgcagaaagttgaccagggctaccacatcgcgccgctgtagaccgataaactgcaaactcatgctggcttttctccagaacccggaagcgtcgtcgccccggactgcgcccgcggtctgctattcgcccgcgatggacaccatcatccacaactcggtgagcgtcccacccaaagggagggggggtagtttaatagcggaggcggatacgcggttttcttttaagcgccgctgacttgtttcttctgttttttcgccccgtgtgctgttccgcccagacccgcaacaacactcctccgcacatcaatgacacttgcaacatgacagggccgctattcgccattcgaaccaccgaagccgtactcaacacattcatcatcttcgtgggcggtccacttaacgccatagtgttgatcacgcagctgctcacgaatcgcgtgcttggctattcgacgcccaccatttacatgaccaacctctactctactaattttctcacgcttactgtgctaccctttatcgtactcagcaaccagtggctgttgccggccggcgtggcctcgtgtaaatttctatcggtgatctactactcaagctgcacagtgggctttgccaccgtagctttgatcgccgccgatcgttatcgcgtccttcataaacgaacatacgcacgccaatcataccgttcaacctatatgattttgctattgacatggctcgctggactaattttttccgtgcccgcagctgtttacaccacggtggtgatgcatcacgatgccaacgataccaataatactaatgggcacgccacctgtgtactgtacttcgtagctgaagaagtgcacacagtgctgctttcgtggaaagtgctgctgacgctggtatggggtgccgcacccgtgataatgatgacgtggttctacgcattcttctactcaaccgtacagcgcacgtcacagaaacaaaggagtcgtaccttaacctttgttagcgtgctactcatctccttcgtggcgctacagactccctacgtctctctcatgatcttcaacagttatgccacaaccgcctggcccatgcagtgtgaacacctcacactgcgacgcaccattggcacgctggcgcgtgtggtgccccacctacactgcctcattaatcccatcctgtacgcactgctgggtcatgactttctgcagcgcatgcggcagtgtttccgcggccagttgctggaccgccgcgctttcctgagatcgcagcagaatcagcgagctacagcggagacaaatctagcggctggcaacaattcacaatcagtggctacgtcattagaccccaatagcaaaaactgcaatcagcacgccaaacgcagcgtgtcttttaactttcccagcggtacgtggaaaggcggccagaaaaccgcgtccaacgacacatccacaaaaatcccccatcgactctcacaatcgcatcataacctcagcggggtatgagctttcctgttactttattcagaaagcaccagaacccgtcgccatttcccctcatatacggtacacgtccccctgatctgtcatcacggtacacagatttcgcccgactgcggacgccgacggccaatcgcgtggcgtaggagtggcgccccggcttcattataacgccacgtcggagcccctgcgcgccacaacgccgtccggcgcaacttctgtctcggcacggtacgataaaaacgacgtcccccgtcgacgttgttttctccgagcggtgatcgttcccgtccctatcctccctccgcggcccccacggcggcggcctgctcgcacggacctatactattaccgccccaccgccgtcgtcgtcatgaacttcatcatcaccacccgagacttctccaacgacgattcagtcctgcgagccgccgagatgcgtgacaacgtggcaggctcgatttccaaagcgtacaagggcacggtacgcgccgaaggcaagaagaagctgctgctgaagcacttgcccgtgccgcccggcggctgctcgcgccgcaacagcaacctcttcgttttctgcaccgaacgcgactaccgcaagttccaccagggcatcgcacagctcaagcgcgcgccggccgaactggacccccacgagatccagcaagtcacggccagtatccgctgccgcctgcagcccagtctccgcgagccgcccacgccggccgacgagctgcagacggctgtgtcgcgcgtgtgcgcgctcttcaaccagctggttttcacggcccagctgcgccactactgcgagcaccaggacaaggtggtgagctacgcgcgcgacgagttgaccaaacgctgcggcgaaaaatcggcgctgggcgtggaggtgcatcaactggtagccttgctgccacacgagcgccaccgcgaactgtgccacgtcctcatcggcttgttgcaccagacgccgcacatgtgggcgcgctccatccgtctcatcggacacctgcgccactacctgcagaacagcttcctacacctgttgatgaactcaggtttggatatcgcgcaagtcttcgacggctgttaccacagcgaggcctaccgcatgctcttccagatcggtcatacggactcggtgtcggcggccctggaactctcacacagcgcggcggccgggctgcccgaggccgatgagaacaacgacgagggagaggaggacgacgacgagctccgtcacagcgacccggcgccgcttcacgagtccaagaagccccgcaacgcccgtcgtccccgcacacgcatgccgcctcacgagcaaaagcccgaagaaaacgaggaggaagaagaggagctgtttccctcctgcaaggcaaccgcagcattcctgcgggcagaaccctccgtctccaacgacgacggcaacggcggcgaacgctgcgacacgctagcgaccgccctgcggcattgcgccgacgaagaagacggacctctagccagccagaccgctgtgcgggtcgccgcgaccccctcaccttcagtcaccccagcccttacccccgtcacgtcccccataaccccgttgtgtatttaacgtcactggagaacaataaagcgttgatttctcaagttccgctctggttttggtttcgttttcaaagggagccccatcatggcccaaggatcgcgagccccatcgggcccgccactgcccgttctccccgtggacgactggctcaactttcgggttgacctgtttggggacgagcaccggcgcctgctgctcgaaatgttgacccagggctgctccaactttgtggggctgctcaacttcggcgtgcccagccccgtatacgcgctggaggccctggtggacttccaggtgcgcaacgcttttatgaaggtaaagcccgtggcccaggagattatccgtatctgcatcctcgctaaccactaccgcaacagccgcgacgtgttgcgggacctgcgcacgcagctcgacgtgctgtactcggagccgcttaagacgcggctgcttagagggctcatccggctctgccgcgctgcgcaaaccggcgtcaagcccgaggacatcagcgtgcacctgggcgccgacgatgtgacattcggcgtgctaaaacgagcgctggtccggctgcaccgggtacgcgacgcgctggggctgcgcgcgtctcccgaggccgaggcgcgctatccgcgcctcaccacctacaacctgctgttccacccaccgcccttcaccacggtcgaggcggtggatctgtgcgccgagaacctgtccgacgtaacacaacgtcgcaaccgaccgctgcgctgcctcacctccatcaaacgcccgggctcacgcaccctggaggacgcactaaacgatatgtatctgttgttgacgctgcgacacttgcagctgcgacacgcgctggagctacaaatgatgcaggactgggtagtggaacgctgcaaccggctttgcgacgcgctttacttttgttacacgcaagcccccgagacgcggcagactttcgtcacgctggtgcgtgggctggaacttgcgcggcaacacagcagtccggccttccagccgatgctgtacaatctgttgcagctactgacgcaactgcacgaggccaacgtgtacctctgcccgggatatttacatttcagcgcgtacaagctgctgaaaaagatccaatcggtctcggacgcccgcgagcgcggcgagttcggggacgaggacgaagagcaggagaacgacggcgagccgcgcgaggcccagctcgatctcgaagccgatcccacggcgcgcgagggcgagctttttttcttctccaagaacctgtacggcaacggtgaggttttccgcgtgccagaacagcccagccgctacctgcgccgacgtatgttcgtggaacggcccgaaaccctgcagatcttctataacttccacgaaggcaagatcaccaccgagacgtatcacctccagcgcatctatagcatgatgatcgagggcgcctctcggcagacgggcctgacacccaagcgcttcatggaactcctcgacagagcgcctctgggccaggagtcggaacccgagatcacagaacatcgcgatttatttgccgatgtttttcgccgtcctgtgaccgacgcggcttcttcgtcgtccgcgtcttcgtcgtcgtcctcagcatctccgaattctgtttcgctgccgtctgccaggtcgtcatccacacgaaccaccacgcccgcgtccacgtacacctcggccgggacttcttctaccacgggtctcttgctctcctcttcttccttgtcgggatcgcacggcattagctccgcggacctggagcagccgccccggcaacgacgccgcatggtcagcgtgaccctcttttcgccctactcggtagcctacagccaccaccgacgtcaccgaagacgacgcagcccgccacccgcaccccgagggccggcccacacacgcttccagggacccgacagcatgccgagcactagctacggcagcgacgtcgaagacccgcgggacgatctggccgaaaacctacggcatctctgaacgcggtttttcctctttttctacgtgtctgtctcaggacgagacgtcgatatcaataaaaataccgtcgacgtggtttttttaacagtgtggttttctttattgactagcggagtacacagtttacgagtaaaaaagacagggaaaggttatataaaatgctgtattatatacaaaaacatgcacataaacagacgggaccaccgtgctcgtcatcctctcctcaatcagttgttcatgtaggcgtgtggcggggtgaggggcggcatgccgttggcggcgccgggaataatgtgccgtcgaccgacgtcgcacaccttgaaacgccgtcggcgcacgcagcggtcgcaggacgggatatcccagaggaagcccatgtaggtctcggggtcctcgtcgtgaaagcggtaggagagttcaaagtggtgcaacgagcccgtccgagctcgcagcttctggcgaacaccctccacgtcatcggtgcacaacgacagtgctgggctctcacacagggcctgaagctcctgcggccacaggtgcgtggccaggggcgagtccgtcgtcaccagtttgacgcagtgcatcaggttctcggtgatggcgtcgtacaggcgactctcagcctcctcgtgcgtcatcacgtttcgaggcagcgacagctcgtcgtcgtcatcctcgtcaaacatgatcatggggtcaggggtttttttgggatgttgacaggtgggtgtcttttccagacgcacgatggcctcacgccggccgctgaaacggtggtttcggtgtcccttctttcccatgacgcaggtgaacataaccacgtcctcggccaaacggtagacggcgtccatggcggggtcgtagccgtagacgacgccgaaagtgtccaccaagacgtactggcgtacgaggaactctttgcgttctggcacctcgtggcccagcgcgcccaacaactggtggtaacaggtgatgcgcggcacggtacggatcatgagctccatggtctggatgctgccgcccgcgcggacgacgctgaaggatgtttccttgaacttcataacctctgtgttgtgggtccagaaggcgaaatgggtgtcgggacactcatcgaaagggtcgtcgatggtgtaggaagcgtagccccgcttggtcacctcggccgacaggctctccacgtcaccgcggtagagcatgacggcgttccagtaatcgtcgtactgcaccatgggccgctggtagtcgcgcatagtgtggaagtggtcgcagtgacgaaagccatgccgcagaaagtccttcatggtggatgccagctcgtagacgcagtcgcgcaggtcatcgtagcagtagatgccgccgcgctgcccgatgagcacgatgagttggtagcgcataaagcccggaccctcgacgaagccaaaggggtgcaggtattcctgacagcacacgtaagcacctggtggagaaataagaaaaatccacgcacgttgaaaacacctggaaagaacgtgcccgagcgaacgtcctctttccaggtgtcttcaacgacgtggggcttaccttgcgaacagacggtgcccatcttgcccacgaagggccccagggcgttgcgcgaacggagctggatgaagcagcgttcgggccaggccacgtgcagccgggtgccgcattcctgctccagaaagtcgttgagaccgttaaagtccccggctcgaatggcgatgcagccgtaggccatcagcgtgtcccgtaggtcgtccatgacggactcctctaccttcgctcgccgacgctgcgcttctccagccaccgctgcggtcgacagactccttcgtccgccttcggagaactacggcgcggcggcacggcctttatagacactatcagcgttgacgtcagacgatccgatgaacgtcgttttttgtgctggaacttccctcgtcccgacaaatgtagcggaaatcttcaagcaaatcgcgacgaagtccgatgaggaggatgcaaaagaggctgagcaacgcgatgctgcccgccgccacagtacatatgctcaacaacgcccagtgtcccaacgcgcgacttttggctcggagcagagccgaacggcggtttctccacatgacagataacgtggtccagtacgtccatcctttgcattccggcgtccagacgggaagcgttgtcatgttagttcccgtaaaggtcgtgttttgtcttgttttgtttctcatgagtttaacagtcctttttagaaaccgcgggcacatgtcttgtagaaagatgtaatcactctccgcgtatgtcgctagggttgacatcacagtggtagtgttttccgaagaagtgacgttgtcagtgatattgtcagtgacgttaatttcttcccagtgtacggataactcgaacggtgtcgtatgcgccaccgctctcaacacgtaactacggccggtgaggttaagtgttagttgtcccacggtcacattggtgtcatttgtaaaacacgcgatttctccgcgaacttccgtgacgttggtttcacgggtctcgttgagaacacgcagaggaaaccagccttccagatgatactggaaaccaaacgtaagcatgacgctatgccattgtctccgtggttgccgaaacgttacgttcagaggcagtttggcttcggctcctgcgcaaggcccgttatagatttgcgtgtcattgcgcgtacagtttaaccggcagttcatactcgtggtgttagaagtgatgttaacacccgtgccgtggtacgtgcatcggaccgaaacaccgtgtcccgtgctccaaaacagcgtcaacaacagccacacagacacctacgtggagacgacacgggactttttattgacggagactcacgtttctaccctcccctttcccgtaggtaaaaacccacgtttatcacacacgttgtttttacctgaaacccgcgcagcccgtggacgcgacaaaaaaccgcggcactagaaagaaaatgaaacaagtatgtttattaagcagcatgtggggctaataggggggataactgaggtatagcaactatgaaaaaatactacaaaaaaaaaagctgaacatggtcatctagcagcaaagttctccttctagaccacgaccaccatctgtaccacgtcgccctccccggtcgtgtacatcacatccttcaccacgaccggtggcaacggcggcgacgaggacaactcgctctcgacggaggccgggacgacagaggacgggggggtggtggcggcggaggacggaggggtggcggcgacagcggggtcttcttccgacacgggcgacggcaggctcggcggcgcggacagcacccgttgcgccggggcgtgagaaggctgagccccggtggcctggatgtgggccaacgaattggctcgcagcgagtcgcgatccacgaaggtcataggaattttcccttcgcggatccgccgctcagattccaggatggcgcgcacgtagctgttcaccgacttggcaaaagtgcgcggcccttccgtattcttgtcgcgacgcgcttccagcacctgcttttcgtagtccagctggtggaagaccatcaccaggtcgtccatagtgtgcgcgtgctgacggacgtgggagcgcacctccaccgggaacaaagcgttccaatactccagcacgatggcaccgtgccagaactgcgccatgctgggcgccaggaaaaacaggataccggagtcgtaggcgaacacgtcccacttgggcgtcatgaacaacaccagctgacgcgtgggccgcaccgaagcttcctcccaggcctcgatgaccccgaacatgatgagctcctggtccaacggggggcagtgtcgctccagccaactgatcttgctcaggttcatctgcagaaactcgtaagaggggtcgcagatgcacacgtagagacccgagtcgtgccgcagcctggctccgcgcttcatcagtttcctcaccgcgtagcgaagcgccaccttgcccaacgccgacgcctggatcagtccccccacgtccatctgcgtctgtcgccactcggcctcgtccagcaggctcgtgatagcggaagtgctatgcgtggtcgtagtcatcctttctatccttctctatgaatagcagcaatagcggtaaagtcccttcttatactatcccggagtctgtggttttttttgtttacccctgcttactggtgagactgctgggggccgttgtgctgcagcagctgagctcgtcgccgccgttgccacaggaaccggtgcctccgcagggcctttttgagggcctcgcaggcttctcgcgcaagtcctgagaggccctcggcgtcgatggggttcacctcgggcgtccgagcctcgttttcttcttcttcatcctccctttcctcctccgtgtcctcccgctctgtgtcctccgttacgctctcctccccggcctcggccaagagcgcagccaccaagtccacggaccgctcggtctccgagttctcaccgtcaattacgccatgttggcggcgtaaccggtgccgagaacgccgggtgagcgcacatgcttttttctttcttaaccaaggcgggagaggatcttcaaggcgttttcgctggatccagcggtagctaaagtaccaaaaggccagcaggcccacgctacctaacagattcacgtagactggagacataattaaagaaagaagtgaaacccgcgtgtgggtctcacgtcgtcttgaaacaccgtcttatatacatgaagatgccggacatgacgcgcccaagacacgtggggtttcccccttaggggacccggtttcttaagatgtttttcatcttcgcacgcgatgtactacatcaaagggtcggctgaccgaccgcattgacgcacagtttccgagtacgcgcgtctcggagcacctgacggtgagccacccagctcacgcggataggggacaacactgacgtgaggggcgattcacgtcactgacggctgacgggaataagacgggtgagggatttccacctttttcttaagtgtgactctccttacggtaaatcgcacctgtgacctcttaacccctcctccctggtacccaataacagtgaaaaacacacaccacacgtcacgacaccgatcgattttctttattcttagtgtgatgataggtaagggcactcgtgaggatgtgcagttatcattatcaagccttcttcaaggcgtagtgatgatcgttgggcagaacccccaagctcctagcgatctgggaatagaaggaggagaacgaccccagggccagaatgcccacagtgtacatggcccaggtctccagaccgaacgtggcgggtcgcagcttcagatggtaggccacccgctccgagagttgtgaatgctcgttcaggcaacaggactgcaggtgggtgagcccaaaagcgctttcgtttacgccgcgcacgtgcaccgtctgggccgggcaatcctggtgttgcgcgcgaaaatggtcctgacaggagattccgtctacgtggcggcgcgtgttgttacccacttcgatcagcaacgtgttatcggcaggatgatgcgagaacgcgacgacggtgttgctggaggtctggcggcagcagtacacgtcgagcgtcatgagggccatgtcgccttggtggtacacggcgtacgcccaaccctggaacacgagcggacatcgcggaccgtgagcggacatcgcgccggcggttgttaccgtcgtctcggcaggagaacacaataaactcctgatcctcatacacaggagtccaagcgtcagaattaaagtccgcggagccataaccgcgcaagtgaagccgatacgagtgttgctgaatttgttcattctgccgactgttgctcacgagcgttcggaggcggtgccacaggctgttggccattaaaaagtcctggcccgaatgacgacgagacagagcccgaggcgaagaaaaaggcgcccgtcatgaagacgtaggcaggggaattcccatatttttatggcttcttttaaaagtctgtatccgactccatccggcgcttttcccaaaccgtggtctcctcgtcgtccgactcggtacccaggaggtggtaagtcttttgccgcacgtagaaagctttcaacgtggagcaaaaaatgagaataaagaccccgaaaacgaaacaaaccacgccgatcatgccgatgcagacgttcatgtcgacgtagccggcggtgctgttggcggtgcggcaaaagagtgtcatgtcgtgcgtgcacaaaaaacaacacacaccacaggccaggtcgtagcgtagttattattccgtagcagcaatgatggtacagtcaagcacatgctctatttcccgttaccccgatgatgatgatgatgttgtccccgttgcagtggaattgtcccggttaatcaccacggtgaacaccacggccaagaaaatgatccctaatatagcgaccactaagagagcaaaagtccatttccagccgttgtcaaagtacgcccccgtggtgggatgcatggtggcgggcatttccatcatatccatgtcgaacgtgtgtcgcggcgacggcgaactaaccaggcagtacgggggtcgatagggcggtgggctgcagtcgggtggtggcggcggtggcgtggaaaccgtcgtcgggcacagacccatggcctgctcgtaggtggggggcgcgtcgtcgtgatcccggtcgcggagcatcggcgtgggctccatgtcggtggcagtgacggcgacggtggtaactgtggtggagacggtaccgacggcgtccgcggctcaccttcgagcaaagagccccttctttttgcgcaaacgacggcaaaacagttctctgggacagccggtggcgcggtaagcgggtgccacgctttcagggtgggtaaaacagtcgcgggcgaagcagtagttgttgcagaaccgcaaaaacccgacgcgaaagaagcccaggagtccgcgcgccagaaagtgcgcctgccgcgtctcgggatgcacgccgaagacggcgccgctctcgttcaccagtatggagatgtccaggcgctgctgcgactccaccggcacggcccgcaccacaaatacctgcagcacgttcagcgagcacgtctcttttaaccagttgccgtgggccggatcctcgtaagtctggctcccgttcaagacgaccgtcgtcagcgcctcattaccgtctcgccagctgaagatggaaccctcgcgcttcatgcacaggcgccacagggccagcaggtcgcgcgccaacatgaactcgcgacccacgtcgccgccggtctcgaagcggacatagcccagttcttcgcgcagcggcgcgtagttgcgcaggccctcctgcacgaagccgcggaaaccggaccgcgacaccaggtacagcgattccaccacgggcgagtagacgtagacgcggccgccctcgccgatgagtacgggtagcggtgggcggccgatggcttcgcaacgactcacagtgcccaccggcagcaggaacttgtcgcagcacaggaaggtcttctccaaacctttaatattgagatgtccaaagtagccgacgcgtaacaggtcgcagtaggtgaaaaaccaaccgttcggccagctgagacgcagcaccgtgccgctgacgcgacgaaccagcttctgcaggtccttgcgggcgtcggcggtgacagagcagcggaaggtctcgttgaccagctcgacagccagcgcgtcctccagcgtacgttccttcatctcgtcgttgatgctctggcggcgccgccggatttcgtcgaaacgagccgcggaggcggcgaccgacgcggaggtcgtccgaacgccctctgtgacgctgtcgtccggccagtcaagaaagctaaggctggcgctgcgccgcctaaagtgtccgatccgcgcgggacgtcgctgagggacggtggctggtctgctggggcgggtacggccgcgggtgtccgcggacacgttagttatacacggaattgagtcacgtggcacgttgccagctgaaaccgccgtcgtctccgccggcgttttctccatcacgggaccgcgccgtgcgcgcgttcccaggcacgcggcccacgctctacccgcacttttgcttcttggtgttagggacgaactcgaacgttacagaatcctcgctgtcgctctcctctttcgcgtcgttaaagtaattgccggagttgcgatccaaaccgccgcctcctcctcctccgccgccgcccgatccacctttggacgtcaggtagctggtgatcttgtgctgctcgtatttttccttggaggaaagaccgtggtcgtgatcaccgccgccgccaccgctgctcattttccgcgtaccggaaccaccgccaccaccgcggtcgtgcttcttgccgccaccgccgccacctcctcccagaccgccgagacccatgggttcgttcatgagatcgttatccagacccgggccgtcgtcgtgcagaccgccggcattggccagcgaagagaggctgccgccaccaccgccgccgccacgcgacttgccgctgttcccgacgtaatttttatcgaagggatcgccacgctggaaaggttcctcggtgagaaaattctccacggcgaacagaccgttgcgactggccacgtacaacagcgtgtcgtgctccgtaactatacgcaacgtgcacggcagtttggtgacggcgcaattgagcagcgtctggtagaagttcttcagctgcacgttgatacgcatgttttttacgccgtggaaactgacgcggttattggccgtgaattccagctcgctgccgttggtcaggatgaatttgatggccggcggaccggcgtgcaccagaatctgcacggtgcccgtagggcagggcgcttttttaacgttacgcttgacgcgggtatgcggcccgatccacttaagcaggtcggccaccacgccgaaatctagatccacgtgcacggccgaattctcgctttcgcgcacaatgtcttggccgtgcacgcaggccgagctgaactccatattgaaatcgggcgcgcacatggagatcttggccgaaaggtccgagatgtcctgcacgtagaacttggtcaggtccttgctggaagtcaggtacatgaaattaccgagcagcggcgtggaattgttaatggtcttgggctgaaacgacttgtcagtgatgtagagacatgagctgttaaaagtgatttttgacacgcagtgactgcgtaccgtttgcaagataagcgacggcgtgggcaagaaggtaaccgtggtgttctccttgagcgcacggatcacagatcgcagctgctggatagccgtcttgtacggcttcagccgcagcgccagcgtcggcggctccgagaggcgcgtcttgcgatccatcccggacagcgtgcaagtctcgactaaggagcgggcgcgagcgagcgaaagttttatagagagcacacacgacgaccgggaacgctgcgaagacgcccggcgtctaataatacagccgcgccgagccagcgggcccccgactaagaggcacagtacttatatactccgaccttaaagcgccagtggtaccacttgagcatcctggccagaagcacgtcgggcgtcatccccgagtcatagtagaaaaccagggccacgcactggtccacaaacacgctcaggttcacggccgccatttccacgtcgttttggatcgccggcgccgcctggaacagacactgcgtcgccttaccctcctcctggtgctgctccaaccacgcgtaattcaccacgggcacgcgcagcggcctccgcaccacggtggggaagtaacactcacggttgggcgggcacaatgaccacaccgtctcctcctcgaacacggtgccgcgcgaagcccacactgacggcgtcacgccccacagatgcgccacctcgtcgtcgggacccaccgccagaaactgacagttgcgcaatccgaactcgagcatgtcggcgcgcagcgcttcccagcgcgcgctggcgatagagagccgcggcaaccgatacaattcgaaaatgaatttgccctcttgatagatggtgcgttcgaaccactcgcagcgcggcaaacccgacttgcacaaatcgacgctagcgcgcaccgcggcaaagtacatgtgctcaaagatgcgctcgatcaagtcccaagaggcaaagtacgtgaaccctaaccgcatgagcgccgtgtgcaagccggccacgccgatgtgcagcggacgcagtttttccagcgcgctctctacccaccattcggacgctgacattagcgcgtccaggcgcgcgttgccccaaaccaccgcctcggtcaccaactcgcgcagcacgctcaaatcaaagtaacgtcgcgtgttccccaaaaccacgtcgggtagatgcagcttctgctcgtcgctacgcgcaaacacgcagcgagccacgttcaccgtcagccgctgcaccggcatgtcacactcgccaaagtggcacgacgccatatcgggactcaagcacggcggcaggcacacgctgtcggccataatcgagtacttgactacgtgatggacaaagaccaccgaggcacggcccttgagcgcgcacagcaacatctttttcagaaaatcgtccgtgttcacgatcaccttggggcacgattgctcgcagcgcgaatactctttctcgaaagccgactcctgacccaggtccgagagccgccgggagacaggccgcccgaacagcgagtagcgctgctcacgcgcacggtatcgcttcattaacacgctaggcacgttgaaagcgtagcaaacccccgtcaactccgacgtgctttctttgagaataaagttaatcacgcggatagcggccacgtcccacatgtccacaaacacacgtaccacgggtcgatgcacctccttctcgcgtatcaaatcgcagtatccccccaggcaacgaatcacgctgttcacatcggcgttaagtcgcgttacgttcaccgacacagaaacgccgcaactcaaggtgctcatccatttgcacatagccgcccaactggcgtcacgcgaaaaagggtcggccgagatcagaaagtcgtactgcggcacgcgatcgaaacccacggtagacatggtgaaggtggacagcgacagctgcccatcgcgacagcgcttcaacaccgattccaacacctcgccttcgaaacgcgcatccagatggaaacgatagatgcgcgagtgcctactgttctcgatagccgccgtcaacgccacggcgatgcgcaaaaacacgccgcccggactctcgtcctgtccgtgcagttggcgacacaccttatccaaacacaaaatggccgcgtacaagccccagcaaccggccaattccacaaaacgcgccgtctcctcggccagcttgggtagatcctccatgtgacgcagcacaaaacggcgcaccgactcatcgcacagctccgaagcgtaacacagtggcgtgcggctttcacgcgcccagttggctttgaaataaaagcgacccaacagcagatcgcaacgcggcgagtgacgaattagacagggaccgtggcgcatgataagctgaaacagcctgaaactgcccaaaccggcactgtgccgcgacacggtgtccatctcgcgccacagcgcgttcctgtcggacggcagctcccgtgccggctcctgtacgccgcaaaagcgaaacttgccccaatagccgtgacaatgacactttttgcccatcaacatgcgcgtagcctgtatcggcggcgatactttgcagagcgaagccccgaaatcgtcctcctcctcgacactgtccagctccatcctggtcgcgccggtcggattgaaggtgctcaaaccgctactcacgcgtccaccgcgactgggcacggcggaaccgctgtcacgcgtcaacgacagcacagacggcgtgccgtcaggagacggcgactcgggacgccaactgacgacgccgccaccactcgtaaaacccgctacacacgctacgccgctcgacatgttagtattttcagcggatgcttccttgtcacccccgggcagcggcccttcctcgagctcgctgtcatctcccccggtagtatcagcgacggcctctgccgacgattcctccgtctcggtttccgcgccgcggctcggaatcctacctggccggcaccgatgtgcgggcaccgaggacacccgctgttcctcgtccgcgtcagccggagtcataagtttacgaggaaaagaacaaagaaatcaggtagatttcaataaagtgagtctagatggcgccgataactacggtttataaagtctgtgtgcgatgtgtttatttttttcttctgtgtctcctccccgtatgctgtcagcgccgctcagacgaattctcgaaagtctcccaattcgacgctaaagttgtccaaacggacgacggacagtttgagttctttgtgtaccaggaacgaggtgtgaatgtcgtcagccaggcaccagcccagcttttgtatgaccccggtacacagagggatctggcgtgggcgcgtgatgcgacggttgacaaagctacagcgctcgcgggcgaactttccgcgtgcaacgtcgaccagggtctgccagtgtgcgatgctggaggtgagcacgtagatgccgggacgtgtttcgggcccgtcatagtcatagacgatgattaaatacacgtattgcagccgtccccgggtctcttcccacgtcagatacatgtctttcggtatcatcaacgcgaacacctccgttttgagcgtgttgtaaaggtagccgcgcatgacgcaggtgagcaacgaggtgatgcccagcgagacggtcttgacgcagcccagcgtctcgaggcggcggtgcagcagatgcgggcccagatccagccactgcagcgcggcgcgcgcggccgaggccgtgtacacgctttcgagcaggcagcgcgtgctggccgagacgttggaggcgcgaatgcctaacaggtagaggctaatgtagaggtgtcgcggcgagtcgcaacccgtctccatgcggatgagcagcgcgcccggctgcgcctcgaactctaccaggccctcgggcacgaagaaacgcgccgtgagcgcctggtgatcggcgtggtagaggtagcgcaccgatatagtatttacctcgcgtttggctttgagcgccgtcactagttcattgtcctcgtcggccgggtcgcgcggccgtttggccaccgcgcgcgcgtccatgatggcgaggcgcacggtagatttcaaaaagttgatagagcagctgcgggcacgggccacggacaaagcggaggcgttaaataccgtgagccaattggagatcggcgcggtggatgcccaggacgtgaccgcgagcgccgtgcgcgccttcgtgggtgcgttgccgagctcgggctaccactttggcttcgtgcgtcagaacgtggtcttttacctcctaagccacgccacggtacagacggcgcgcgacccgctgtacgccgccgagcagttgcacgaacagctggaccgcttcctgcgacaccagcacgacggcggcggggacgaggaccggttgccgttctaccacaacggggccacactgacggctttccagaagctgttgcagaccctgcgcgagatccagaccgtaatagccgaacagagcggcggcaccgcggcagcggcggacttgatcgccagtaacaacgcgtcgaccgagcgccgcggcaagaagggcggttcgagttccgggggccagcagccgctggtccgccgggtgatcacgcagctggaaacggctgccacggaggcgcggccctacgtcaattgtcgcgccgtggccgaactcctggacctgacctaccagcggctcatctactgggcctgcacgctcatgccctacgtgttgtttcggcgcgacaccgacaccgaactggacacggtgcttctgatgcattttttttacacacactaccgttcggttaacggcgatttggccgtggagtttcaaaactacgtcaagaacagcgtgcggcacatgagctctttcgtcagttccgatatcgacggcgaccagaagcccggtgccgaacacatgcgtgacgtcagctacaagctgttcgtgggtaatctgcaggcgcgtgacgccagcggcctcatgtttcccatcattagcacgcgcatctccaccgtgaacctttacctgtcgcccgaacgtatgtttttccacccgggtctgatctcgcgtctgttgagtgaggaagtttcgccacgcgccaacctagacgcttacgcgcgcgtgtgcgatcgcgtgctggaagaccacttgcatacgccgcgacgcgtgcagcggctactggatctgacgcagatggtaacgcgactggtggaactgggtttcaatcacgatacctgcgcggcctacgcacaaatggcgctgatccagccggccagtcagaagagctcgctctttgtcagcgagattcgcgagaaactcatacagatcatctacaatttttacacgtttttcatgtgcctctatgtgtacagccccacgttcctgttcgaccaccggcggcggttgattttggagcagcatcgatccacgttgatcggctccaaggaggaactacagcacgtctggagcaacgtgatactgaacgtcaatacgcactttgcggttcagtacacggaagaagactttgaggcacatacgaagggtgccacggaggcggagcgcgagtacctgtatcgggacctgcacagcaagtggggcgtgcacctgtttaccttgcgtccgtctcgcggcgcggccggcgcggcctcgcctttgcctccgcttgacggcgtcacacgctccgacatcttacgcgaatgcgcgctcgttaatctgaacgaaggccgcgtcaactacgcctccctgctagccttcagtcatcatcccgagttccccagcatcttcgcgcagttggtggtggtaactgaattttcggagatctttggtatcccgcagggcctgtttcaagccgtgggttcgccgcgtctttttgcgctcattcagctgtgtcgtgtattgttgcccgagcaggtgacgctgtaccagaacctggtctccatctacaacctgaccacctttgtcaagcacatcgacgccgcggtttttaagacggtacgcgattgcgtcttcgacatcgccacgaccctcgagcacctcagcggtgtacccgtcacgcccaatgtggacctgctggccgagctcatggcgcgctccgtagcgcataacctgtacaccaccgtcaacccgctgatcgaggacgtgatgcgcagcagcgccggcagtctgagaaactatctgcgacacacgcgactctgtttcggtctggcgcgtgggcgggcgcgcctctcggaggacggcgtgacggtgtacgtggaggtacagggtcagtacggactgcgcgtacctaccacgcgtttcgtagaacagttgcgcgagctggttcgccgcgatcggctgttggccgagaatctgcgcggcttgaatgagcgcctgctgagtgttcgcgtgcgcgtacgtcagatcagcagcgacacagaggaagtaagccgacacgccaagggtcaccgcacggtggcccagatgagcaaggcgctcaaaaagacggcctccaaaatcaaagtgttggaaacacgcgtgacattggcgctcgagcaggcgcaacgttccaatggcgccgtcgttaccgcggtgcaacgcgcgctagccgtctttgacgtactaagtcgcgagaacttggaacgccgcggcgcacagctctgtctgacggaagcgacgagcctactgcaccgacatcgcgcgctagcgccgatgacctggcccgcgggcacgggcgttgcggcggcggccgaagcggatcgcgccttacgcgagttcttggaggcgccctgggaatcggcgccccaaccgccgcgactccgcatgacgcccgacaccgatcacgaagaatcgacggcaggcgcgacgtccgtaccggaggtcctgggtgcgcgctacgaacccgcacacctggccgcgagcgacctattaaactggtacatcgtccccgtaagccaggcgcagcaggacatcttgtcttcgatcgacccgcccgccggctcgacatcggtgtccctgccgccggcctcgccatgaaagtcacgcaggccagctgccaccagggcgacatcgctcgctttggagcgcgagcgggcaatcaatgcgtctgcaacggcatcatgttcctacacgccttgcacctgggtggaacgagcgccgtcctgcagaccgaggcgctggacgccattatggaagagggcgcgcgtctggacgcgcggctagagcgcgagttgcaaaagaagctgcccgccggcgggcggctgccggtctaccgactgggcgacgaagtgccgcgccgcctggagtcgcggttcggccggaccgtgcacgcgctctcgcggcccttcaacggcaccaccgagacgtgcgacctggacggctacatgtgtccgggcatcttcgactttctgcggtacgcgcacgccaaaccgcggcccacctacgtactcgtcaccgtcaactcgttggcgcgcgccgtggtcttcaccgaggaccacatgttggtctttgatccgcacagctccgcggaatgtcacaacgccgccgtgtatcactgcgagggtctccatcaggtgctgatggtgctcacgggcttcggcgtgcagctgtcgcccgctttctactatgaggccctttttctctacatgctggatgtggcgaccgtgccagaggctgagatcgccgcgcgtttggtctccacctatcgcgaccgcgatatcgacctcaccggcgtcgtccgggaaagcgcggacacggcggcgacaacgaccaccgccgcaccttccttacctccgctgcccgaccccatcgtcgacccgggctgccctcctggcgtggcgcccagcattcccgtctacgatccctcgtcctcacccaaaaaaacacccgagaaacgccgcaaggacctcagcggtagcaaacacggaggcaaaaagaaacccccgtccacgacgtccaaaacactggccaccgcctcctcctcctcctcagcgatagcggcggcctcttcttcgtccgcggtaccaccgtcctacagctgcggcgaaggggccctgccggccctgggccgctaccaacagctggtcgacgaggtagagcaggagttgaaggctctgacgctgccgccgttgcctgccaacaccagcgcctggacgttgcacgcggcgggtaccgaaagcggcgctaacgcggcaacggccacggcgccgtccttcgacgaagctttcctcaccgatcgtctccagcagctcatcatccatgccgtcaatcaacgctcgtgtctgcgtcgcccctgcggcccgcaatcggcggcgcagcaggcggtacgcgcctatctgggcctatccaagaaactggatgcctttctgctcaattggctgcaccacggcctggatctgcggcgcatgcacgactacctgagccacaagaccaccaaaggcacgtactcgacgctggatcgcgcactgctggagaagatgcaagtcgtcttcgatccctacggacgtcagcacggcccggcgctcatcgcctgggtggaggagatgctgcgctacgtggaaagcaagcccactaacgaactgtctcaacgactgcaacgtttcgtaaccaagcgaccgatgcccgttagcgacagcttcgtctgcctgcgacccgtagactttcagcgtctgacgcagatcatcgaacagcgacgtcgggtgttgcaacgtcaacgcgaggaataccacggcgtttacgagcacttggccggcctcatcaccagcatcgacattcacgacctagacgccagcgatctgaaccgacgcgaaattctgaaagcgctgcagccgttggacgacaacgccaagcaggaactctttcgcctgggcaacgccaaaatgctagagttgcagatggacctggaccgtctgagcacgcagctgctgacgcgcgtgcacaatcacatcctcaacggctttttgccggtagaggacctgaagcagatggaacgcgtcgtcgagcaggtactgagactcttttacgacctgcgcgacctgaaactgtgtgacggcagctacgaagagggattcgtcgtcatacgagaacaactgagctacctcatgacgggcactgtgcgcgacaacgtaccgctactgcaagagatcctgcagctgcgacacgcgtaccagcaagccacgcagcaaaacgagggtcgcctcacgcagatccacgacctgcttcatgtcatcgagacgctggtgcgcgacccgggcagccgcggctcggcgctgacactggccttggtacaggagcagctagctcaactggaagcgctaggcggcctgcagctacccgaagtgcagcagcgcctacagaacgcgcaactcgcgctaagccgcctctacgaagaggaagaggaaacgcagcgtttcctcgacggactctcgtacgacgatccgcccaccgaacagaccatcaagcgacacccacaattacgcgagatgttacgtcgcgacgaacagacgcgtctgcgactcatcaacgccgtactgagcatgttccacacattagtgatgcgactggcgcgcgacgagtcgccgcgaccgacgttttttgacgccgtcagtctgttgttgcagcaactgccacccgactcgcatgaacgtgaggatctgcgtgccgccaacgccacgtacgcgcagatggtcaagaaactggagcagatcgagaaagccggtaccggcgcatccgaaaaacgcttccaagcgttacgggaattggtttactttttccgtaaccatgaatatttctttcaacatatggtcggacgactgggcgtcggacctcaggtaacggaactctacgagcgatatcaacacgagatggaagaacagcacctggaacggctagaacgtgaatggcaagaagaggccggcaagctcacggtaacttctgtggaggacgtgcagcgtgtcttggcccgggcaccgagccatcgtgtcatgcatcaaatgcaacaaacgttaaccaccaagatgcaagactttttagacaaggagaaacgtaaacaggaagaacagcaacggcagctactggacggctaccaaaaaaaggtgcagcaggatttgcaacgcgtggtggacgccattaagggcgagatgctctccaccatcccgcaccaaccactggaggccacactcgagctgctcttgggcctagatcaacgcgcccaaccgttactggacaagttcaaccaggacttgctgtcggcgctacagcagctgagcaaaaaactagacgggcgaatcaacgagtgtctgcacggcgtgctgacgggtgatgtagagcgacgctgtcacccgcaccgagaagcggctatgcaaacccaagcctcgctaaaccacttggaccaaattttgggtccacaactcctgatccatgagacgcagcaggccctgcaacacgccgtccatcaagcgcagttcatcgagaagtgtcaacagggcgatccaactacagccatcacgggcagcgagttcgagggcgactttgcacgctaccgcagcagtcaacagaagatggagggacaattacaagagactagacaacagatgaccgaaactagcgagcggctggatcgctcgctgcgccaggatcccgggaacagctccgtcacgcgtgtacccgaaaaacccttcaagggtcaggagctggcgggtcgaatcacgccgccacccgccgacttccagcggcccgtcttcaaaacgctgctagatcagcaggccgacgcggcccggaaagcgctcagcgacgaggccgatctgctgaatcagaaagtacagacgcagttgcgacaacgcgacgagcagctgagcacggcgcagaacctgtggactgatctggtcacgcgccacaaaatgagcggcggactggacgtgaccacccccgacgccaaggcgctgatggaaaagccgctggagacacttcgcgagctgttgggcaaagccacgcaacaactgccgtacctgtcggcggagcgcacggtgcgctggatgctggcctttctggaggaagcccttgcgcaaatcaccgcggaccctacgcacccgcatcacggaagcaggacccactaccggaacctacaacagcaagccgtcgagagcgccgtgacgctagcgcatcaaatcgaacaaaacgcggcctgtgaaaattttattgcacagcatcaagagacgactgccaacggcgcgtccacgccgcgggtcgacatggtccaggcggtggaagcggtctggcagcgactggaacccggacgcgtagccggcggcgccgcgcgtcatcaaaaagtgcaggaactgttgcagcgcttgggtcagacgctaggcgacctagaactgcaggaaacgttggcgacggaatactttgcgctgttacacggaatccagaccttcagctacgggctggactttcggtcgcagttggaaaagatccgcgatctgcggacccgttttgcggaactggccaagcgacgcggtacgcgtctctccaacgagggagccctgcccaacccccggaaaccgcaggcgacgacttcgctgggcgcctttacacgcgggttgaacgcgctggaacgacacgtccagctgggtcaccagtatctgctcaacaagctcaacggctcatcgctagtctataggctggaagacattcctagcgtgcttccgccaacgcacgagaccgatcccgcgctgataatgcgcgaccgcctgcgtcgcctatgcttcgcgcgtcaccacgacaccttccttgaagtggtagacgtcttcggcatgcgacaaatcgtcacgcaagccggcgaacccattcacctggtcaccgattacggcaacgtagcctttaagtacttggcgctgcgagacgatggccggcccctggcatggcggcgccgctgtagcggcggaggactcaagaacgtcgtcaccacacgttataaagccatcacggtagccgtggccgtctgtcagacattgcgcactttctggccgcagatctcgcagtacgacctacgaccctacctcacgcagcatcagagccacacgcaccccacggagactcacacgttacataaccttaagctcttttgttatctggtgagcaccgcctggcaccagcgcatcgacacgcagcaggagctgacggccgccgatcgcgtaggaagcggcgagggtggtgacgtaggggaacaaagaccgggccgcggtaccgtgctgcgcctgagtctgcaagagttttgtgtactcatagcagctctgtaccccgagtacatctacaccgtcctcaagtacccggtgcaaatgtcactaccctccctcacagctcacctacatcaggatgtgatacacgcggtagtcaataacacacacaaaatgccccccgaccacctccccgaacaggtcaaggccttctgtatcacccccacccaatggcccgccatgcagctcaataaactgttttgggaaaataaactggtacagcaactgtgccaggtaggcccgcaaaaaagcacaccacccctaggcaagctatggctctacgccatggccacgctggtctttccacaagacatgctgcaatgtctgtggctagaactgaaaccccagtacgccgagacctacgcctcggtgtccgaattggtacagacgttgtttcagattttcacgcaacaatgcgagatggtgaccgaggggtacacgcaaccgcagctccccaccggagagccggtgcttcagatgatccgcgtgcgacaccaggacacaaccaccacagacacaaacacgaccacagagccaggacttttagatgtttttattcaaacagaaaccgccctagactacgcgttgggctcctggcttttcggcatacccgtgtgtctcggcgtgcacgtagccgacctgctgaaaggccaacgtgtactagtagcgcgccacctcgaatacacgtcgcgagaccgcgacttcctccgcatccaacgctcccgggacctcaatctcagtcaactgctccaggacacgtggaccgaaacgccgctggagcactgctggctacaagcccaaatcagacggctacgcgattacctgcgtttccccacccgcttagagtttattcccctagtcatttacaacgcacaggaccacaccgtcgtacgcgtgctgcgaccgccctccacgttcgaacaggaccacagtcggctggtgttggacgaggccttccccaccttcccgctgtatgaccaagatgataactcatccgcggacaacgtcgctgcgtctggcgccgctccaacaccgccggtacctttcaaccgcgtgccagtcaatattcagtttctgcgtgaaaacccgccacccatcgcgcgagttcagcagccgccgcgccgacatcgtcatcgagcggccgcggccgcagacgacgacggacagatagatcacgtacaagacgatacatcaaggacagccgactctgcattagtctctaccgcctttggcgggtccgtctttcaagaaaaccgactgggagaaacaccactatgccgagatgaacttgtggccgtggcgcccggcgccgccagcaccagtttcgcctcgccgcctatcacggtgctcacgcagaacgtcctcagtgctctagaaatactgcggctagtgcgattggacctgcgacaactggcgcaatctgtgcaggacactattcaacacatgcggtttctctatcttttgtaaccgacactgacagtagcgggtaataaaaacaagaggattgttatcgtttttttatgataaaaaaacaacgtgtcattttcacggtgatttattcttgctattatttttccccatgggctgtcagcgtcgggtgcgcgacactgctaccatgcgcaacaggtccagtttaaaggcgcacttgtcgttaaacaggctggacatgcgtgtatatttgctcagcatggtggccagcaccgggtgggtggcctctgagatctcggtcggcaactccaaaacgacgttgacgacgtgacggtgtttttcgtcccgcttgttggccaccgtgggtcccggcgcggtgttagacatggggcaggccgtggggggaggacgaggaggaagtcgctgctaaaccgccacgcgcctgctgcacaatgtggccgccgacgtggcaggcggtctgtttaaccagcgcgcagccccgacacagcggggcgccgtcttcgctttccaaacagctgtcgcggtactcgcccgtctgacagcgcgcgcacagcaggccgtgcccgtgcgaagtgaggcgcaggagacgcgggaccgtcacgccgcgtaccaccacagtggagtcgcaggtgcgtgccgcgcagggcagaatgacgtcgaaagccagccggtgatcgtacacggcgcaagccgcgttgaggcccagcacggctttccagcccacgcgtacgcagcgctgtccaaagagcgtctcggagacgagctcgtagacgcgctgccgcaccacccgctgactgccgcagagcgagcagtgtacgagctcggcgtgcgtgttgaagatgacgctcttttcttgacggtcccgataatagaacatcgagttgagcggaaaattttgctggcagtgtagcttttccttacccaggttgaggcagtgtccgcactgccgacagaccacggccaccagcgagcgcgcgtccagatggcgctcgcacttgagtcgacacagacaccagagcggcaggtcgatgacgctgccgatgaggccgccgcgcagcgcggcgctgagtgcaaagaggacgatcttggtgggctctacgtgacgcgcctgctgtccggcgcccgcgtgtcctaccgccgcagctgccgccgtcgagcctcctccgcgcgtctcgtcgtgcagacccagtgcccgcaacggcaccaggtatcgcggacacgtgtcgcaaaacgtctgcaccgcttgtcgggccagtacgtagagcgggtttccgcagggtaccttcccagcgtgccggcgcaaggctgcgatgaggccccgcagctgcggcgaccgcggctgccgttggtgacaccactggttacggtggtatacggccaaatcagcgcgggcgtcgaagcgcttggcgcgtagtagtgctaggcacggcgagctggtggggtgaagcacgggcagccgaaggtccaccccgaaaaggaaacggtgaaggtcacctagcagcgaggcggtgacaccgtccaacaacgcgtgcagccgctcgggcgggtagagccgcagacggcgcagcaggtagtcggtgtcgtagcgttcgaaacgcagaaaggccatcgtgcggacggccacggtgtgcagacagtccatgctgtagacgtaagcgagaaacacaaagtagggcttggtcataaccatacgctgaaagagcgccgtcaccgcctcccgctcggcctgccgacacaccagccattcgcgcaggaagcgttggtagagacggtcgcccagctcccgattcagaaagcgcttatccgtcacgaagagatgaaggacgcaagaacgtggcacgtgatgcaccagctgctgctggaggaccgccgacgtctgcgccgcaaactgcgccggtggctgcgacgtttctaccgccgcttcctccggctgcagcgcaccgcggccgatcaccagctgcacatggaaatggtcctcgtgaacgcagaggggcgcgaagagacggcgcagagcctggtggaactcatcagtcgcggtgtgcggagcgtgtcggagacgacgactggccatgaccgcgccacagcagagccagcaccagcagaagagccagcaccagcgggcccagagtcgcaaagcgcgcgggcagccacggcccagactgcggtcgcgatggcccggagcgcgctcgccaccacgatgacggtgcccaacgataaccagtccgctccaaggacggcgcgcacggcggagacggcggatgacggtgatgggtcgacacccctcgccgacgactcacgtgctcctccagaggccgacgcgcggaccctccgacgtcctggcccgccgctgccgccgccgccttcccttctcccgccagagccagcaactcctcctcctcttcatcagcgtctccctcgcttgcgcatccgcatcgtcccatacaggcctcacaacgacacagccgccacgaccccgccgccatgggtggcggcggcggccgaggcccggcagcggcgccgccagcggcgaccatggtgggagagcaactcggatgacgaggaggaggaggaggagggggagatgcggtccgagaggaccgctttcccgccgttcgcgtgagcgcggccgacatgcgggcgcgccacagggacggaccgctgccgctgtgactgcttacggtgacgtggttccggaccgccaacgacgtcgacgcggctttcttggcgtacagctcgcgcagcagattctcgtactcgccctcgttttcgggtccgaaggcgatgagctcgatgttgaagaccgacgccgaattggatttgcgcaccacgcacttcgtcagcactccgtaggccgagggcttgatctcctcgatgtccttgagcgtgacgatgagcgactcgttcaccttaagcacattgaactcacctacgtggcgcgccggcgagacgagcttgacgggcgctcgcacaaaacagcagagggagacggcgcagccagtgtttttaaagataaaacaaggcacgtggtctgtgcggctctcccagtagctgagcagatactcgacacaatagaccgtgtctgtcttgagcatggcgtcgcacaccgagtaattgggatttttacagataaggccggcgtcggtgacgcgcagctcgctgggacccaacttgaggatacgccgcgtggcctgcaccagatcctgatggagaaccttgttcatctccatcgcaccgacgccaccgccgatttatttacccggcgccggctcgtcttttccctccaggattccgttaatgtccatgagcttgctgacgatcgccgttaatagttgcgtcttctcacggaggatctctccgtgactgcaggtcgcgcagtcgccgtgcacgtacttgaggaaggcggcgtacttctgacccgcgttcacgaaatttaagcgcgcgtccagggagggcagcaacagatcgtagacgcgcggcagcatcggctcgaactgtaatagcagatcgtcgtcaagatcgggtagcgcgtgcccgtcttcaccgtcctcgtcgtcaccacctcccccctcgagcccaccgctcgtaccagccgcgggctccgcgtcctcgtcgatcaccagcggtcgcgtcggcaccggagaatccacgtcatcctgcacgtcgttttcctcctctccgtcgtcatcgtccagaaacggcacccgctgcttagcccaggacattctttctccgcgtcctcaatcagcggcgccgatcgccatgaatccgagtacccacgtgagcagtaacggcccaacgactcccccccacggggcccacaccacgcttcttcccccgaccagcccggccccgtccaccagctccgtcgccgccgctaccttgtgcagtccgcaacgacaggccgtttcgcgttacagcggctggagcaccgagtacacccagtggcactcggacttgacaactgagctgctatggcacgcgcacccgcgtcaagtacctatggacgaagcgctggccgccgcggcggccgcctcataccaggtgaatcctcaacaccccgccaaccgttaccgtcattacgaattccagacgctcagcctcggcacctcgggggtagacgaactgctcaactgctgtgcggaagaaaccacgtgcggcggcacgcaatccaccgtactcaccaatgcgaccaacaccaccaactgcggcggagccgtcgccagcagtagcaacgcaggacctgccggcgcttcggccgcctgcgacctagatgcggaactggccggcctcgaaacctcggcggccgactttgaacagctgcggcgactgtgcgcgccgctggccatcgacacgcgctgtaacctatgcgccatcatcagcatctgcctcaaacaggactgcgaccaaagctggctcctcgagtacagcttactgtgcttcaagtgcagctacgcaccccgtgcggcgctcagcacgctcatcatcatgtccgagtttacgcatctgctgcagcagcacttttccgacctgcgcatcgacgacctgttccgacaccacgttctcacggtcttcgatttccacctgcactttttcataaatcgttgctttgaaaaacaagtgggcgacgcggttgataacgagaatgtcaccctgaaccatctggccgtggtgcgggccatggtcatgggcgaagacacggtgccttacaacaagcctcggcgccacccgcaacagaagcaaaaaaacaacccttatcacgtcgaagtgccgcaagaactgatcgacaactttctagaacacagctcacccagccgcgaccgcttcgtgcagcttcttttctatatgtgggccggcaccggcgtcatgagcaccacgccactcacggaactcacgcacactaagttcgcgaggctagacgcgttatccacggcctcggaaagagaagacgcaaggatgacgatggaagaagaggaggatgaagaaggggaagaaaaaggaggagacgatccgggccgtcacaacggcagtggcaccagcggggggttcagcgagagcacgctaaagaagaacgtgggtcccatttacctatgtcccgtacccgccttttttaccaaaaaccaaaccagtaccgtgtgtctgctgtgcgaactcatggcctgctcctattacgataacgtcgtcctgcgcgagctgtaccgccgcgtcgtctcgtactgtcagaacaatgtgaagatggtggaccgcattcaactggtattggccgatctgttgcgcgaatgcacgtcgccgctcggcgcggcgcacgaggacgtggcgcgctgtggactcgaagcacccacctcgcccggaggcgactcggactatcacggcctgagcggcgtcgacggcgcactggcgcgacccgacccggtattttgccacgtcctgcgtcaggcgggcgttacgggcatctacaagcactttttctgcgacccgcagtgcgccggcaacatccgcgtcaccaacgaggccgtgctcttcggacgcctgcacccccaccacgtccaggaggtgaaactggccatctgccacgacaattactatataagtcgacttccgcgacgtgtgtggctctgcatcacactcttcaaggcctttcagattacaaaacgcacctacaaaggcaaagtgcacctggcggactttatgcgcgatttcacgcagctgttggagagttgcgacatcaagctggtggaccccacgtacgtgatagacaagtatgtctagcgtgagcggcgtgcgcacgccgcgcgaacgacgctcggccttgcgctccctgctccgcaagcgccgccaacgcgagctggccagcaaagtggcgtcaacggtgaacggcgctacgtcggccaacaaccacggcgaatcgccgtcaccggccgacgcgcgcccgcgcctcacgctgcacgacctgcacgacatcttccgcgagcaccccgaactggagctcaagtatctcaacatgatgaagatggccattacgggcaaagagtccatctgcttacccttcaatttccactcgcatcggcagcacacctgcctcgacatctcgccgtacggcaacgagcaggtctcgcgcatcgcctgcacctcgtgcgaggacaaccgcatcctgcccaccgcctccgacgccatggtggccttcatcaatcagacgtccaacatcatgaaaaatagaaacttttattacgggttctgtaagagcagcgagctactcaagctctccaccaaccagccgcccatcttccaaatttattacctgctgcacgccgctaaccacgacatcgtgccctttatgcacgccgaggacggccggttgcacatgcacgtcatcttcgaaaactccgacgtgcacatcccctgcgactgcatcacgcagatgctcacggcggcgcgcgaagactacagcgtcacgctcaacatcgtgcgcgaccacgtcgttatcagcgtgctgtgtcacgccgtctcggccagcagcgtcaagatcgacgtgactattttgcaacgcaagattgacgagatggacattcccaacgacgtgagcgagtcctttgagcgctacaaagagctcattcaggagctgtgtcagtccagcggcaacaacctatacgaggaggccacgtcatcctacgcgatacggtctcccctaaccgcgtcgccgttgcacgtagtttccaccaacggctgcggcccctcctcctcctcgtcccagtccacgccgcctcatctccacccgccgtcgcaggcgacgcagccccaccactactctcaccaccagtctcagtctcagcagcatcatcaccgtccccagtcaccaccgccgccgctgtttctcaacagcattcgtgcgccttgacactgtacggcagaaaagccggctccaagtgcaagcgccgcggcagcaccatgtgcaaaaacttgtccttgcgcgcggtttcgccgccgggaaagacgggcgacagcacgttggttacagccttgagaacctgctcaaagtacttgtcggtgtgaatgggcacgccgtgctcgcgcacgtagctcggatcttcggctacctcgtagttgcacacggccgacggtggtttccgcgccctcttctttgccggctctcctcctctcctgttgctctcctctaccccgccgccgtcagcgtcgtcgtccgtgccatcaatcgcgtccgaccgggaaaccacgccggcggttacagaatcaccgttgtcggaggaaccctgcggcgccgtccggacaccgggcgccgtcaggacgtaaaagacccgatccccgaccgagggtagctcctcagaacgggccgccagtcgcttaatgacggcaatgtgcggcaggttagattgacggtacaacgagatgtccttagaaagcaccgacgaaagcaccaggtcctcgacacgcacacggtgcaggtacagatcgtcgcgggcctgcaccaggcggcgcaagatacgccagaaaccgcgtggcacgccgtatttcttgacttcatcgagtgagaggcgcgacaggcgcacggctgcttccgagacctcgcgatcctcaaagagcagcgagaggacgtcacgcgtgacgcccttgacgaactcgcaggccgtcttgcgcaccagatccacgcccttcatgctcagacccgaggcgccctccactttgccgatgtaacgtttcttgcagatcatcataagagagacgaagaccttttcaaactccagcttgacgggctccacaaaaagacaggccgtcacgtagtgcgccaggctgggcccacgcgccaccagagcctgcggcgtcaggccacgaaagcggacaaacacgctgtccgtgtccccgtagatgacccgcgcctccacccgccgttcgtccgagccccctgacgatgtttcgagcccctccggtaacgtgctgctctcctccgaatccccctctcgcgttctcactacatagtcttcctgattaaaaaaattgtgcaaaaaacacggctctgaaaaattgtctttgatgaaccgcgccgtgcgctctagcatgtcgcgaccgatgcgcgtgatgctggcggcgatgggcagacacggcatcatgccgttgaccacgccggtaaaaccgtagaaagcgttacacgttactttgagtgccatctgttccttatcgagcagcatacggcgcacggggtcttgacactcgcgcatgcattcgcgcacggcacggcgctgcgaaacccacttgttgagcagttccgaaagcaccgagacgcgcaccgaagcacgcacaaagcggtgagtcacgccgttctctagcgtgacgctgtatacgtcggcggggtccacggggtactcgccacccggcaccagcagggtggagtagcagaggttgtgagccatgatgatggaagggtagaggctggcaaagtcgaacacggccacggggtcgttgtaataacccacctcgggctcaaacaccgtggcaccctggtacgaaaccgccgcagtaccgccggcgccgtgactgtcgttggaaacgccgacgctgccactactgccggagccgacgctgaaaacgccgacgctgctactactgttactgccagagccgggtaaaacgccgtcctgactcgacggcgcagattgcaagggcggcgacatctgaaacatggccgccacagaacccgcgtcgccgggcacggcagcggtagagatgatagcggcgttaggtgacacggcaacgctattcgtttcgggcaccgtcgtacctttgctgtagtggttgggcaggataaaatcgcggcaggcgcactcgtccagcagcgaggtgtagatacggatctgctgtccgtcaaagatgacacgccgcaacggaattttagccagccgcgcgatggccccggcctcgtagtgaaaattaatggtgttgaacagatcgcgcaccaatacggcgtcctgcagacagtaacggcctacctgggcgcggccctcggcattagccacgaaacaacgcgggatgtccttgtaggacaggtcatccttgcgttgccgcaggtaaagctcggccatagtgttgagcttatagttgggcgagttagtcttggccatgcatacggggtacatgtcgataaccaccgaacccgcaatatacaccttggtggcggccgtgctggccggattgttgtgagaagccgagggaaaggcggcggcgtactgccgcttaaaacccacggcggggctgtgtaaaaagaaacggccgccctgcgccgtgggcaacttgcagaagcgctgcgagtccaccttatacaggtactcgaggcgcgtgaggatgtacttcaagtcaaaagagttgatgttgtaaccggtcacaaaggccggcgcgtaccgttgaaagaaaagcataaagcccagcagcagctcgtattcggaagggaactcgtagacgtccacgtctgggcccacctgcccgcaggtgccgatcgtaaagagatgaagacccgagtgcccaaagatcacaccctccgaagtgcagccccgaccatcgttcccgtttgggatcccctgatccacggcggtgtttccccccgtctcgtagcacacgcacgagatctgaatgacaatgtcatcggacttctcggcgcagggaaaaccaccctcgccgctcatgcactcgatatcgaaggacaggcatcgatagcgcggccacgagctgtcgtcgggcacggccaccaggtcagagacatcgcagtcgacctcgatatcacaagtcgacgcgcgaccctgctgccgccagtcgtaacgattcacggagcaccagccgaacgtggtgatccgccgatcgatgaccaaacgcgtcagcggatccacacggacctcgtacacgggaaaaccctgctccagcagatactcgccgatttttctggccatggtccagttgctgatagacacacactgcaaatcgggcacgggtcgcgtcccgtacccgtagatggaggtcttggtggccggcgtgacagacacggcgtatggcgtccgcggctcgggcactagttcgcccacgctggcaatgacctcacgcagcctatcggtgtcgctgtactcacagtaaaagtagctgcgctgcccgaaaacgttgacgcagatactgtagccgtgttctgtggccccgaagaaacgcaacacgttccccgaaggcaccagatgctgacgatagcgcggcgacacgttttcgggcgagtcgaagaagagcacggcgtccgtctgatcgtaggtgtgaaaacgaataggtcccaccacgcgacccaccagggtctcgcgccaaggacacggccaaaccatgtcatgactcaacaaatgtttaatctctcgatagaacatgagaggcagccgtcccgtcttatgcttgatcaaccccgtctgaccgtcgaacatgacgcctcgcggcacgatctgcaaaaactgtttctgtggcggccgcttgcccgagccctgcgcggagccgggctgcgaacgctgacgccggccacccgcgaccgcaccgccggtcacgccgccgctcagatacgggttgaaaaacatagcggaccgtgagaggctgacagcttacgaagcacaatcacaaagaaaatacacatgcagcacctagatatccagtttgaccccgtatatcacaagtctctgtgtcactttttttgtctgttttttttttcttctcctggttcagacgttctcttcttcgtcagagtctttcaagtgtcggtagccgtttttgcgatgtcgcagtcggtctagcaggttgggcttctgtcccttgtcctgcgtgccagtctgtccgtccaaagaatctgtaccgttctgctgcgctcgctgctctgcgtccagacggaccagggccagaagcatctggtaagcctgctcgttggtgtaaggcggagccgccgtggatgcatcagacgacggtggtcccgatcctttgcgaccagaattataaacactttcctcgtaggaaggcggagcctgtaacgacgtgtctttggtgttgcccgacgtcacggtggtcccgttggcggacaccagatagggaaagaggttctgcagcggctgcatgcagagacgccgctgtcgagtatagatcaaataagtgataatgactacggctatggccacgaggatgatggtgaaggctccgaaggggtttttgaggaaggtggcaacgccttcgaccacggaggccaccgcgccacccacggccccaatggctacgccaacggcctttcccgcggcgcccaggccgctcatgaggtcgtccagacccttgaggtagggcggtagcgggtcgactaccttgtcctccacgtactttacccgctgcttgtacgagttgaattcgcgcatgatctcttcgaggtcaaaaacgttgctggaacgcagctctttctgcgagtaaagttccagtaccctgaagtcggtattttccagcgggtcgatatccagggcgatcatgctgtcgacggtggagatactgctgaggtcaatcatgcgtttgaagaggtagtccacgtactcgtaggccgagttcccggcgatgaagatcttgagactgggaagctgacattcctcagtgcggtggttgcccaacaggatttcgttgtcctcgcccagttgaccgtactgcacgtacgagctgttggcgaaattaaagatgaccacgggtcgtgagtagcagcgtcctggcgaatccttcacgttcatatcacgcagcaccttgacgctggtttggttgatggtcacgcagctggccaggcccaagacatcacccatgaaacgcgcggcaatcggtttgttgtagatggccgagagaatggctgacgggttgatcttgctgagttccttgaagacctctaggctgcgccgttgatccacacaccaggcttctgcgatttgcgccagcgcccggttgatgtaaccgcgcaatgtgtcataggtgaactgcagctgggcgtagaccagattgtgcaccgattccatgctggataaatgagttgcattgttgccatctgcacttcttttggttctactatgagtaagattcagactggagcggttggccaaacgttcgagttccaccagagatttttgcttgataccttgccagaacaccaccaaaccaccagtggtttcaaacacggacacgtttccatatttttcatatgtttgattgtatgaagtattgaaaatctgctgtaacttatttatggcctcatcacgtacgcagtccagcgcagagtcggacatgttcacctcttgcttcttagataagaaagtggcggtcattttggcagaagaaaagtgatacgagtcctcggcttcggaacgaatggtgcgttccgaggcttcccagaaagtgagttgacaagtaacattcttctcgtcctgtatatcccaggagatcactgagtccgcacgttcaagaaaagccaccaacctgtgggtctctaacgcagaattcggtcttccaaagtcggagacgatagtgtagttcggaaaaatgaaaaacttgtcggcgttttctccaaaatagctggcattgcgattagttccgttgtagaaaggagaaatgtcaaccacatcacccgtggaagttgcgaaaaaatgatagggatacttggagcgcgcagtagtgatggtcaccatacaattcagattacaggtctcacgatagagccaggtgctgccgcggctgtgccattgatccttgaccgtcacgtaacgggtactgtgggtgttggaataatcgtcgggcattaattgcatggttttgttttcatagctgtccctatgataagccacgaaaaccgtgcctgctataacgcggctgtaggaactgtagcactgactgtggctgttgatatgatgaatctcccacataggaggcgccacgtattccgtgttgctgcccagcagataagtggtgtggatgtaagcgtagctacgacgaaacgtcaaaaccttctggtagactcgtaccttaaaggtgtgcgcgacgatgttgcgtttgtagaccaccatgatgccctcgtccaggtcttcattgataggcttcatcgaggtgcagacgatattacgttcaaagcgaataagatccgtaccctgtgccatagaacacacgcgataggggtacttggtggtattgacccccaccacatctccgtacttgagggtagtgttgtagatggtctcgttaacaccatggctgaccgtttgggaagaagttacgcgttgagagactgaaccggatcgagagtgagcagcagacgtcgtatgagaggaatggtgactgtgagtagcagaagttccacgagaagtagaagatgaggaaaccgcagcacccagacagacgatacacaagttaacgcagactaccaggcaccagatcctggattccatgttcgtcgcgggccaaatccagcagcgatgaggcgcgtcgtggtctcttgcgtgttgcgcggaccctccgggaaacgcccgcggtcgaggaggaggggtacggacttggcagccaaggtcggtccggctccctgaaggcacccgagacggccgcggcggccgttagggtggagggcttggccacgggagctgttggcacgtcgccactctcatccggtctggacagatgcctgtagaggaggagatatagatctttggacttataaagacttccttcgtgacgaagcagcagcggccactctttgttatacgtgagaatcacatctctgtccgggtgcagttcgtcgcgcaggcacgcgatcgagagttgtttcccgaaagtttcattatatagtgcgacggagagcacgagctcccgcacgtgcatccacatctccttctgcagcacgtttaggtcctgacagtccgaaaaattgaaaaaacccatgtacttcaccaccatccactcactgggatacacggtaccttccgcgcatttgaccaaatcgtccttgacgtggggtagtacgcccgcgttgtcgcaggcataggccatgtccacattgtgagagaggggatagcgatcggtacagtgtgtgaagaggggcccgttacacaactcgtagatctgctgacccagtagcgggagggattccacaggcagactcttgtggatcaggttattgaccacatacaggtgctcatcgtacgtgaactgatcccccacgtccaccacgtcttggtcctggtggtattggctgcggtatagaaacccattcatgagcttagagataaagtccagacacaagggccccactaggttgacatcgatgagtttgctagtcagacgctcctgcgttttgatgcaacggatcaccttgccatagcccacctctgagaccttctgcaggtaggcgcgtttgcgcacgttcacctcgcgggtgacgttgtggatgcgggaacgcgcgtccaccaagtcgagagcctcgtgttcgtcgcagttgcgcacccgtaagccgttctcgccgccgtcgccgtcctgcccattcgcccctccccctaccgctttcttgcctcctccacgggcccggccgccgccaccgttattcctctgactgtgagtactgctgttgctgctgttgctggccgtcatcaaagtcgtacccgtccccgacatcgcctcccgtccacgcaggtgaatagcctcgccctcggggccgtcgccccccgtgccatcgggcagcggacgtcgaatctcctcgagaatatgcttgattttggtgtacatctcgttgctttcgtggagcttgttgaacaccgggttgtcctcgaaagcttgaatgctgagggatgtgatgaggtcgatgatcctgttgggggcggcaaagaccgaccccacgaacatgcgctcctccccgtccaacgccttttccccgagcacgaagatgtcctccacgtcctccccgtacagatggcgactgatgccgttcatgagcgcccggcacagctggtgatacacatttagctgctggatggtgatgcccacccgcttgacgataacctccgaggtacgggaccagtaggtaaaatccgacaaggaatatattcgttccggtatatccgtaaacaggttgtactccctcagcgcctcctccgcctcctggatgtagctgtggtaggccgatgaagaagagaataggcttttgagggccgaaaggactccagccaagtgggggatgcgcgttgtcaggtccagcaggtcctgctccaccgtctggatattcacatcggactggcttgacggacggtggaccgctatatggttgcacagcaagccctgcagccgcttgttcagcgagcggccctgattcgggatgatggtcagctcctcgtagcattgggcgcatgtcgtcccttcgacgtacacttcctgacgcgccaccggcgagatgccgcataggcgacggaggagctccagcagctgcgcgcagacctccaggccggcctccggcgccaggatcccgtacacgtagttcattttgcacaggaagcgctcgatgtcgttgagtgtggccagactgacgctgaaacggacgttgtccgtaaactggagctccacggtgtgatggcgatcgcagcgatccaaacggaggacggtacggtagaaggccgcccggtccggctggcgcgagtaggccatcagcgcccgatccagcaaagccgtatcctcgtgcagcgccttcagcagcatctccagatagagcgtcagcagcgaactctgcgtacgattctgcgccaccacctccgggtagatcttccggtacagatacactatagccgccgcgtttctcttgaacggcgtggactccgccagtaacacgttcggatcgcagtactttagacactccagctccatggcgtattcgttgcatttcgaacacactacgcatagtttctgtaacaaattcatctccatgactcgactcgctcacgtacgagacgctgtcgtccggtctggcgccggccagagacatggagtcggtgcacaaataactcgcgggccgctcgctatgccgactgacgttgacgttaatatataacgacgtcgtcgacgacgcgggttctgctcccgaagctgttgccgccgcttgcggcgcaacctcctccaccaccgccgccgccggctcctccgcctcgggcgacgggggctcggagatgaccggctgtgtctgacactcctccccttcctcaggcggcccgggcgccgacgcgaatgtcggagtttgccagcgcggcggcggtctctgtctctggtgccgcggcgctaaccttcggggctgttgctgctgttgatgatgcgacgccgtctgtcgccgctgttgcggcggtagctgatacggtgtcgcctggtgctgctgtgtcggtggctgctgttgctgctgttgttgcggtctgaaaagcggccacgggggctgcgactgttgctgctgttgttgcgatgctcgtggctgcggcggccgttgtcgcggcgtttgctggcggttacaaccggctgcgtttggccggcaataacccgctgcccccgccgcccccgctgctcccgccgacgccgccagcctcgtcttcgccggcgttcacgagaaagcagccacctcccgtctcgccgggcacgccgaagcaaatggagttgcccgcgacggactcgccgagaagaagaccgccacccccgacgccggacgccgcgccgacgccactgggcgcgaagagcgccgacaggtcgtgcacctcccccccggcggcgtccgttaatcgctgggcgtcggcgtccagcacgcgtcgcaagttctccagcgaaaagtcctccacgccctgctcctgcaacgcggcaaacttgtccatcagcgacgcggccagcgcctcgcagccatccacgaagaagagcacatcgtcggacgcggggatctcctcgcgcacgctcagaatctcgtacacggccatcacttcggggtcgcaatccaagttctcggcgtccagcgccagcatgacgcggttttttataagatccgcgtcaaaaagcacgttctcgcggcgcgagcgtttgatgagcacgtcggccagacgcgtagccaagaggtagcgctggcgcatgaaacgataatcttggccgctcatagagctcacgttaaggctgcgttccacaccgttgcccgaaaagtagccgatctgcccaaactgatagatctccttgctgttgttgatacccgcatacttttccacgctcacgggcacggtcaccaaggaacgatgctcaaaaacgctccgtaccaacgattcacgcgccacagtggcggccatgggcgccggcacgcctgcggtcttcaagcccttgacatgcaacgcaaattcggcgggcgacgagaaacgcggactagcacctaacacgtgaggaaactgcgcgtggttctgcgtcgttaagcgcgtcgtcaacccgtgcagcgagccaatgtagtctttgaagccgtagtagcagaggaatttgttatggaaacggctttccacgtaactcagcacacagtctggcgccacatccagcagatcgtgctcctgatagtcagccgtcacagccaccagaaatttgacgaaagcattgaactcgcccatgtcacctatgggcacattcttgggcaacgcgttggaacagaccttctgccaaaactgtaagcaggggagaccacattcaggaaagagtcgctcgtgatgtcgatacagcagaaatcccaagcagcccttagccggattacgacgcggaacgtgatcgcggcgaaaaaacacgctacccgcgttgcccttgcccgcgcggtagatgggtcggtttttcactcgcaccatgatcaacgtgggtaccgacagccgcgagagcttgatctccatgggcaccacggcgtacgtgccctgcgcgtacagcctaaagtccagcaggcggtcgtgatccgaattcttggacgacttgatctgcttggtgaagagaaagcccttgcgcgacgacgtggtggagaacgcgccgtgaatggattgaaaatgctgcgtcatccatttggataccaagttggtggtcaacggattgtccacaatgtatgaggtagcggtaataagcgccacgttctggatcacgtaaaagacggatctgaaataggcgtaggccagcagcggctggaaggccacggcgtagggattcagatccaggttgaaggcctgcgtggcgcccgccacctcgtcgcggctgctcttgaggcgcacctccgaaacgaaacccagggcctcgtcgtccacaaacttgttgagcgccgaaaagacggccacaaagtcgcttttgccgtgcgcgctaaaggtatcctcgcccgtcacggggtcgatgagccgcatcttgcggcagtaatccaagatgcgattgagccgataggtacggtccacgctagcgcccagcatgcgaccgccgcgccccatcattcccccggaatccccgccacccccaccaccacgaccgccgcccagaccgtcgctcgggcccccgctcacgtcccgtccaccacccccgccagcaccgccgcccggaaccccgtcgtcacctttgccgtccaaacccccgtccttggcgtcgacgttgtaacgccgaccgaagctgcccaaaatatccacgtcgttgagaaaacgcgactgcacggtgatcacgcagggctccttcttgggctgcttgggcaccacgggcaagcgggtgcgcacccgcacgaaggccgtctgataacacgtgtggcaacaagtacccccacaggcctcgcacagccccgcggcgcagcccaccaggtgattcgtgagcgtcgacgaacccgacaagcccgtgttatacaccgagacacgatttagataccagacgaagcccgaaactagctgcggacacgtgccacacaccaacgccaaatgctgcggcccatagcgttcgtccttgagcggcgcgccttgaaatttgagcaccttgcgcgcgtcgttgtagacgtcttcgcaggccgccgacaacccgttggtgaactgaatagccttgagcaacgtctcctgactggccgtaccgccggcgctgggatgccgcgccgacgactggagatacaccagcctgtgctggtagagcaccgaattagcgctgaagaccaaggcggccacgtgcgtcgagagatgcaacttgagctcggtcagcgcgcggatcagatcgcggtgatcggttgcgttggtcactaaaggccactcggaaaagagcatagactcggcaggttggtaggccgaatcgaaaaataccgaggcaaaactgaaggccaactcgcaaaccaccgcgtcactcagcatcagatgatccttttccagactgctgagtcgctggctcatgtaccccaagtagcgcttatgtggcgccagcttcaccgactgctgactgtcgtgcacaaactgccgcaacgccgcctcgatcagcacacgcggctccgagaagcgcagcgattgacaccatgacgtgtacacgtagtagaaaagcgtctcgcttacggccggcacgtagagccctcgcgcctccacaaaagcgctgcgcgcatccagcgagacctcgtcggcttcggcgtcaagctgcagcgaattaaagagcgtaggcgggtacaacggcacgcgcaccgcctcgccgccgtacagtcgcaccgtggtcgcctcctccacgcatggaatcagctgaccggcaaagagaaactccttcaagccgttgcccaccaccacgtgcacagtcgtctcggacgcctgacagcccaccgccgcgcacaacgccgacagatcggtaggcacgcgatccgcctcgggcgtgtaggcctccaacgcgtacttctggcgggcgtcctcgcacaaccgatgcacgtctccgtgatcctcggtaaaagccacgatgccttgcgtatgatgaaagtagagcgcaaaaggacagaaggacgtgactttcgtgagcaccccgccgtcgtaacaaagcacaggcgtgcgcacagagacgccgaaatccgcctccaccgtcagccccgccaacagaggagcgatcaccacgctcgaggaacggtcgcatagcgagagagtggccagaatctcctgcgtttctgcgttcaacctgctgaagtagagaaaagccgcgggccccaccggcgctagcgcggttagttcctcgtggctcatggtggatgaacggaagacaatggctacgccgccactgagtgaattttataccaaggaaaagttcagcacgtcatgtttgacgcacgacgtctgatacaccaccgtggccaccactgcggtctggctgcggttgcggaccaccaaaggcgacaaccgcaacgatcccagcaattcgtaagaaaagctaaccgttacggtcgggcagcctctcgcagccagaccgctagccgacgcacccgcccgcgaaaatagcgtgatgttcgggacggcttcgcgtcaccgcaaactaacgtcggtagtcgcgcacgtcgtttatcctcagcacaccgtccgatcacaacccgttttcccactcagtcgcacaagcagcacataaaaaccccacacagtgcacgtgaaaacaacgtccctagaaaacggtgttttctgtcctaccgtcaccgggccacacaggcaaatcccgagcccgatccccgaaaacaccgtacggtgtttgtggcctccaaaatcacatcagataacaaaccgtgaaaagtcacgtttcacgaacacggtgtttttaaatcacaaagaaccacctgacggtttacaagcagaaacaccgcaccacggtggtacaagcgcggtggatctggtctcgcaacctcaatcgccgctatcaccaccgactttcgctgcgctccgccgacaaaacgccgtataagctacacaccccaaaaacccgcacgcctatgggcgccaaacgtgtgtattatctcaacgtcacgacacgacacaaacagcgtaacgtggtttcccgaacacgtacgcggcacagacccccgacacgtactcgaagaccttacagtttacgagtcaataaaacaggaaaagatccgaactttaaaattgtgtatttttattttcccatccccctctttttaccaaaaaacacatttttcgtcttgtaaaaagtaactttcgcccattgccatgaaacaccgtgatggggaacggtgttgtgtgtcgactgacgtcactacggcgatcagtatcgacgtcgtgtatacataacggtgcccggtgtttttattcggggcgttgtcgcgtcttgatgtaatgtaacctgaaaccgccgtgtccaagaatgcggaagccagcgtgtaatcataacggggttttgggtacaatctgacgacatctggcggcgagcgtacaccatcgaatgtggcgatcgccggctctacgtcacaatgacgcaaaaacacactgtaaaacacgcgtagacagctttcctggtcaacgagcgccatctggtgtcggcataagaacaggcatcaaccccgtggccggcgaggcggtgagcacttttgctggtcacgtgaccatcagcgcaggaagcgaggcccgtagaaccgcccaagaggcggtgccagatgccaacgtcataatcacaaggtgatttgttacgtcacgcgcgcgcacgcacgcgcgcgcggtagaatacagcgatccctagtgaagccacacccattacgtgtagccatatccgcttacgtatacagccacacccctaggtacgccaccttatctaccaatcatagaaacggatatacaatgacccctccctagactccaccccttgtacggaaatttcagataggtggaacccgttagggttccaccgtcctcggtgtacgtacaggcttctccgtctaccggaaatatacacctgctgacgtagacgctactcccggatacgcgtcataagctactggaccctaggggggagtgtctacagggctacgtgcacgcccccttacttagggtatccgcccccttcctctgttttggcctagtaaacttaacgccgccgcttctcacgtgacccctggcaagcctacgtcacactcgcgtgaccacacccactccggatatacgtcatcctgtggaattccggacatacggtgacgtagcgagcgtagcgagctacgtcacgtatgcgtacgtcacctccggcggaaatcatctctgatgacgtagcgagcgaagcgagctacgtcatcagtccgttttacgtataccgggtgctaggcgacgccccgtaggggcggagcctagcttccacccctaggatgcataccctatatagcataattcttctaacgaaacgttctacgaaaacggactggcggaacgggaaccaccgtaacccccccccctcacccccccccttctcctccggaaccggggggggcaaatttttaccaaatttgggcaaccatgttttccaatgggacggcgtttccgtgcgcatgcgcagtcggggcgaatttttggttgtcagggcgttgccacgcggattatgggatgggggctcgagtgcgcatgcgccggggatgccgcatggaaagcctatatataaggaggggtgaaccaggggccccggtgcgcatgcgcggaccaggccccgcgggagggtcgccctgcgcatgcgccggtaaaattccactgggtgtgtgtcgtgcgcatgcgccagtatttttccactggaggcggtcagtgcgcatgcgtcggtaaaattccactggatgtgcaccgtgcgcatgcgccggtatttttccactgggcggccgcacctagggagcgcgagccccgtgccgggcatgggccgcggcggtggaaaattaccgctccgcccacctaggcggggcatcttaaaacctataaaacccggcgtacccgccgccccccggcgcagtccgcggcagggttccggccgtgctgcggtccgcacgctgcgcccgctcccgcctgcctcccgccctaccccccaccctccccggccgaggcccggcgccggtccgtccgcgggcccgtcccaccgccctggagcaccatccggggccgtgggccgggcaccgggcgcggcccgctccggacctcggccgggggtccctcccctccccccgctcgacccccccatccgacggcccggccgggctgggacccccgcaccggggtcccggttcccgtccgcggcccggggggacccgagcgggggcttcccacccccaccccgctcctccccgggctccggcccgggatccctcgctgctcccggcgacctccgccggcttcccggtccacccgccgcggaacggacgggacccggggtccgcgcccttcccctccccccacggggggctgggtcacggaccccggttcctaggctcgttccgcggtgggcgaccggggatcccccacccagctccccttcccggcccgccccgctggcttttgggcccctccgggctttttttccggctgggggtcgcggcgctcggccgacgacgacggtaggtgggccgggtggacggtggtggggacgggcgacgccccggctcgacggcagtcggtcccggaaggttgggggctgggggcccggtcaggagctccgggagcggggtcgaccgcgacggcttccgggtctcgcggcggctccctctcggcggctccggttgggctcccctcccccctctcgagggtccggccgccagtcgtgaccgggggtccctcggcctagccgccggctctcggtccgccttatcctgggcgttggccggtcccgtgacgctcccctcccccgctgctccccaaaaaactccgcccgaaccgtcgcggcttgctggccctgggcgtggtcccccactcccctccccccatcggccgcccagccggggtcggcgcctcggaccccaccaggctgtggcgtgtgtgctggccgatgcggcggcgaggttgggtgtggccggaagcgctcggggtcgacggtgggccgtcatgacacctcaattgccgtcagtacgcccctccacaatcaccgtccctacacgatgggcccggcaggtcacccaacgttggttcaggcccagtcgggtttttccccggcacaaacgcacgtccccgtgggctccacgcgttttccaccctttcctggaggggtccggaacaccgtgaatccgcggggagggtctcggcacgggccgaggagaccacgaccgtcccacccggcgtgtcgacccgtccgagacccgggaagggaacaggccccacccttttttttcccttctccgatttgccgtggaaaacccgtgaaccgatacgggtacagacggccgaaaaaattcgagacgacaatacgacggcagggcgtgattttcttccccatccgacaaaaccgtgtccctcaaaattccccacctttctctgttcaaatggccccgaaactgtaaaacaccgttcgaccgcaccccaaccggcgccatcttggtgaccttctcgacggttctctcgctcgtcatgccgttctgagctccgacatggcggacgagagaaaatggcgtcgagagcataggagcgttttcgctccaggcgggtaaaagaatagcacgataacttttctgtgctttttttgagacgttttagaagagctttttttctgctcagagcgaaaaaatgatagccctgaaaatctcgacgagtctggccgagcggcgccatcttggaggaggggcgagtcgcgggcaccgcctcggtaccccctggccgaggcgagtccgcggtcgccgcctgttccgtgatgctacctagagggcgccgtcgaggcgactcttcctgttttcgccctgagggctaacggtcgctgacgtcaaaccatctcgtgctcgctgagtcacatccggttgttgacaagcgatggaggaccgcacccaaagtgcgccctctagtcatcgcgcctgaccccttttataaactgctcgaagaaaagaacaccttatgtgaaaaaatacagaatgatgacaagttcatccaacacaaccgctcaacaacgccatatctatcagtgtccaaaaactatcttctatcctttgaaactataaatgctgcctatatacatatttagtatccaagactcttaccacgtagacgaaaagaagtgatacaatgatcttgacgtgtatcgtctatatcgtgctagatatattcagataagacgcgcaaaccatagatttctcatcagtatcatgaaagacctatagctctatatacgaacctagtcattttaggacagccgccggagaagccgacgagggatcgggcgggtgcagccagaacctcacgcccgatcccgcctccggtaggcgatttgcatctgtttggtaaaaagctcataagtctgtatgtgacctatatatatattatacgctatgtacaccgaactgtcgctgttgtataagaagaaaaaactctccatatttatatcgtctgaatttttgcttgatagacacgtgtttggaactctgtccccccacgttttcactgtgtataacaaaaatatgtgtttctcaaaagatcttgaggtgtttgaaaacgggggaaacccgcgtttgggtgcgctaagccccggactgggacgtagccggcgtccggcacctatatttttctattttttttacaaaatatatgatgaaccaagaataaaactctagctctcgtctatttttaatatgctctacttagaacctttttaatgacagaatgaactccatgttatacgctctttatatagtttctctgcactaacctttaaaatcgtatccttccctgttgtacaaatcatcttttgatacacaatgatgacctgatatccctccatatatatgatcggatattattccgttagacttgtcctccttttttttcctcatctcctgtatctggagatatatgttgaccaccaccgccatgaccaccaaaaagctagccgtcacgactagaaatgtgtaggattcggactttccgttcgagaagaaagagaccgcgtctctggacgctctttttgtcggtctgaatcgacccgggatacgtaagagagcggccctacatcggggggcgctcgagaccgacgacgttccatctgaccagaaaaaaaaaaggcacccctcggtagcgacctctcaccatcgtttgcccgtccgcccgtccttcgtagccatcatcatcatctcaggctctatcggtaccatcgttgtcatctgaaaaaaaaaaactgcctcacccacctgcgtaaaaacaccatctttccggaggtgcggtaagacgggcaaatacggtcgtgccgaggcaaaaaaacgcaccatcgacaccacaccctcatgagcaccacctgtcggtgttggtcgtcctccatcgttctctacgaacatctcgacgcccgggtgacggacgacggcaagacgtcccggagaagacggtgttctctcgggcggtacgctctctggatctataatatctatagtagctaaacgagactgtgagtacgacgaaccacatcatcttttttttatgttgctcctttagaaaatgacttatgtcgacgacactcggcatcagccatctcgtgaaacacgctcgcttttcgtctctccaaggaacactgggtccgctgaaagggaccgtgtaccgaccaaagcaaaaaacacacacgtagtaacatgatcaaccacgtctgaatgacacgaaaacacaatcgtataacgctctattcatggaacgaacttggaataaaaaaaccatcgcaggccagaggctaagccgaaaccgtccggggaagcgggcgcgagttttccgacttagtctctggtgctcgttgagcctctttttttttcctgattctctgaagaatcaccgtcacagccctatgacgcgaaatcaattgctagaacataaacgttctcaacaggtatgaaatgaacaaactagatgatgctataaccttatattgtgtgtatatagataggtgtgaaatttgtaggataaaaagtgtcgttgtatgatgcacaacgatcgtgaaactggagactgtagctctctaccgaatgcaaatacacaaatgacatcgattcccgtccccacataaagaaatgtgctttactgtgaaagaatgaagaagattcttgttcctcgtacgacggggccctcgctcgtcgtacctcttcccccctccgggagaggggacgtcggggccctccgtcgcaccgggccgaagccagtgaaatgtttactacactgtcatcagaatatatgatgtatattatttcctccaaactcctcaccatagccaccaattcgcatcacttaagaaagtagtagcaaccgcggcggcggcgaccggccggtcgtcgtctcctcgtcctcaaatgttgtacatgtgcagaaaaatgtgtaaatacgtgttatttatcccatgcgtcttgtacatagatatatgtttttatatacgctatttatactttatatatccttttgcataaccatagacagtcaaggattttaatgatttgctcatccgcctttgagccatcgcttaggagttagttcctctatgttctcggcccaccttttcgactacagtagcaaacccttgtactaccaccccgataaaaaccacatcatcatcgtcaccacgacctggaaacgacacacgttcccccccaatcttgggcatgtgtatatatataaagaatgggagggagaggacgtggggctcgagaagaaataaacgccaagctcgattcgaaccaaaaaaccacatgtgtattgtgctttttttgtttttacggtggggaaaaggagggggccgtcattaacgaaaaccgtgtatggggtccggacacgaacagtacacagcttatggggaaaaaagctcacagagagaaaaaaacaccaagctcaggcacgcgtacatcattatcatcatcggatatctcaccacgagtcatagtagtaccaaggagtgtgtaacaccattttttcttttttctttgtaacgggataagggacagcaatcatcacgcacaacacccttcactctctttttagtcatccatatcatcgctgtaacacagcatgtcctcgtaatcgggcgtctggcagcgcattaccaccgagtcgtcttcttgcggtaccggtggtggcggcggcggcggcggctgctgctgggttaccgtcgtactgtgattaccgttggcggactgcaccgggatgataggctgcttgtggggaacctggggtggactgccgccgtgagaaggcgacggcgtcatcaagttaagctcaccacggtgactccggacaccggcgaggggccccgggggactgggagggaccgcggtcgtcttgtagacgacggtgtccccgtgtcgatccgtggctcgtaccagatcttgactgctagcgtcgtcactgtcttcgtcctcttccagctcgccctcagagtagtgctgctgcggttgcgacggtggctgggcgggaggagcggcggcgatcattggagagggatgtcgatgactcccttctctgtcctttttatcgtaggctgtcagcgttgctgggtccgtcctgctttccatatttgcgcattgctcatcggtgggatgaatttggtctcctccccgctgttgtccgccggcagtggcgtggttgctggcggttgtcgttgtcgtaccggcaaagacggtgagatccaatagtgactgctcgtcgaagggacagtacgctatcatgaaacgatagggtgccaacgcgcgttggatgcgcagttcgcacatctcgttctgacactcgtggcactgcagggcgcctaggatcaggtccgagacagcgccgcagcggtaggtacccatggcgttgttagtatcgaactggtcaaaaaattggggcgtaccggtgacttgcaacgcgcgacggcgtagcgagacggccacgcgcgagaaagagcacacgtaggccatggcgcggtgcatgggttgcgagaaggtctcgggcggacgcttctgcagatcgcagacgtcgtcgcgtagccaggcgctcatttgacctggctttttgactagccgtttgagcgtgctgcaatggtcgccccagccgtcctggtggtccaggatgcagcccaggtccaggttgttgagtttgttgaagagcagctgacgcatgccgcccaccgtctccagatagggatcgtgcgggttgacgggtagcccgtgcaggtggtggtacttcatgtagctgagcgtttcgtcgatgatggccagcaacgtgtgcaagttgggagcgttgtacacggcgaagatcttttccaccaccagcttgcgcagcaacggttcctccagccaatcgaactgttgacggatgtgcaacaggtagtcggtgtgcatgagctcgtcgtgtgacagcaggatgcgaccgcgcggctgatgatcttgcgggaaggcggtggggaccttgagatcggcggggtagggtgccagacgtagactctcggccgtgtagcgctgaaggtcgtagacgggcgaggtagaactcggtgaggtacccgacgaggcggcgccgcgctgcagacgcgctcttttcttcttttcgatcaaacggctgagttgctgtagttcgtcctcgtccatggcgtccagttcgtcgtcaataagcgccagcatctgttgttgttgcggtccggtggacgatccgtgatgattattggctgaagaggggtgagaagaaccgaaagtcgtaggacaactgggaactcggcgacgaagatgcgtcgaatcgccgccgtgatggtgcggttcgccgtcatcgttgtcgtaagacttaccgtagtgggggttaaggggcaccgaggcggacgcggccacgcgtcgcttgaaagaggaggacgccctatgtccgccacggaagcccgcggtgcccatgatgatgtgtccgccggtgcccccgagtgcgtggcgggaggagggtggaaggggaggaggatagtggtccggatcgccttcggtatcatcgtctttgctgtagcggggtcgtcgtgcggggacgcagggtcggtgatgatgcgaggcggcgccgacggtatcttccgcgagatggtattcgctggcggctgctccgttccgtgtcgacggcgaggttggacttcgctcgcgtcggaacttccgtggcacgggttcgtaatctagacagaagcgccgtgcgcgacgggcgcggcgttcgcgctcgctcagggaagataacgacggagcgtcgtgacggccgcgtgagtgcagctccatggccgccgtcgctaggaaggtcacgttcgggcacgctgatgtatatatagatgagaccgctgccggggggcgggtcaccggcgccgtggaaagtgaggctcagacggcggtcgccggcggcatgggcgcgtcgggcggtctgattttgatggaaatgtggacgtttttggcgttggagtgacactttttggtgaaacagcggctccagaggctggcccagagcgcgtagctgtgctcggtgcgcaggtcgatgaacacctgcacggtctcttgcgggttgcggtgcgtgtagttgagacagcgaaaatcccgcgtgcgcgcgccgtcgcgccgcttgacggccacgcagcaggcgccgtggggctgaaagaggaggacgtggggtgcggtaaactgctcgctgacgtgcggctcgtagtgttgcgtgaggtgctcgagcagcggcggccacacgcgggtgacgacgagccgctgcaagtccgtgtcggaaatcgcagcggcagtggcgccgtcgccaccgtacaggtgataggcgagcacctcggtgagaccgcggcgtcgataacgcgtcacgttaagcgagcgcgtctcgataaagttggcttcggtcgaggggcagattttgtcgcgcacgctgagaatgacgcgtggcggcggcgacaggggcaacgcgggcaggtcgtgcggcgggtggtggtgaagcaggttacgcagatccagttgggcgcgcacaaagcctagcgggtgttcgcggtaggcgtcgggcacgatgaacagcggcaacagacggcgatgcatgaaatagccgtcgtcttggtccattttatacatgtagggcagacgtacagagcgtccatggtggtagatgcctgtgtctaggctgctctcgggatgcgagatggggtccagcagcgtgtgcagttcggcgtcgagacagacggcgtgattgagcacctgcgccacggcgcgtaaaacgctggggtgtacggctacggtgcaggcggggaacggcgtgatgatgcgcagccccagtttgcccttgcagcggcagtaagggggtgacgtgtcaacggaggacgttggtttttgaaaaacgccgttatcagggacgttatttttgtcctctttcccgtcttcgtcttcctctgtgtcgcgctcgtcccggtaatcgagatagtcgtcgtcatcgaaaggcgcgccggccgcgtccacgggcacgctgttgggtgggcacgcgcttttgaagaaatagaccgggtgccggtcggggtgcgtgtagccaaagaggctcgcccatacggtcatccagacgcgtcgtagtccgcgacataattcaaagacggtgtgtcgcgccagaccggagacgccgtcgcgcagtcgtaaatcaaagtcggccacaaaattgaagacgggcagacgttcgttgaagacttcgtgtcgcgtgtagtagaactgtgtctcggggctggtgctggccacgtcgtcgtcgtgtagccacacggtctcggtcagggcctcgtccgagaaacggctgtcgggtacgtgacggagcaggtcgcgcggaaagaggctgcgatgccaggtttcggaggccacggcgcagaagacgtgctggtcattgggcaggtgtacgcggtagacgggcagcggtcgctccagcagcggtgccagcgcgggctcgggtagcaggtagcgacgttgcgagtaacgcgttagcgtgccggtggtgtaggtctgggctgtgcgcagcgaggcgcatagacgtaacaagccggacagggagcgttccagtggcgagaagacagactcggaaagcgtgttgatgcgttcgagctggcgcgccagctgcgtggaggtgccaaagaagcccgccaggtgcgtgccgtcgatgcggccgccgtagccggccagccccaggccgtgcgggctggtcgccgagtggggggattcgtcgagacccagtaggtgcgtctccacgtagtcgtgcagaaagttgtcgagcgagaagtatttttgcatgacgtccagcagctcggtggaaagccggcggcccagaaaacccggttcgcgcgtgcactgcgcttcgggcgccgcgtcagcgtcgtaagccaccacgcgccggtactcgagcaaccgcgcgcgtgccagcgccgtgcggtaggccaggtagacgtagtgcacgcagaccgtgtcgggcagacgcgcacgttcgcggaacgcgttgatctgcgtgtccacctgctctagctcggtgtagtcgcggcggttgcgcgccacggcgtacgccacgaaagcggacacgcgctgacggaagggcgagcccagtagcagacgcgcgaactcgcccatggaggcgtgcgtggggatgatggtgcccaggtcgcgcgtgcagaagctgcgcacgtactcctccacggtggagatggtgctgtactggccctcgaataggtagtaggccatggtcagcagcacctggccctcggtgtgcccgaagacgctgatgaaccacgagggcgaggtggggcagaggaagacctggttgagatgacgtagcacggccgcgtggtgaaagtacaccaggtgcttgaattcgcgcacctcgccgccgtgttcgggcgagagcacgggcgtgcggaagagatgccggtagagcggttgcgtctcggcctcgtccagactggcgatgagcgccgagagggggatgggctggcgcgcggccaggtagcgcgagagctgcagcgtttcgttgttcacggcgaagacgggcgccacccgccgcgagtccgagcacttttgcgtttgtaggcagaaataaacacgtcgcgagacctggtgtttgaccagcagggggaagacgcagtggtccgtcggtgtctgcgagagtacgttggcgactatatgagcagaatcatactctgttgcgaacagaacgagcgtcatcgtcgcgccggcacgatgcagctggcccagcgcctgtgcgagctgctgatgtgccgtcgcaaagccgcgcctgtggccgattacgtgctgctgcagcctagcgaggacgtggagctgcgcgagctgcaggcgtttctggacgagaactttaagcagctggagatcaccccggccgacctgcgaaccttttctcgcgacacggacgtggtgaaccacctgctgaagctgctgccgctctataggcaatgccagagcaagtgcgcgttcctcaagggctatctctcggagggctgtttgcctcacacgcggccggcggccgaggtggagtgcaagaaatcgcagcgtatcctagaggccctggacattctcatcctcaaactggtggtgggcgagtttgccatgtccgaggccgacagcctggagatgttgctggacaagttctccacggatcaggcctcgctggtggaggtgcagcgcgttatgggcctggtggacatggactgcgagaaaagcgcgtacatgctcgaggccggcgcggctgcgacggttgcaccaccgacgccaccggcggtcgttcagggggaaagcggcgtccgcgaggacggggaaacggtcgccgccgtgtcggcctttgcctgtccctcggtttcggactcgctgatccccgaggaaacgggggtcacgcgtcctatgatgagtttggctcacattaacaccgtctcctgtcccaccgttatgaggttcgaccagcggctgctggaagagggcgacgaggaggatgaagtgaccgtgatgtcgccgtcacccgagcccgtgcaacagcagccgccggtcgagcccgtgcagcagcagccccagggacgcgggtctcaccgtcggcgttacaaggagtcggcgccgcaggagacgctgcctacgaatcacgaacgcgagattttggatctcatgcgacacagccccgacgtgcctcgggaggcggtgatgtcaccgaccatggtcaccatacctcctccccagataccctttgtgggttccgcgcgtgaactcaggggcgtgaagaaaaagaaacccacggcggcggccttgctgtcctccgcgtgaacagcctggcacgttttggaaaacgtacgtgatcacggacacgacgagcacggggtttctcatagacgtactttattaggtcagggatgacggggaggtttcgggccgacgtcaaaaataacgtcactcgtgttgacagggctttctgcgtcggagctcttttcatcttcttctgtctcgtcgacgtcatcgtctaccggcgagggtgtccgttgcagcaacgcgtgctcgggcgtgtgggtgaaaccgatgtcgggggtgggcggcacgatcatctgtcctagggggtgactgcccaccggcagataggtaaagcggtgggtggtaaaaaccgctttggctacggtggtgtgtggggagatgcagacggtggtgtgcgaagtgttgaccaccgtcacgccggccgcggtacccgggagccagatggtgggtcgaatgatgagatccgattgactaaactggcgcacgcccactatgagggcgcagataccgggcgcgtgcacgtaggccgcgtcaaaatagacggtttgcgtgtgacccggaccgatcaccagcgtctgacgggtacgtaatgaaaagaaacggtgttcgttgggcggcggcaagttcatgagctgccagggttctggcacaaaacaggggaaaacgccgatatcgccttcgatggtgcccggaaagatggactgaaaagtgtcgttgaggttgacgacatccaactgcgggacttgcagcccggattccagcagctcgggcatgcaaacgaattgcgcgtccaggcatttgtaaaaggtaatgccaaaaaaaccttcggggatatagaggctgactcccagcgaggtgggcactttgcgctcgcgtgatagccaaatgatgtgtttattgtaaaaagccagctgcgtgtggcattgtttaacgatgaaactggaaggcatccacttgtagggaactttgagcggcgacggtaatggcgacgacgcttcatcctctcccggatgctgctctttgtcgtatttctcctcggtcgattggggcagcgtaaatgtggtttgaaaatcgctatcgctagcgaaacgcacgcagtaacgcatgttgacggatttctcggctaggatgatggagcctgatgacggtgcggactcttccttcattattaacgtaggggtctcccagaatcgctgaaaacgggagcgcggcagccgcgacagtaccagttgagagtcgattctgtcggtcaacattgtaagcatcgtggcggtggtgtgatggagtggaaaacagtgatactaggtgtttttgttttatcggtggcagcggggagttctggtaacagctcatccacgtcaacctccgcaactacgttaaaatcgtccagttctagcgtgtcaacaagcaaattgacgacaactgcgacaactacgacaactacgatgagtacgacctcatcgacaactaccactaaaccaagttccactactcacgaccctaatgtgatgaaacgacatactcacgatgatttttacaaggcacattgtacatcgcatatgtatgagctttcactgtccagcttcgcggcttggtggactatgcttaacgctctcattctcatgggagctttttgtatcgtattacgacattgctgtttccagaactttactgcaaccaccaccaaaggctattaagggtggacagatttacagctcgacggtgttccggcggggtaaggtttccataagtgggtgactggagactaaagttacggatctcatctagaaatagcagcgagtctagatagtcccacaggggatctataaacgttctctgaaatcccgttgatggtgacgtaggtgtagtttcggaagccgttttgttttccacgaacatggtttcgttgtaatataaggagctcatatcaagagtaccgtaaatagtgtacggtgtttcattacggattagtacatgcgtgtttttcataaattctgatacggcggttcggttgcggcttgattcacaaaaagggttttgccggtaacgtagagtggtatacacccacgtcgctaggtcccttaattgcgtggtcataatggacttcataaagctactatcaggacgataagcaattgtagacgtggaaacccgccttgcggtggtagtaacactataagttgcgttagtagtgacgttcagagcggttgacgttgtatagggagaatatggcgtagtagtactttgagatttcttactctttttttctgattgttctttgactggagcttgtttacgcttgagttttcgcatagtgtttttcaacttagtaccgttaatatacttagggacgcgaaataaatttcggctcatggcgttaaccaggtagaaactgtgcgtacagttgcgttgcgcgtaacgtagaagcaaggcggttaggcctaaaaagtagatcgtttgactatccacgtttactttcttggaacctacatataacttcgtgttccaacgtggcacattgaaaaacatggggttgaacgtggtgaaattgccgcagccttgttcgccagtatcattacgtttggaaacgtttagcatttcggaaagacaagtcatggaaggcaccgtaccgcaagatgggggtctgaatgttattgttttagccgtatgattgtattctgagaaaacgtacttagccggttttcgaagctgagtgctataaaaatcgaaccaaagataggtaacactgttattttgaatgggtcccgctaaaatgtaataccgtggaaactcggtcatgttcatagtcagatttttaatgtgttgtctggtcatattaaagtattttgtatagatatccttttctagttgtttcaaaatctctaatttgaacttgtctagtctttgcttgcctatcgtagacagtactttacctgaccagtaacgtcctacggataatcgtaccgcagccctacagtttatgaaagagaatagcaggaaagttagcgacataaggaagaataaattaaaaacacctctcatctctccttttctccccatgacagaggaggagaccccgcaccgtccgtctgccttgtggtttggcttgcctgcgtgtactcactgctgattctggtcgttttgctgctcatctaccgctgttgcatcggcttccaagacgacctagtttcccgcaccttggctgtgtaccgagcttgtatccagggaccgatatgtaaccagacccacaacagtacctcgtaaataaagacgcacacacctcacgcatatagtaccatcacaccgtgtggcgtgtactttattacaacgagcaagagtgccccctaactattggggcccgtaccgttttagaaggttttgtgtgaatgtctttaacttctctgtcccttttctcataaactgtcaggtcctacagtcagcatgtcttgagcatgcggtagagcagatagatgccgatgatggccgatagcgcgtagacggacatcatgaggagacgactgtcggtggcgtccacgacaacgtcagttacttctaggaccgtaccgtttttcaaaagcatgaggtagtgagttcgcggagatgagaccaccacttcgttgtagggatccagggcgaaaaggacgtcgtccgagtcgtgcatgtacatgatgttgatgacgccttgcgtgtcgtcgtattctagcagggcgctttggcaaaaggcgcagttttctagggaaatgttgagcgccgctgtgatgctgtgtgtggtatgcatgttgcgcgtcagttcgcatttagtttgactgtccgtctgggtgatgatgaggctttggcctacgacggtggtggagacagggtaggagatacctttgatcaggtactggtttgttacgacataactgacgtgttcggagacggtcagcgcggagaaggattcgcctagtggcagacaaaacaggtcggggaaggtttccaacgtgcttggttgcatggtagataggatggagagggcggcgggaacggtagtggggacggtggcatcggggaagagacgtgtgaggcgttcgagcgagtgatcgcgtcgcccgctactggaacagggtgtgtacaggtcgctgaggtattcgtggtgcggatgagctagcaactgcgtaaagtgtgatagctcggccaatgaacagaggcccgtttctacgatgaagatttcgcgtctctccgtcgtatgtaccagcatggagtggacgaggctgcccatgaggtagagttcttgacgcgcgaaggctgaaagaaaagaggccaggtgcgttttgtgtagttttagggcaaagtcggcgatctgtcgtagtgcccactgggggatgagatgttgctgattctgtttagagagtatgtagaccaggcgtacgaggctggtgatgtcggtgatctgattcggtgtccaaagggctcgtttggccaggtccacggccgtgggatacagtagcaacgtggtgcgtggtggtgtttgtgagaggcaggtgatcataaattcttgtatttgtaagagtgcggcctggcggtctagggcccgtgggacggagacttgggcgccggcctcttcttgtcgggctgctgcgaacagtgctaatgcgtaggcgaaggccatttctaccgtgcggcggtccagcatctgacatcgaccgctcttgagtacatccacggcgtaacggtgaaagctgttacgtagtagtgcgctgaggtctaggtagttgaagtcaagtgcggcgtcaagaaagtccgggtctttgagataagagtgacggttcagttgatctttcttaactagcaccaggagctcgtgtttttcagtttgtcgtagtataaagttgtcgcgttgatagggcgctttgaaaagtacgcgtggaagatggccgaagataagcagcatgggtgtgtcgtcgtctatggacaccgtaactacgaagaagtcctcggtcagtgtgattttaacgtaacgtagttcgtcgatgaggtaaaagccttggtgcaaacaaggtgtgacggtgctgaatagtagatcgtgtccatcaaagaggatacaggtctggttaaagtgtggtcggtgtagtcctgaggtggtatgtgattctgtccagccgtgtggagtggtttgcggtggcatccaaacgtgaggtattgacaggtcaatgggcggtggcacagtggtgggctgttcacctaggctgtcttgtgcctttagctgctgcgaaaaagatcggtagctggccaggtctttggataccagcgcgtaagtgttaagtctctgttggtatctttccagggtttcggtcagatctacctggttcagaaactgctccgccagaggacccgcaaaaagacatcgaggcatatggaatacatagtattgattatagctttggaaaaagttgaaactgatggcgttttccctgacgaccgtgctgttacggaggctgctgttgtaggtgcactgggtggtgttttcacgcaggaagcggatgggtctcccgtaggtgttgagtagtaggtgaaacgcgtgagggtccagcgcttcggatgcggcgtctgcgccatatcgttgcgaaggtaggtgactgaggaggtagacggcgaagacggtgaggtaggaggggaggccgggccgcatagcgcggccgcgccgctgggttcagcggcgtgatccaggtggtggttggcgttacacccgagagaaggagaaaaaggatcccaggaaggagcacccgggtgcggcgctacgggttacaaaagtcgcgtctccgtctatttaatacgatgtcattggccgctgcgaagggagaagaggggacacgcgaataagccatgccgtccgggcgtggggacgacgctgatttgacggggaacgctctgcggagattgcctcacgtgcgtaagcgaatcggtaagcgcaagcacctggacatctaccgtcgtctgctgcgggtctttccctcgtttgtggcgctcaaccgcctgttgggaggccttttcccacccgagttgcaaaagtaccgtcgccgtcttttcatcgaagtacgattaagtcggcggattcccgactgcgtgttggtgtttttaccgccggactctgggtcgcgcggcatcgtgtattgctacgtgattgagttcaaaaccacgtactcagacgccgacgatcagtccgtgcggtggcacgccacccacagcctgcagtacgccgagggcctgcgccagctcaagggcgcactggtggactttgattttctgcgtctgccacgcggtggcggtcaagtctggagcgtggtgcccagtctggttttttttcagcaaaaggccgatcgcccatccttttatcgggctttccgctcaggccgttttaacctgtgtaccgattctgtcctggactatctagggaggcgtcaggatgagtctgttgcacaccttttggcggctacccgtcgccgtcttcttcgagccgcacgaggaaaacgtgctgcgctgccccgagcgcgtgcttcggcggttgctggaggacgcggcggtggcaacgcgcggcgggggctggcgcgaggacgtgctcatggaccgggtgcgcaaacggtatctgcgtcaggagctcagggatctgggtcacagggtgcagacttactgcgaggatctcgaagggcgcgtgtccgaggcggaggcgttgttgaaccagcagtgcgagctcgacgaaggaccgtcgccgcggacgctgctacaaccaccgtgtcgtccgcgttcgtcgtccccagggaccggcgtggcaggagcttccgccgtcccacacggtctttatagtcggcacgatgccatcacgggacccgccgccgccccgtctgacgcggcgaccgcgtcagcggccgccggtgcttcttctacctggctggcgcagtgcgccgagcggccgttgcccgggaacgtacctagctactttggaatcacgcagaacgatccctttatccgctttcacaccgattttcgtggcgaggtggttaacaccatgttcgaaaacgcctccacttggactttctcctttggtatctggtactatcggctcaagcgggggttgtacacgcaaccacggtggaaacgagtgtaccatctggcgcagatggacaacttttccatttcgcaggagctgctgcttggcgtggtcaacgctttggaaaacgtgacggtgtatccgacgtacgactgcgtactctccgatttggaagccgccgcctgtctgctggccgcctacggacacgcgctttgggagggccgcgatccgccggactccgtgacggcggtgttgagtgagctacctcagctgttgccgcgtctggccgacgacgtgagtcgtgagattgccgcttgggaaggccccgtcgccgtgggtaacaactattacgcgtatcgcgactcgcccgatctacgctactacatgcccctaagcggtggtcgccactatcacccgggcacttttgatcgtcacgtgctggtgcggcttttccacaaacgcggcgtcctccagcatttgccgggctacgggacgataacggaggagctggtgcaagagcgtctgtcgggccaggtgcgcgacgacgtgctttctctctggagtcgacgtctgctggtcggcaagctgggtcgcgacgtgcccgtctttgtgcacgaacagcaatatctgcgttcgggcctgacctgcctggctggcctgctgttgttgtggaaggtgaccaacgcggatagcgtcttcgctccgcgcacgggcaaatttacgttggccgacctgctgggttcggatgccgtagccagcggcgggttgcccggggggcgcgcgggcggcgaagaggagggctacgggggacggcacgggcgggtacgtaactttgagtttctggtgcagtactacatcgggccgtggtacgcgcgcgaccccgcggtcacgctgtcgcagctctttcccggcctggctctgttggccgtgaccgaaagcgtgcgcagcggctgggatccctcacgtcgcgaggacagcgccggaggtggcgacggcggcggcgccgtgctcatgcagctcagcaagagcaaccccgtggccgactacatgttcgcgcagagctccaaacagtacggcgatttacgtcgcttggaggtacacgacgctctgctctttcactacgaacacgggctagggcggctgttgtcagtgaccctgccgcgtcatcgtgtgtccactctgggctcgtccctctttaacgtcaacgatatttacgaactgttgtactttttagtgttgggttttcttccgagcgtggcggtgttgtaatttccaccacgtgtcgctcgctgcataaagggcgagcgtccccggagagggtatattcgtttggcgagagcgggcagcggtggtgggtatgtccccttctgcggagaagactacctcagtcaccgattccatcatgctcgctatcgtgaatttcaaatacatgggcccgttcgaaggctactctatgtcggccgatcgcgccgcctcggatctactcatcggcatgttcggctccgttagcctggtcaacctgctgactatcatcggttgcctctgggtgttgcgtgttacgcggccgcccgtgtccgtgatgatttttacttggaatctggtacttagtcagtttttttccatcgtggccaccatgttgtccaagggtatcatgctgcgtggcgctctaaatctcagcctctgtcgcttagtgctctttgttgacgacgtgggcctatattcgacggcgttgtttttcctctttctgatactggatcgtctgtcggccatctcttacggccgtgatctctggcatcatgagacgcgcgaaaacgccggcgtggcgctctacgcggtcgcctttgcctgggttctttccatcgtagccgctgtgcccaccgccgctacgggttcactggactaccgttggctaggctgtcagatccctatacagtatgccgcggtggacctcaccatcaagatgtggtttttgctgggggcgcccatgatcgccgtactggctaacgtggtagagttggcctacagcgatcggcgtgaccacgtctggtcctacgtgggtcgtgtctgcaccttctacgtgacgtgtctcatgctttttgtgccttactactgcttcagagtcctacgcggtgtactgcagcccgctagcgcggccggcaccggtttcggcattatggattacgtggaattggctacgcgtacccttctcaccatgcgtcttggcattctgccgctctttatcattgcgttcttctcccgcgagcccaccaaggatctggatgactcctttgattatctggtcgagagatgtcagcaaagctgccacggtcatttcgtacgtcggttggtgcaggcgttgaagcgggctatgtatagcgtggagctggccgcgtgttacttttctacgtccgtccgagacgtcgccgaggcggtgaaaaagtcctccagccgttgttacgccgacgcgacgtcggcgaccgttgtggtaacgacggccacgtctgagaaagccacgttggtggagcacgcggaaggtatggcttccgaaatgtgtcctgggactacgatcgacgtttcggccgagagttcctccgtcctctgcaccgacggcgaaaacaccgtcgcgtcggacgcgacggtgacggcattatgagcggcggcgctgtacgccagcggggagaaaagtggcagataaatcacgtcaggttcacacgtcgttagccagcgtcggcatatgaagggcgcgggcggccagtacggcctctgggctgagacaggacgaggcagggtgagaaagaggaggatgggggggaccggggtggtggtgctgctgctgttgtgggtgtggacggtgcggatgccgggacagcgtgccggcgaacgttctgtaatcttccataataaaggtaaaaatgcccgtctcgtgtcgactccgctggatctcgaaggcgtcgggggtaatgcgcatcttgccggtgccgatgagataaaagtaccacattttttgacagatgatgcgaatcaagggttcgtacgcttcggcaccccagtggcgcgtgaagaaggccgccagacgaaacaagcggtgtccgtagagcgtgcctagggagaagaggatgttgccgttgcgcgccaggtcttcggggaaaacgaccggcaggccggtgtggcgctgcacaaagcgcgtcagcagtccgccgctcaagcgcgggtgacacaggcgctggctgagacgggcggcgcgcgtttcatcgaacacggccgcctcaaagtccagccccgggaaggcctgacgcagttcgcggtacagatgaggccagtagggttgcggcgtcttgcgactaagcacggcgtggtccgagacgcccaggttgttcatggtttcgcgcagtagcagcgtttcgagaccgcggtgaaagaggaggacgcagatgaggcgtacgattttgagttcttccaaacgcagcgagctcagcggctgtccgcgcgacatcttctcgctaatctgtaatattagatgattggcgcaagtaaaggagaatttgcccgtgcggacccgcgggacggcggggttctcttcgtcgcgggccatcatcgttcgctcggtgagcgggtagcgacggtgacgacaatgacgatggacgagcagcagtcgcaggctgtggcgccggtctacgtgggcggctttctcgcccgctacgaccagtctccggacgaggccgaattgctgttgccgcgggacgtagtggagcactggttgcacgcgcagggccagggacagccttcgttgtcggtcgcgctcccgctcaatatcaaccacgacgacacggccgttgtaggacacgttgcggcgatgcagagcgtccgcgacggtcttttttgcctgggctgcgtcacttcgcccaggtttctggagattgtacgccgcgcttcggaaaagtccgagctggtttcgcgcgggcccgtcagtccgctgcagccggacaaggtggtggagtttctcagcggcagttacgccggcctctcgctctccagccggcgctgcgacgacgtggaggccgcgacgtcgctttcgggctcggaaaccacgccgttcaaacacgtggctttgtgcagcgtgggtcggcgtcgcggtacgttggccgtgtacgggcgcgatcccgagtgggtcactcagcggtttccagacctcacggcggccgaccgcgacgggctacgtgcacagtggcagcgctgcggcagcactgctgtcgacgcgtcgggcgatccctttcgctcagacagctacggcctgttgggcaacagcgtggacgcgctctacatccgtgagcgactgcccaagctgcgctacgacaagcaactagtcggcgtgacggagcgcgagtcgtacgtcaaggcgagcgtttcgcctgaggcggcgtgcgatattaaagcggcgcccgccgagcgttcgggcgacagccgcagtcgggccgccacgccggcggctggggcgcgcgttccctcttcatccccgtcacctccagtcgaaccgccatctcctgttcagtcgcctgcgcttccagtgtcgccgtccgttctccccgcggaatcaccgccgtcgctttctccctcggagtcggcagaggcggcgtccatgtcgcaccctctgagtgctgcggttaccgccgctacggctcctccaggtgctaccgtggcaggtgcgtcgccggctgtgccgtctctagcgtggcctcacgacggagtttatttacccaaagacgcttttttctcgctacttggggccagtcgctcggcagcgcccgtcatgtatcccggcgccgtagcggcccctccttctgcttcgccagcaccgctgcctttgccgtcttatcccgcgtcctacggcgcccccgtcgtgggttacgaccagttggcggcacgtcactttgcggactacgtggatccccattatcccgggtggggtcggcgttacgagcccacgccgcctttgcattcgtcttatcccgtgccgccgccaccatcaccggcctattaccgtcggcgcgactctccgggcggtatggatgaaccaccgtccggatgggagcgttacgacggtggtcaccgtggtcagtcgcagaagcagcaccgtcacgggggcagcggcggacacaacaaacgccgtaaggaagccgcggcggcgtcgtcgtcgtcctcggacgaagacttgagtttccccggcgaggccgagcacggccgggcgcgaaagcgtctaaaaagtcacgtcaatagcgacggtggaagtggcgggcacgcgggttccaatcagcagcagcaacaacgttacgatgaactgcgggatgccattcacgagctgaaacgcgatctgtttgccgcgcggcagagttctacgttactttcggcggctctccccgctgcggcctcttcctccccaactactactaccgtgtgtactcccaccggcgagctgacgagcggcggaggagaaacaccgacggcacttctatccggaggtgccaaggtagctgagcgcgctcaggccggcgtggtgaacgccagttgccgcctcgctaccgcgtcgggttctgaggcggcaacggccgggccctcgatggcaggttcttcttcctgcccggctagtgtcgtgttagccgccgctgctgctcaagccgccgcagcttcccagagcccgcccaaagacatggtagatctgaatcggcggatttttgtggctgcgctcaataagctcgagtaagagagacgctatatttagggtttccctctcttttttttttctacaccgtgataccctaataaagcacactgcggttattatcaacgtctctgtgtttttattatttagaaataaatacagggaatgggaaaaacacgcgggggaaaaacaaagaagtctctctctactggctcagaggatcgttgccgaacagggacttcagggacaccagggggggcacctgctctctgtccttctgctcctgcttgggcaggctggcgatgccctcgcccatgccgaacagctcggcgggaggggcggtgggctcgggtctgctctgggggaaattgccgggtctgcccttgctgctaggccaaatcttgcccaggaaattggcctgcctctcggtgcagtccttcatctggtgcccttccttgccacacttccagcagcccttcttcctgggggctctgcagtttctggccaggtggccctccttgccgcagttgaagcacttgatccgcttctggcctctgaagttgccccgctgcatcatgatgttggtctgctgggcctggctcatggcctcggccagcactctggccttgtggccgggtccgcccactccctggcaggcggtcatcatctcctccagtgtggcgccgctgcccagggccttcaggatgctcttgcagtcggggttggcgttctgcaccagcagggtctcggtcatccagcccttcacgtcctgggtggcctgctcggctctcagggccttgaagaaccggtccacgtagtctctgaagggctccttggggccctgcttgatatccaggatggacacggggctgtacatccgcacaatcttgttcaggcccaggatgatccaccgcttgtagatgttgcccacagggatgggagggttgccggtcatccactgcagctgttcttgaggggtggaggtggtgccggcgatgtcgctgcctctgggctctctgatctggccaggggggatgggtccggcctgcacggggtgcagtctgtcccactcggcggcctcctcattgatggtgtccttcagcatctgcatggcggcctggtgtccgcccacaatgttcagcatcacgttcaggtcctggggggtggcgccctcgctcagggcgctgaacatagggatcacttcggggctgaaggccttttcctcgatcactttcacccaggcattcagggttctggggctcaggttctggtggatcatctggccctgggcattctggatgatggggtagttctggctcactttgctgctgtcgccggtgtcggcagcggcctgctgggttttctgcttgctcttgttctggatctcctcgatcttgtccagggcctccttggtatccttcacgtcgatccgctggtgcacgcagtacagggtggccacggtgttgaacaggctcttgatctcctcggtgccggttttcacggcgggctgcagctggttcatgatctgctggcagccctcggtggtctccagcaggctaggattcagggcgaagcgatccagctctctgctggcccacaccaggtgcttcagccggtacttcttcttgccgccaggcctcagtctgatcttctcccaggcgtccagcttgcccccgctcaggatgctggctctggcggccatggtggctgcgaaggcgggatggggggagggtcaggggatgcgcaaaggtgaacgggtcttcgtgggaggtcgggaagggttccggcaactgtcgcaaatatagcagcggcgacaggtgtggcgcccaaaagtcgcgtgtctgagtggacgtgggtttttatagagtcgtcttaagcgcgtgcgcggcgggtggctcaacctcgatgctttttgggcgtcgaggcgatgcatggcccgggcagggcttcttgccggtggcggcgacgtttgggttgcgcagcgggctgccatacgccttccaattcggcgaagatgcggtagatgtcgttggcgtcccagaagaactcctggtacttcagattctgaccctgaaccgtagccaccatgggcaccaggttgcgggccaggatgccggcctgccagggcggccaggtgaacacggccggattgtggatttcgttgtcggaatcctcgtcggtgtcctcttcgggcgcgacggtggactcggccttaaggcggccgcgtgtcataacgcccgccgtgcacgccgtcgccgaggatgctgatttgcgtttgcggcccgcggaagtggaggcgcccgccatggcgccgccgccggtaacgcggggcgtcttgcgctcggtggttacgagttcttcgtcggagtccgatccgctggtccagacgtcgtcgtcgccctgggcggcaccctcgtcgtgccggtcccaggtgtgtcggtactcaagcttgccctggatgcgatactggctggtgaaggtggggtgctcgctgtactgaggcccgcgctgcagcagcaagtcgatatcgaaaaagaagagcgcagccacgggatcgtactgacgcagttccacggtctcgcgtatcgcttgtacctccaggaagatctgctgcccgttcatcaacaggttacctgagatgctcaggcccgggatgctcttgggacacagcagcccaaaatgctcgtgtgaggtaaaagccacatccagcatgatgtgcgagatcttgcccggtttgattatcatatttttgggacacaacaccgtaaagccgttgcgctcgtgggggcgcatgaagggttgcgggttgcgggtcatcgtcaggtcctcttccacgtcagagcccagcgtgacgtgcataaagagcttgccggagggcacgtcctcgcagaaggactccaggtacaccttgacgtactggtcacctatcacctgcatcttggttgcgcgcgtgttctccatggagcaaaccagctcgtgcgcgcacaccacgtgccgcagtgccacgtccttggtgggaaacacgaacgctgacgtgtagtagacgtcgggctctttccactggttctgctgacgcgtccaggccagtcccgagaccgtgagacgcgcctgccacatctgcttgcccgacgcgtgaatcacagcgtcagctacgggcaggtgtcggtgtttgcgctcggccgccgacgggtagtggtgcacgttgatgctggggatgttcagcatcttgagcggcagcgcgtacacatagatcgacatgggctcctggctggggcagatgcttcggcccgtggggttgtgcacgttgaccgacacgttctccacctcgctgcccgtaaagtacgtgtgctgcacctgcagctgattgtcgccgcggtggcatggcgtcgagtcgggcgtgtactgcgacaccaggatcagcgagggctggctcacgcgtacgtggatacccgtctgcaggagtcgcgtctcgtgcggcagcaccggcgtgtcgccgcgactaaacacggctttcagcacgtgccccgaaatgggacccagtacggatatcatttcgggacaacggcgaccgcgcgactccatgctgcctgcgcgtacgggtgtaggcgactgagcggcgcgccctttgcggccgccgccttacataggcaggcgaccaaacgcggaacccgaaataaaaacgttctacacagagacaaccgcggattattgagtgtctttttttattacaaaaaaaaagaggcaaagccccaccgtcaccacaccccatcacacaccaccaccgattttttttgttttaaccccgtatcgcgcggacgcctagtgtccgtttcccatcaccagggtcctctgtttagagatcgccgcagaccatggctaaagtgacaggactcgttttctctgtcgtattttccgtgagcttacagtcttgcggttccgtctccggggacgccagtcgcatgggcagcaggtcctccagcgcgatggaagcgcccagcaccgagagctgctgttgcgacggcgaatgggacgtggaccgcgagtgtagcgtggatttgacttggtgcgtcattgctgacaggcaaccgcgattcagcgtatgctttgacgagataaaatagaggcgtcccaggagcgcgtcccgtgggaacgtggcgccgttctcgtcgctcaccagtacggttaattccaaccaggagcgcggtagccagaccgtaacgggcattttgagtccctgacggttgtgtggtacaaaaacacccagataaggcccgtaaaagcggcggtagatacgtaacgtgtgcgagtttttcagcgtcaattcgtaagggacgcgcacctccagtccctcgtccgccgcaccggagcgtggcggtacaaagtaaggcagtggcgcgtccgaaaagaagggtcgtcgcaccgtttcgcgtcgcagccgcaggcgaaacgccactgggtcggctggcgcctcggtgcggtcgcaggtcacgttgaaacgtaacatgccgtcttggtatagcgtgagtgacgacagcgtcaggtccggcggtgattcgttcgggtctagctccaatcgtccaaagacggagggtcccaatgtcttggcagtggtttccgagaggcgcgccgagatacggctggtgagtccacgcggccccgagatgccgccttccactcgatgccagcacagcgcgtgtcgtacgcgcaccgtcagcgtgggcgtcagatccgcgtccgttgattccgcggtatcagcgacggaagccgcgttctccgttacgttgtttatatccagcgtcggctcgaacgtgagttctggcagatgcagcgcaagacagtcgtgtaacgccgtgtgatgcgcggctttacgtcgtagcggtagccgtttcagcagcggcgtgatgatacggagcgcgaagagattgagtgataagcgcacgatggccatgcgcgtcagttgctggtcgattactgagcgcaggatatggcagcctgggcgtgcgggaaagagagagaaggccgggcgtacgtcagaatcctcgttagataccacgcatagaatgccgcgttcacgatcgtcgttgcggtcatcctcgtcctcttcttttttcttctctttttccttttttttctcgggctcatgggaagccgccgtttcttcttcttgcgacgtcgcggagtcggtttgagactcgccgttcgcttcccccaattgcagcggcgtagagagcagaatctggaagggatcccgcaattcttcgggtcggaggtcgaggtgcaactggatcagatggtaggtgccgcggtgcacccgaggctgacggatgtcgtgtttatccgtcagtgtgaggatggtctgcggcgagccgctgtgcttgtccagctcgtccggcgttttcaggaggaggctgtcgtcgtcggtactggcgacgcccatcatggtcgtggtggtagtggtggcgaggaaagtgagcggcggcgctgacagagctcggcgttggcggcggcatttgccgctgtgtcggctgctattgctgccaacgccaccgccgccgcctcgtctggctcgtggccggcgggcccgattccgaaggttggggtcgacgcgtggcatgcttggtgtctgcgggcgcgagagggctggctcagcctttaaatatgcaggtcgcggatttgttatcgggtgaaacgtcacacaccgtgaagacgacctgttcgcggatgaggtcatccagctgtcgcagcatgacgaaaagcgccgacagccgcgcgatctcgtcgtcgggcgacacgtgctgcggccgcgcgggcgtgcgcggctcgccgacgctgcgctcgcggtccagccgcatcagcagctcctggcacttgacgagcagcatggagctgtcctctagcgccaacttgcgcacgtaggtcatggtcagctccgaggctaggttggccaccatggacatggagaggcaggcggtcttcatgtcgatcagcaggtgctggtcgatgaccggatcggggatggtgaaggtggcgtcgcgaaaagtaatggtctgcagctgctgcacggcagcctttacctcctcgtacgaacggtcgagcgagaagaggcccatgatgagtagtcgctggttgatttccagcgccagtggcatgggtacgatccagggcagcaccagctcccactggcccagcgtcagcaggttctcgcgcgccagcggtccgtggaagagcggcggcagcacgcatagcgcgtcgcccttctcccaagtcacgggtcccgtgttgaggacggtgtagagcagtccgtgcgtcggtacgtgtaggaggatctggttgccttctacgcgccgcatcaacgtcagcgtcatattgcgcagcaggccgcgcagtcgtacgtagccgcgggtgtgatctacgaactggtgtaggcccagctggtagtgtttgatgagatgtagacgctgcggaatgggcacaacggccgctactagcttggtcagtttgcctacgtcggcgatgctgagcttgtggtcgaaagtgcagaagatgttggcctccatggccgccatagcggcggtgaaatcctggccgcgacggaggagaagcagagacgaacaacgtctgcaccgggcgcggcgtcagagcgagcgtggcgcgtccgggcccgcgtttgcgtctaggtgattcgccgttaacctgcggtcgtcgccgtcctcctcaccggacggcctcacgagttaaataacatggattgctgtagcgggatgatttcgcctacgacgtagttaccaaagtgcgtttcggacgtggcaaaagccccggcgccacccttgagtttggtctccatcagcgccagcgtggtggtgctgaggatcggtagcgcttcctgcgtcagacggcacgggttttcgatgagttgttccgtgccttcgacgcagacgtactgcgtgtccgtgtcgccgcggatgcagtccttggcgcgtagcaggtactcgtcgatggttttgaagagcgttttgttggccgcgataatctcttccgtgttaaagtactgcgcgcaggggctgtagaatttggagttgtagcctagacgttcgcgatgtcgggtgttgtagagtacgtcgctcagacagccggcttgcgaggcccaggggttgtgtgtggccgcgaaagtctgtgcgtccgcttcgcgatggtcgtagatggccttggtggcggcctccgtgtcgtacggatcgacggccagcatgcaggaggcacgcccgcgcgggttgttggggatcttaaagtaattaacgtccatcgtcaccggcgtaaggattagttcgcacgcggccttttgtccgtgcaccgtggcggcggcattgcgctcggacatgctgccgaacgtcagcatggagatggtctccgtgtctaacagttgcggccgttctacgccggccgcgtgccggatccagcggtccacctcgtcgtgccggtacacgttcatagggaagacgcgaaagaggtcctgcacgcggacgcccatgtcggttcgcacgcggtttacgtaggctacgcaggtatttgacgtgtaacccagacccatgtctacggtgttaatgttctgcgtgacgtggtacgtggtgctgatgtcgcgttcctccttggtcacgatagggttgttgatgataactgacgtgcacgatttgccgctgtagagcagcatgtccacctcgaaggtgtcggtgcgtacggccgtgagtgcgaatcccgggtggatgtgcgccttggtctgcagcaccagtgaaactggtgagattttgtataacatggcggccagcgtcatgactgagtgcaacacgttgggacaggtggccgagtaacgcgaaaagggcgagcgcagccagttgtggtactcgtgtgcgaaggctgtgggtagcgggaaaccaccgtcgtgacggtgatagtgcgggaactcggtcacgtagcgtttaatgtcgtcgctcaacgccgcgcagatggtggggtttgagtagaaacggtggaaaggtacgggtaggctgtactcgatcaacgtcttaggcgccgtcacgacgcagcagccgttgtaaagcacgtgctgacgtgagataaagtccggcaggccctgacgttgcgcgtggtccagaggcgcgcgcacttcgagcaccttgacgtgctcgcccacgaattgcacggccaaaaacagttcacgacaggcctgcagcagcggcgtgtgcgcgtcggtggcgacgtcctccaccagctcggtcagcatctcgcctacggcttgacgttgcgccgctatcgagtcttcgggggtgacgccgcttgtgctctctttcgacgtcgtacctgacgtggagaccgcggtggcggccggcatcaggagaaacgccggtcggtaaaagaggtctactagcagcgtcttgaggttgagtcccaggccgcaggcccggttgttggtcatggcgggcatgaggcagagataaaagaccttttgtaacgtccattcgtcgtcggtggcacggtaatcgtccacaaacagcggctcgtcggcatccatggcgcccaaacgcggtacgtcagaaacgccgtggtgtcgcgcctcgatgttggccgggttcaacggttgccggtcggccactacctgtacgccttccatgttacgcggcaggtgcgtaacgaaggggggccacagccggtggtcgtgcagcgcgttcacgtaagccgatagcggttcctcagccagttgaccgttgttaagtcccggcagcgctgagatgcgcgttaccagacgcagcacggcgaccagattgcggtagtgaaagagcaactgcggtggtagggcgccatcagccaggtgttcggcgatcaacgtcaccagcgcgtagctgtgcgcaaaaaccagcagctgacgtgtgtgaaacatgttgacgatacaacgtgctacgaaagtgcggattagcaaaaaagcgtcgacgttgccgtgtaccagcacgtcgaccaggtagcagagctcggggtaattggggcttgtcacggtggttttgaaaagtcgcaacgtctcttcgtagtcgggtggtggccgcagtcgcatgtgttccatgatctcccaggtgcgcagttcgtggaaggggcccggtgccagtccatctggcaaattaccgatgacgatacgcggtgtacacagcgccaccgtttcgctgttttcctggcagtgcgtaaagtcgaagaaggggtgcagctcggtgtagagcgtgatgttgcccaccttgtagaagtcggtgaccacaaagtcctgcttcatttcgttcaccgtgcgcgggacctcgcgtcgtacgcggtaaaaatgcggtatgcggcgcgccgcaccgcccatgggttcctgctgaaaacgacactcgagcagtcgttgcatggcgggttccgagggcggtccgcgttccgtgaaggtctgtagacagggcgcgggctcgtgcagcaccgggtggcacagcgtcttgagcgcgtccacaaagtctatcttttgtacggcacggtcccggtttagcaggtaggccgtggtgggcaacgcgttgcgaacggtgtcgttaagcttaactttgctttccaccgtggtgtaaccgcgatcctcgggcagatacagccctacggggaagaaaaacgtcaggtccacgttacgttctagcggatctttggtatcggtgtttttgtagacgcgccgcaagttttccataatcaccgttttttcgcccagtcggatcacgtccatgctcagcggcgttaagctgtgcgccccggcctgcgaaagcgagtcgttgggcaaatgcggttggcccgaagtcagatgagccttgtacgagttgaaatcggccaggatcgagtgataggatatggcagtgacggcattttcgggactgagtacaaaattgccgtaggtggccggcgccgagaccgtttctttggtgatgtggcttgagagcagcgacatgatgatctgcataacgttggccgtgcttaccatcacgccgctgatcttggcccccgagctcgtggtgtacgtcgtggggttgtctaggatgctatcggtggccgcttcggctagacgcgtgaggaacttgagcacatagtcgcgatcgcgcgtgcgattcagcaaaaagagcgtggccagcattttggccttgaagctctgcaagatgttgcttcgctggatgcggttcagcgcctgtcgcgccagcgtggcgttctctaccagcgtctgcactacaaagtacggcggcgccttgcgtagcagtgtctgtaaaaagctgtgaatcaagccgcgttccatggcgtcggccgtgtttttgagcgcgcgcagcaccgtgtgcatagcttccacgttgaggatcttgtccaggatggtgccttcgaacgtctcgcgcagatacgtgaggcaggctgcgctgagctcaaaggggatggtgatgggggatttttcactgtatttggtgaccataatggtggtctgacgactggtgggcaaaccggcgccgctggccacacgcggcacctgcacgtggaacagcatttttcccgtagtcagtttattgaggtcgtggaacttgatggcgtgcgccgccgcggccaagccgctggtcaaaaaataaacccattccaggcgattgcagaaggtgccgaagatggcttcgaagtgaatattgtaacgctcggggtcgtcgccgtagtagatgcgtaaggcctcgaacatctcctcgccggcgctggtcttgacgtgcgtcagaaagtcagtgggaatgcctactttaggcaggagctcgagcgccgaccagttctccatcgcggcggcggcgtgagcgcgaggcgtcggagctcggggaaagcagcgcgacccggagaatggccggcgctgcgccgcgccgcctcggctgtgacgctctaatagtcgtcggcggctccgctacgccgcgccgggttttacacgtccccgtgcacgttcgcgcctgcaacctcacccaagagctatcgacgggcgaggacgcccgcttctgtcgtccgcgacccgttaacgtcgaacgggtgcgcgctgtttttgcggctctctaccgtgcctgtccgatacacgtgaggaccgagcccgagcgtgtcaagctggtactgggtcgtctgttactgggacccgtggccgtaccctgtttttgcgacggtgaagtggagggccacggtgaacatctggtacctacgacgcagttttgtcgcgggccgctgctctacgtgcaccgacgttgttgttgcggatccgtgaccgccgggcgcgcgctgtcctaccacgttctcgaaaaccacgtggccacgcatgtgctacgcggattgctctcgctgacggaatggaatcgagaattgccgagcctcttttgcgactgtcctggcggcggtggcgcctcgggaaccgaggaacgctacgccatggcctgcctgccgcgcgacctcagcctgcacctggacgactatccttacctgatggtggaaatcggacgcgtactcagtgtcagcgaggtagacgactacgtaaccgccgtctccggctacctgggcgaggccgcggcgccgcgcattcaggttcactacaagctgctctttggactcaacgtgcgtccgcaagcgccgtgcgcgttggacgctacacgcgacttttttctgctggagctgcaaaagctttggctgggcgttgaatatcaccacgaagtgacgtcggagtttttcggtcgcgtgctggcccagctgcatcgcgaccgcgcccgcgtcatgatggcgcttcgcttgcccgagcagacggtgtgccacctgagcaccttcgttctcagtcgcttcaagcgacaggtactgtacttcaagttacaggtgagctacggcaagtgccggactggccacgctgacagaagtgggggaggggggaacggtggaaatcagggacaccacaacctactgtgttatcgacgccttagcgtcacatttgccgacacagacacggtgtggagaaaccttttctacgtttattacgaactagctcgggatctggggtcccatgggacagagaaccgacccgtaaaccgcggttacggtgtttcttgcgctccgaggacgtcgcggctatcaccgtcagaatcgacggtggtttcggcgaacggacacgcgctgtcttccaccgcgctcccgacgacgagcgcgggtcacaagctgtcactgccgcgcgacccggccgccgatcgcgttcgacgttacgtgtgcattatctcgcgtctcatgtacgctcggtacggggagagatggcgtaaacaccgtcaacggcggtcggagacgggagaagaggaggaggaagagacgctggaatcgggggagactgacgccacgccgccatttgactttacggggcagcagctgcgccgggcctatcaggaacaccgacgtcgtaaacatctagccgtgcagcgttacgcgccgtgccgtcgtaagctcatcggcgggatggagtttgccgaggtgacgggcgtgagtctggaccgcatcgccgtcaacgctttcaacaccaaccgcgttatcaatatgaaggccgcgctctcgtccatcgccgcgtcgggtctcggcgtgcgcgcgccgcggcttcccaagaacatgacccacagttttgtgatgtacaagcacacctttaaggagcccgcttgcaccgtcagcacctttgtttccaacgacgccgtctacatcaactcgctcaacgtcaatattcgcggttcctaccccgagtttctgtactcgctgggcgtgtaccggctgcacgttaatatcgatcacttttttctgccggccgtggtgtgcaatagcaactcctcgctggacgtgcatggactggaggaccaggcggtgatccgctcggagcgcagcaaggtgtactggaccaccaactttccgtgcatgatctcgcatactaacaacgtcaacgtgggctggttcaaagcggctacggccattgtgccgcgcgtctcgggcgctgacctggaagccattctgctcaaagaactctcgtgcatcaagaacatgcgcgacgtgtgcatcgattacggtctgcaccgcgttttcacgcaactagagctgcgcaattcgtaccagatccccttcctggccaagcagttagtgctgtttctgcgtgcttgcctgctcaagctgcacggtcgagagaagcggctgcagttggaccgcctagtatttgaggcggcacagcggggtctctttgactacagcaagaacctcacggcgcacaccaagatcaagcacacttgtgcgctcatcggcagtcgtctagccaacaacgtgcccaagatcctggcccggaacaaaaaagtcaaattggatcacctgggccggaacgccaacgtgctgacggtgtgtcggcacgtggaagcccacaagatccctcgcacgcgcctcaaagtgttagtcgaggtgctgggcgcgttgcagagtatcagcggtacgccgcacacgcgcgaagtgatccaccagacgttgtttcgattgtgctcggcggccgcagccacatcgggcctgtgttcatcccctcccccattgtgtgtgtcctcatcttcctccgtcccctctgtcccaacctccgtcagcgttgacggcagttctgaacccacgtcgccgcgagcgcggtttgcatcacgatgatggaagccgcggccgctgccgccgcggcgtttcgtccggaggagcgtccgacgccgggttggcacgacgcggcgttgttaatggacgacggtacggtgcgcgagcacgcgtttcgcaacggaccgctgtcgcaactgattcgccgtgtgttaccgccgccgcccgacgccgaagacgacgtggtttttgcatccgagctgtgtttttattgcagcggtcgttttaaccgcaggtcgtccgtcttctccatctattggcagaagcatagcgatctggtgtacgcgcttacgggcattacccattgcgccaagttggtggtggaatgcggtcagttggggagtagtaggctacggtggcgcgacggtgatgcgagtggtgaggagcgccggggagacgacgacagcagggacgagctgtacgacgtgccgggcatttatatgattcgcgtcaacgacggcggcagcaccggtcccagacacgttatttggccgggtaccagcgtgctttgggcgccggacgttgtgatcactacggtgcagcgacgaatctcggcggcgcgcgccctggtgaacacgttccgccaatatttttttttgctggaacggcgctcgcacgaggagctggttctttgtccgcccgagatggaggagcgtctagcgccgttgttgcagagtgccacgcgcggtgattcggacatgtttgacggtgtggtggccagcgcttatcaccgtttgcgaatgagtaatattccgcgttcatccgcccgtctgctggagcactgcgtggggctggcgggtgctaagaagctgctcttgctcgacgtgccgcgtctggagaactattttctttgtcaggtctgtctttacgagctggacgaggacgagatgggcgaggagatgctgggcatgttggccggaaagcccgaggatgccgccgtctcgggcgcaagcggcggttttctgctacatcgcaagacgatgaagctggccgcctgtctgtgtttgttgctcaattcgctgcatttgcaccaggaggcgctggaggccttggatcctccgccgccgcgcgtcgaggagaacgaccttgtcaacgtggtgctgcgccgttattatcgcagtcacggcggcgtgcaggcgcggacgctggcggcggcccgggctttgttagccgactacgctgaaacgttttcgcctttggggagttttacgcgcctgggttacgatcgtctcgtttctgccgatgccggcgtcagtcgccggcacctggtggctctgctgcgtgcctagctgaccctgaaacggatggcgtgtatatcgtcacacaggtaggtggccatgatgacggcgatgataagatcgtccgagatacgattctggcgcttggccgagtagcgtgccgtcgtgccttcggccagcgtgacgcggtgcaggttctgaatctgctccagaagatactcgatggggtcgtggctcagcttgatggtgtaggagacgagctcttgcgaggctttgatgtagcccgagttgaaacgcgagatgaactgttccacggccagcgccttgtcgcggcccatgaggtagaagggctgttcgatgtggttctggtcgggcgtgtggtagaagagcacgcggatgagcgtgctgctctgcacgctctgtcggatgaggcaggcgatgcgcacggccgccgcctggttggtgttgccctccacggcgatacgcagttcgtccaggtaagggtgcaggctcagcaccgagatgatcatgtgcgccgcgcactcggcgatggctacctcagaactctcggagaggtcgcgcaaaaagaaatgctctaggccgtaaatgagaaactggtgtcggtaggcgcctacggccgccacgcccgtgcccgaggccttgcggttggtggtgaaggccgggtccagatacacgtaaagcgtcttgccgaaataatcgtaggcgttggtgttgagcgtgctgtaacgcaaaatatcgaactcttcgcggctctggtccgtgatgagcacggtgttctgcgagattttattggtaccgccgatgatctcgtccatgaaagcgcccggcataaacatgttggccgtcttgcgcacctgcgagttgaggctgatgaaggtgggcttgtgcagtcggtagcaaggacacgccgtggcgtcgcccttctccgtgaagctgtgcaggtgctcttcgcacacgtaagagaccacgttgagcatgtcaaagggcgcattgttgaggcgcgtcaagaaacacgtggcgtcactggtagtgttggtggacgatatgaagatgatcttggtggtattctgggccaggaaccccagaatggtgttgaaggcctctttcttgatgaagtgcgcctcgtccaccagcagcaagtggaagttttgtcctcggatgctctgtgtagagaggagacagaaaagggactcttataattacgcacgctcggctggaagcctacagagtcggggtggggccggacaggtgagccaggtgagccgccaggtgaggcgggatcaccgtgtgccaaccgggctgcgacctgaaaaccggaaccaatccgccgacaccggcgccgcgtgacgcgcgcccataaaaacgaaagtgtcgtcgtcgcgacccgccacagccgccatgaactcgttgctggcggaactcaaccgactgggggtcgcgcacgccactacggaggatgtttttatctttgtcgaccgcctctttcaacacttttccttccttttccaggccgaggagtcaggcccgcgccgcttggaactggtcgcgtccgtgttcgagcacctgacggtggagtgcgtcaacgacatcctggacgcctgcagccatccggacgtgaacgtcgcggagacaagcaacacctgtcgtccctgcccttctcctgccccctccgcccccaaaactgtcagcgacgctcagacgtcatgtgcgacgcctcgggcgcctgtgacatgaggcacgtccagaacgcgtttaccgaggagatccagttacattcgctctacgcgtgcacgcgctgctttcgcacgcacctgtgtgatctgggcagcggctgcgcgctcgtctccacgctcgagggctccgtctgcgtcaagacgggcctggtatacgaggctctctatccggtggcgcgtagccacctgttggaacccatggaggaggcctcactggacgacgtcaacatcatcagcgccgtgctcagcggcgtgtacagctacctcatgacgcacgcaggccgttacgccgacgtgatccaagaggtggtcgagcgcgaccgcctcaaaaagcaggtggaggacagtatttacttcacctttaataaggttttccgttctatgcataacgtcaaccgtatttcggtgcccgtcatcagccaactttttattcagcttatcatcggtatctactcaaagcagaccaagtacgacgcgtgtgtcatcaaggttagtcgtaagaagcgcgaggacgcgcttctgaaacagatgcgttccgaatatggaaacgcacctgtattcggatctggcgtttgaagcgcggttcgctgacgatgagcaattgcctctacatctggtgctcgaccaggaggtgctgagtaacgaggaggccgagacgctgcgctacgtctactatcgtaatgtagacagcgctggccgatccgcgggccgcgctccgggcggagatgaggacgacgcaccggcctccgacgacgccgaggacgccgtgggcggcgatcgcgcttttgatcgcgagcggcggacttggcagcgggcctgttttcgtgtattaccgcgcccactggagttgcttgattacctacgtcaaagcggtctcactgtgacgttagagaaagagcagcgcgtgcgcatgttctatgccgtcttcactacgttgggtctgcgctgccccgataatcggctctcaggcgcgcagacgctacacctgagactggtctggcccgacggcagctatcgtgactgggagtttttagcgcgtgacctgttacgagaagaaatggaagcgaataagcgcgaccggcagcaccagttggccacgaccacgaatcaccgtcggcggggcggactgcgtaataacttagacaatgggtcggatcgccgtttgcccgaagcggctgtggcttctctggagacggccgtcagtactccattttttgaaattccgaacggagcaggaacctcctccgcgaacggcggcggcagattcagtaacctggagcagcgggtagcgcgtttgttgcgcggcgacgaggaattcatctatcacgcgggtccattggagccgccttccaagatacgcggtcatgagttggtgcagctgcgcctggacgtaaatccagacctcatgtacgccaccgatccgcacgaccgcgacgaggtcgcgcgtacggacgagtggaagggtgccggtgtctcgcgtctccgcgaggtctgggatgtgcagcatcgcgtgcgcctccgtgtgctgtggtacgtcaattccttttggcgcagtcgcgagctgagctacgatgaccacgaagtcgaactataccgggcgttggacgcttatcgggcgcgcatcgccgtcgagtacgtgctgattcgcgccgtgcgcgacgagatctacgctgtactacgacgggacagcggcgcgttgccacagcgtttcgcctgctacgtgccacggaacatgtcctggcgcgttgtttgggaactttgccgtcatgccttggcgctctggatggatcgggcggacgtgcgtagctgtattattaaggcgctaacgcctcgtctgagccggggtgccgccgctgccgctcagcgagctcgtcgccagcgcgagcgctcggcgcccaaaccgcaggagctgcttttcggaccgcggaacgagagcggtccgcccgccgaacggacttggtacgctgacgtggtgcgctgcgttcgcgcgcaagtggatttgggcgtggaagtgcgcgcggcgcgttgtcctcgcaccgggctttggatcgtccgtgatcgtcgcggacgcttgcgacgttggctctcgcaggccgaggtgtgcgtgctctacgtcacgccagacttggacttttactgggtgctgccgggcggctttgccgtctcttcgcgcgtcactcttcatggcttggcgcagcgggctttgcgagaccgattccagaactttgaagcagttcttgcaagaggaatgcatgtggaagctggtcggcaagagccggaaacaccgcgagtatcgggccgtcgcttgccgttcgacgatctttagtccggaggacgacggctcgtgtatcttgtgccaattgctgttgctctaccgcgacggcgaatggatcctctgtctttgctgcaacggccgttatcaaggccactatggcgtgggccacgtacatcggcgtcgtcgacgcatctgtcatttacctaccttgtaccaactgagcttcggaggtcctttgggtccagccagcattgatttcttgccaagctttagccaggtgaccagcagtatgacgtgcgatggtattacgcccgacgtgatttacgaggtctgcatgttggtgccccaggatgaagccaagcgcatcctggtcaagggtcacggtgccatggacctgacctgtcagaaggcagtgacgctaggcggcgccggcgcctggttgctgccgcgtcccgaaggctacacgcttttcttttacattctgtgctacgacctgtttacctcatgcggcaatcggtgcgatatcccttccatgacgcggctcatggcggcggccacggcctgcgggcaggcgggttgcagcttttgcacggatcacgagggacatgtagatcccactggcaattacgtgggttgcacccccgatatgggccgctgtctttgttacgtgccctgtgggcccatgacgcagtcgctcatccacaacgatgaacccgcgacttttttctgtgagagcgatgacgccaagtacctatgcgccgtaggttctaagaccgcggcgcaggtcacactgggagacggcctggattatcacatcggtgtcaaggattctgagggccgatggctgcccgtcaagaccgatgtgtgggacctggtcaaggtagaggaacctgtgtcacgtatgatagtgtgttcctgtccggtgcttaagaacctagtgcactaacggggtctgacagttcacggggagaagaaacaagaaataacaaaaaaaaaaagaggacatggactcgccacggtttgtggcaaggcgtatgttatcatcatggagctactcacgttggtgttgtagcaactggcaaaaagcgccgtgctcttggcgccgcggtggtcgatgctgatcacgttgtccttgttctcgaccacgtagtcgcgcgcgaaggtgtggcggcagcggaactcgacctctttgagcacaaactgcgacacgtgcttttggtgcgccacgtagccgatgctgatgccgatcatgtgcttaagcagaaacgagataatggggatgatgaaccaagtcttgccgtgacgtcgcggcaccaggaacacggtggctttctgcttaaagatgtcgatggaggtctgcgagaggaagtcgatctggaaggcgtggatgaggtactgcagcacgcgattggccagcacggggatcttggtcacggctataaaaaagatgacgtgtatcaataaattcttttgaaacggttcgagtcggatggcttttgcgtcgccctcgacggcggtactgaagccgccgtcgagccactttttaaagtcggtcatgaagttgttgatctgctgaaactgcggatcgcggtagagctcggtcaacgcgtccagcttctggtaggaggcgcgctgctcctcggagcacgggcgaaacgtcagttcatcgagcgcgctcttgaggcgctcgtgaaacagcagctcgcgctggctttcctcgggcgagttgtagtcgcggtggcggccgcagaaggccatgagcggcaggaaggcctcgttgcacgagtgggccagcccgagttcggggtgcatcatctggtagcgcttgcggcacagcgccgccacattggtgaaggccgtggagatgcaggaggtggggtggctcttgcgcttctgcagctccgcgtagcgctcctggatcttggcggccgaatctccgcgcaacatgatggcggcggcggtggtgcgagcggaggttaggcggcagcggcgagaggagaggaaaaagatggcgtccgcgaggacgacggaggatccacccgaaaaccacgttgtcgcggacgtggcttgtgggacgggcgccgtcactcgttcgtcttcgtcgtccttagtggtgtcgtcctcctcggcgtcaggctcagacgaatcttcatccgcctctcctctcagtttccccgtctcctccccctcaactgccgtcaggtctccggggtccgccggggtttcaacgtccctgtgctcggtggaacggatggtcgagctgtcggcgcagtctccggccgccgatttctcggtctccgaggcttggcgcttcgaggaggccgtaaatatggcgctggtggcctgcgaggccgtgtcaccttacgatcgctttcgcctaattgaaacgcccgacgagaatttcttgttggtcactaacgtaattccgcgcgagtcggccgaggtgccggtgttggatagcagtagcagcggtggcgatagcgggccggaggacaaaaagaaaaacgtcgggaataaaaccgcgggggaaaagaacggcggtgggtctcgggccaaacgccgtcgtagacgacgcgctccgaaaaacgacgccgccacgccgtcttttctacgtcgacacgacgtgctggagcgtttcgcggccgcggctgagcctttgccgtcgctttgtgtgcgtgattatgtgttacgcaatgctgaccgtgttacctacgacggcgaattaatctacggcagttacctgttgtatcgcaaggctcacgtggagctgtcactctccagcaacaaggtgcaacacgtggaagccgtgctgcgacaggtgtacacgccgggcttgttagatcatcacaacgtgtgcgacgtggaggccctgctgtggctgctgtactgtggaccgcgaagcttttgcgcgcgtgacacctgtttcggtcgcgaaaagaacggctgtcctttccccgcgttgttgcccaaactcttttacgaacccgtgcgggactatatgacctacatgaatctggctgagctgtacgtctttgtttggtatcgcggctacgaattccctgcgccgacgccgcaggcgacgacggcgggtggtggtggtagtggtggcggcggcggggccggcgcttgtgcggtcgagacgagcgcgtcagcaggccgggtcgatgacgccggcgacgaggtgcatttgcctttaaagcccgtctcgctggaccgtctcagagaggtattgcaggcggtgcgcggccgcttctcggggcgcgaggtgcccgcctggccggcctcgtcgcgcacctgtttgttgtgcgcgctctacagtcagaaccgtctctgtttagatctcgcgcgtgacgaggcgcggaccgtgagttatagccccatcgttatccaagactgcgccgcggctgtcaccgacgtcactttgagccacatcttgcccggccagagcaccgtctcgcttttccccgtctaccacgtcggcaagttgctggacgctctctcgctgaacgacgcgggtctcatcacgttgaatctatgacgtcggtcaacaaacagctcttaaaggacgtgatgcgcgtcgaccttgagcgacagcagcatcagtttctgcggcgtacctacggaccgcagcaccggctcaccacgcagcaggctttgacggtgatgcgtgtggccgctcgggaacagacccgatacagtcagcgaacgacgcagtgcgtggccgcacacctgttggagcaacgggcggccgtgcagcaagagttgcaacgcgcccgacagctgcaatccggtaacgtggacgacgcgctggactctttaaccgagctgaaggacacggtagacgacgtgagagccaccttggtggactcggtttcggcgacgtgcgatttggacctggaggtcgacgacgccgtctaacaggtatagcaatccccgtcacgcctctgttcatattttattaaaaaaaaacacaacataacgacagtgtcggtgtggtagctagtgcagccctaggaacagggaagactgtcgccactatgtcctccgcacttcggtctcgggctcgctcggcctcgctcggaacgacgactcagggctgggatccgccgccattgcgtcgtcccagcagggcgcgccggcgccagtggatgcgcgaagctgcgcaggccgccgctcaagccgcggtgcaggccgcgcaggccgccgccgctcaggtcgcccaggctcacgttgatgaaaacgaggtcgtggatctgatggccgacgaggccggcggcggcgtcaccactttgaccaccctgagttccgtcagcacaaccaccgtgcttggacacgcgactttttccgcatgcgttcgaagtgacgtgatgcgtgacggagaaaaagaggacgcggcttcggacaaggagaacctgcgtcggcccgtagtgccgtccacgtcgtctcgcggcagcgccgccagcggcgacggttaccacggcttgcgctgccgcgaaacttcggccatgtggtcgttcgagtacgatcgcgacggcgacgtgaccagcgtacgccgcgctctcttcaccggcggcagcgacccctcggacagcgtgagcggcgtccgcggtggacgcaaacgcccgttgcgtccgccgttggtgtcgctggcccgcaccccgctgtgccgacgtcgtgtgggcggtgtggacgcggtgctcgaagaaaacgacgtggagctgcgcgcggaaagtcaggacagcgccgtggcatcgggcccgggccgcattccgcagccgctcagcggtagttccggggaggaatccgccacggcggtggaggccgactccacgtcacacgacgacgtgcattgcacctgttccaacgaccagatcatcaccacgtccatccgcggccttacgtgcgacccgcgtatgttcttgcgccttacgcatcccgagctctgcgagctctctatctcctacctgctggtctacgtgcccaaagaggacgatttttgccacaagatttgttatgccgtggacatgagcgacgagagctaccgcctgggccagggctccttcggcgaggtctggccgctcgatcgctatcgcgtggtcaaggtggcgcgtaagcacagcgagacggtgctcacggtctggatgtcgggcctgatccgcacgcgcgccgctggcgagcaacagcagccgccgtcgctggtgggcacgggcgtgcaccgcggtctgctcacggccacgggctgctgtctgctgcacaacgtcacggtacatcgacgtttccacacagacatgtttcatcacgaccagtggaagctggcgtgcatcgacagctaccgacgtgccttttgcacgttggccgacgctatcaaatttctcaatcaccagtgtcgtgtatgccactttgacattacacccatgaacgtgctcatcgacgtgaacccgcacaaccccagcgagatcgtgcgcgccgcgctgtgcgattacagcctcagcgagccctatccggattacaacgagcgctgtgtggccgtctttcaggagacgggtacggcgcgccgcatccccaactgctcgcaccgtctgcgcgaatgttaccaccctgctttccgacccatgccgctgcagaagctgctcatctgcgacccgcacgcgcgtttccccgtagccggcctacggcgttattgcatgtcggagctgtcggcgctgggtaacgtgctgggcttttgcctcatgcggctgttggaccggcgcggtctggacgaggtgcgcatgggcacggaggcgttgctctttaagcacgccggcgcggcctgccgcgcgttggagaacggtaagctcacgcactgctccgacgcctgtctgctcattctggcggcgcaaatgagctacggcgcctgtctcctgggcgagcatggcgccgcgctggtgtcgcacacgctgcgctttgtggaggccaagatgtcctcgtgtcgcgtacgcgcctttcgccgcttctaccacgaatgctcgcagaccatgctgcacgaatacgtcagaaagaacgtggagcgtctgttggccacgagcgacgggctgtatttatataacgcctttcggcgcaccaccagcataatctgcgaggaggaccttgacggtgactgccgccaactgttccccgagtaaccgggacgcggaacgtgacggttgctgaggggaaaggcaacagagaaggtacaaacccaccggcggggaaaataccgaggcgccgccatcatcatgtggggcgtctcgagtttggactacgacgacgatgaggagctcacccggctgctggcggtttgggacgatgagcccctcagtctctttctcatgaacacctttttgctgcaccaggagggcttccgtaatctgccctttacggtgctgcgtttgtcttacgcctaccgcatcttcgccaagatgctgcgggcccacggtacgccagtagccgaggactttatgacgcgcgtggccgcgctggctcgcgacgagggtctgcgcgacattttgggtcagcggcacgccgccgaagcctcgcgcgccgagatcgccgaggccctggagcgcgtggccgagcggtgcgacgaccggcacggcggctcggacgactacgtgtggcttagccggttgctggatttggcgcccaactatcggcaggtcgagctcttccagttgctggaaaaggaatcgcgcggacagtcgcgcaactcggtgtggcatctgttgcgtatggacacggtctcggccaccaagttctacgaggccttcgtcagcggctgtctgcccggcgccgcggcggcggacggttcgggtggcggcggctcgcactacacgggctcgcgcgccggcgtctcgccgggcatccagttcggtatcaaacacgagggcttagtcaaaacgctggtggaatgttacgtgatgcacggacgcgagccggtgcgcgacggcctcggtctgctcatcgaccccacgtcggggctgctgggcgcttccatggacctgtgcttcggcgtgctcaagcagggcagcggtcgcaccttgctggtggaaccgtgcgcgcgcgtctacgagatcaagtgccgctacaaatatttgcgcaaaaaggaggacccctttgtgcagaacgtgctgcggaggcacgacgcggcggccgtggcctcgctgttgcagtcacacccggtgccgggcgtggagtttcgcggtgaacgcgagaccccgtcggcacgcgagtttctgctttcgcacgacgcggcgctcttcagggccacgctcaagcgcgcgcgcccgctcaagccgcccgaaccgctgcgcgagtacctggccgatctgctgtatctcaataaggccgagtgttcggaagtgattgtgtttgacgccaagcacctgaatgacgacaacagcgacggggacgccacgaccactattaacgcgagtctcgacctagccgcgggcgacgccgctggcggcggcgctgatcaccacctgcggggcagcccgggcgattcgccgccgccgatacctttcgaggacgaaaacacgcccgagctgctgggccggctcaacgtgtacgaggtagcgcgcttttcactgccggcttttgtcaatccgcgtcaccagtattactttcagatgctcattcagcagtacgtgctcagccaatactatataaagaagcatccggacccggagcggatcgatttccgtgacctgcctaccgtctacctggtctcggccatcttccgcgagcgcgaggaaagcgaactgggctgcgagttgctggccggcggtcgcgttttccactgcgaccacattccgctcctgctcatcgtcacgcccgtggtctttgaccctcagtttacgcgccatgccgtctctaccgtgctagaccgttggagtcgcgacctgtcccgcaagacgaacctaccgatatgggtgccgaactctgcaaacgaatatgttgtgagttcggtaccacgcccggtgagcccctgaaagatgctctgggtcgccaggtgtctctacgctcctacgacaacatccctccgacttcctcctcggacgaaggggaggacgatgacgacggggaggatgacgataacgaggagcggcaacagaagctgcggctctgcggtagtggctgcgggggaaacgacagtagtagcggcagccaccgcgaggccgcccacgacagctccaagaaaaacgcggtgcgctcgacgtttcgcgaggacaaggctccgaaaccgagcaagcggtcaaaaaagaaaaagaaaccctcaaaacatcaccaccatcagcaaagctccattatgcaggagacggacgacctagacgaagaggacacctcaatttacctgtccccgcccccggtcccccccgtccaggtggtggctaagcgactgccgcggcccgacacacccaggactccgcgccaaaagaagatttcacaacgtccacccacccccgggacaaaaaagcccgccgcctccttgcccttttaactcataaactttcaggtctcgcgtacgattcgcgagtcgggaatgggacacccgtgggtgtttctccgtgtgtatattatttttttttgtgtgtgtgtgtgtttgcgcccccgtgtgtctaatgtgctgtttgaaacacgtaaagtagctggtggaagaacagataaacctttaataaaaaaaaagtatgtgctcccgacccacggtctgcgtgtctcttttttatgtccatgtctccaagtctggtgcgggtggcggcggggtcaagcgtcctcgaagtcttcatcatcgtcgtcgtcctcttgttcgcggaggcgacggctttccaagctgtcgtggtgactgagcgcagcgacttcttcgccggaggctgtggccagcgcctggtacttgacactgccgctaccgcgtccgcgaaagtagcggacggcgcgacacgtcgtaaacatggcccatatgaaaaagagcatgccgaacgaccagctgatgccggtgcggtattcgttgctgaggaaggtatcgtactgcacgatggggtagatgaggccgcagagtccaaagaaggcgcccaggtggtagccgaattgcaccttgacgtattgaaaaaagacggcctcgatcagtaaaaagtagatgatggagatgatagcgtagaccacgaagacggctaacaccatgtggcctgtacgcacgaaaaagttgtttccgaagccgtagcacagggccatggctaccacggtggtgttgaaaccaagcgctacctccaccaggttgacgatgagcgtgcggaactgcaccgtacctttgagcttggggtgcagacgcgagaagaaaaagagtgagcgtttgtagctgcggtactgcgtgaccatgctcacgttgaaaatggtcaggcagaaaaagtgcacggcggccatgaaggcgatcatgctgggcagccgaaatgacatggtcagtgtgaatagttggaacgtgtccatgctgagaatgaagaggaaggctgtgaggctgtcgcccatgtacgaaatgtcgcgtgtcgactggtttaggctcatgcctttgtccttgcgcatgctgatcttgatccagcataccaggtagtagatggtcacggctaaaaagacgagctgcatgaacacggcgtagcacaccaactgcaccgagtctaagaaaagcataggcgtgtgcaggtgcattacgttgtaggccgacatgttgagcctttcaaagtccacgacgtgatagtagacgcaggggtagcccaggtgcggaaaattgctcagcactagatgcacgctgacgttgacaaaagtgagcaccatgaaaacgatagaagcgctccatgtccgtgtattcactttatccacgtgcgagggggccatggcgatagcggcggcccgctcgctcgggaggcgatgggggcgcgccgatgacgacaggctcgcgggtcgttaaatactacgatgggagccgccgcggctcacgacgcggtttgagcacgtccgggcgatcggtgaaaaaagaccccgcgggccttcgcgactctcttctgtccgaggatgaccgctcagccgccgctgcaccaccgccaccacccgtacaccctgttcgggaccagctgtcatctcagctggtacggccttctggaggcctcggtgcctatcgtacaatgtctgtttttggatctgggtggcggccgtgccgagccgcggcttcacacgttcgtggtgcgcggtgaccgtctgccgccggctgaggtgcgtgctgtgcatcgtgccagctacgccgcgctggcctcggccgtgactacggacgccgacgagcgccggcgcggcctagagcagcgtagcgccgtgttggcgcgcgtgttgctagaaggcagcgcgttaatccgcgtgttggcgcgcaccttcacgccggtgcagattcagacggacgctagcggcgtggagattttggaggccgcaccggcactgggcgtggaaaccgcagcgctatcgaacgcgcttagtcttttccacgtagccaagctagtggtcatcggctcgtatcccgaagtgcacgagccgcgtgtggtcacgcatgccgcggaacgcgtctccgaagagtatggcacccacgcgcacaaaaaattgcgtcgcggttactacgcctacgatttggccatgtcgtttcgcgtcggcactcacaagtatgtgctggagcgcgacgacgaggccgtcctggcacgcctctttgaggtgcgcgaggtgtgttttttgcgcacctgtctgcgtctggtcacgcctgtcggtttcgtggccgtggcagtgaccgacgagcagtgttgtttattgctgcagtcggcctggactcacctttacgacgtgcttttccgtggtttcgctgggcagccgccgttacgcgactacctggggccggacctttttgagacgggcggcgcccgttctttcttttttcccggtttcccacccgtgcccgtctacgcggtccacggtctgcacacgttaatgcgcgagacggcgttggacgcggcggctgaggtgctctcgtggtgcggcctgcccgacatcgtgggctcggccggcaagctggaggtggaaccctgcgcgctctcgctcggcgtgcccgaggatgagtggcaggtcttcggcaccgaggccggcggcggcgccgtgcgtctcaatgccacggcttttcgcgagcgaccggccggcggcgatcgtcgctggctgttgccgccgctgccgcgtgacgacggcgacggtgaaaacaacgtcgtggaagtcagcagcagcaccggcggtgcgcacccgccgagcgacgacgctactttcaccgtgcacgttcgcgacgccacgctacatcgagtgctcatcgtggatttggtcgagcgcgtgctggccaagtgtgtacgcgcgcgcgacttcaatccctacgtgcgttatagtcatcgactccacacttatgcggtttgtgaaaagtttattgaaaatctgcgttttcgctcgcgacgcgccttctggcagatccagagtctgctgggctacatctccgagcacgttacgtcagcctgcgcttcggccggccttttgtgggttctgtcgcgtggacaccgcgagttttatgtctacgacggctattcgggtcacggacccgtctcggccgaagtgtgcgtgcggactgtggtcgactgttattggcgcaaactttttggcggcgacgatccgggtcccacctgtcgtgttcaagagagcgcgcccggcgtgctgttggtttggggcgacgagcggttggtgggtcccttcaacttcttctacggcaacggcggcgccggtggtagtccgctccacggggtggtgggtggtttcgcggcgggacattgtggcggcgcttgttgcgcgggctgcgtcgtcactcaccgccattctagcggtggcggcggcggtggtggtggcgtgggcgacacggaccacgcgagtggcggcggtctagatgccgctgccgggagtggtcataacggcggtagtgatcgggtttctccctccacgccgcccgcggcgttaggtggctgttgctgcgcggccggtggcgactggctctcggccgtgggtcatgttctgggccggctgccggcgctgttacgggagcgcgtgagcgtgtccgagctggaagccgtgtaccgcgagatcctctttcgcttcgtggctcgccgcaacgacgtggacttttggttactgcgcttccagcccggtgaaaacgaagtaaggccgcacgccggggtgattgactgcgcgcccttccacggcgtgtgggccgagcagggccagatcatcgtacagtcacgcgatacggcgttagcggccgatatcggctacggcgtctatgtggacaaggcctttgccatgctcacggcttgcgtggaggtctgggcgcgagagttattgtcgtcctccaccgcttccaccaccgcttgttcttcttcttccgttctctcttccgccttgccgtccgtcacttcgtcctcttcgggcacggcgacggtgtctcctccgtcttgttcttcttcgtcggcgacttggctcgaggagcgcgacgagtgggtgcgttcgctggcggttgacgcgcaacacgctgctaagcgggtggcttccgagggcctgcggtttttccggctcaacgcttaacgagtcacgtaggggaactacgtgggtaagtgacgtggatactagtaaaaaaagtgcgtcaaagttctcagcgtgtgacgtggatactagtaaaagggacgtcaaagctcactacgtgttgcgtgttttttttttttctatgatatgcgtgtctagttcgcttctcactcttcctctccccgttcccagcgcggtggcagcttggggggtgagggcaaattggggtagttggcgttgagcacgtctagcaggcccaggcccacgggccaaccgtccacggtcttacgctcggtcagcttgaggctaaacgagtgtgcctcgtcttgaccggtaaggcggaaaaagaagcgtgctaccagctgcaggcaggtatgccgcgtctgctggaagagcacgaaggtagcgggcacgtactgcacaatgtgcggttctttttcctcaaagagtaggtagagcgcgctgcagatcagccgccgggcgctgtggtgcagcagccggccgaagctttcgcgcacgttcactgcgtccaggtactggagcaggtcgtgcaggcacttgcgcgttaagttgcaattttccacgcatgaaataacggtacagagcgcgaagtgcagcaggttgtcggccttgacgatgccgcagcggtgtttgagccgcagatccgagagcctcacctgcgtgacgacgtcttcggtctcgagcaaaaacacggcggagtagcccagaaaggccgaggtgcacagcaactcgctgcggtactcggccatggaaaccagcagcccgtgctccgtgtgcagccacagcttgtcgccgcgcaccgtaaagtcgagcacttgcggctccatgatcatcacattctgtctagtgaaatccgtatggacctccagcacgccgcggatcatcagggcctccatttcgaaatcggccgacacgctctgggccgcgccgctcctcgtctgccgtgatcaagcggcgcggcgcggacctttcaagcgttcctgggccgccgctcgaggcagttcccctttctggcactccgcccgccgcttcgcggctcatttggcgccggcgcgccttctcgcggctgcaaatcagctccacgtatcggcaaaacttgctgtcgtcgtaggcggcggccacgatctcgccgaaggagagctgcaggtaggcttcgggtacggggtccagcgtgcctagcgccaggatgtgacacagatagggcagggtcacgcgctctaccgtgtaattggagtagacgatggcctcttcggccccttgatgcgtgaccagacgccgtaggcgaaaggtgcggaaatactcgttttcccacaactgcgtgaggaagcgttctagcgactcggtgccaggcacgaactgcgagaagaagctgttggccaccaggcggttgtcttccaccgccagcggacggaagggcgccgcgtcgcgcgccttgcgcacggcctccaacacgggcaggtggtagagttcggcgtcgcgcgcgcccaggctcatggagtcctcgcgccgcgaggcgtagcgcgtgagcaggtcgcgcagctcgcgcacgcgattctcccaggtctggttgagcgtgcgcaggtcctggatctcgtccacctgcgactggatctgctcctccaggcacttgatgacctgcttcttaaacaggtcgcggatgtcccgctcgggcgccgccgggccgggtggcggcggcagcagcccgacgtggcccgcgggtcctcccaccacggcgccgccgggtcccaccacgccgggtccacccggaccacgcgcgggtagtagacggttttggtccaccagcgagggggtcaggtcctgcagaaaggactcgacgctgtcctcgatgccgatgcgcgatttgctgtccgagacgttaagcaaaaacttcataatggactttttggcgtcgctgccccggtcgtgctgctccatcatctccaccagcttcttgcagttgagctcgtggcggctggcggtcaccactttcacaggaaaggtattgagcagctggcagatcttttggtggcggcagagcccgtcgtagcgcagaatctcctcgtgcaggtgtgccaccggcgtggtgaacagcagcttgtcgcgctcataagccagcggttcggccgccacgtacaagcggatgtgcttgccgcgcagctgcgcctccagccgctccgagcgcaccttcttgaagacgcgtacctcgggcgcgttggctacgcgcacggcgcccaggcgctcggccacctgcagcagcagcgccaggttagcctgcagcaggtcctgcgccagcgggtgtgtctcggtggcccgctgcacggccgcgcgtacaaattgcgcccgctcggccgcctcgctcggcttggttttcacgtccagcagcggtaccagtcccaccgttacgcaccaatccacgtagagaccatagtcgtcgttatcggcgtactgatataaaatgtcgcggagcgcgcccagcacgcccgtttgcacgctctggcgcaacgaggcgctccacaccaacagatactgctccaggtcctcttcgtccagcgcgcggtagggaaacagcgccgcgtgtaacttccactcctcggccacgcgccgcaccgtgatggtgtcaaagagcgtcttgcacactccgtagagcagctgcttgcgcagcacgcacgggtcgcgcagcacctggtgcatgctctggccgcgacacgtccccagaaagccgtgcagcaaccgcaggaagctcatcgtctggcccgtggggaaaatgtcgatgacggcctcgtcatccacgccgcggcccacgcccaagtacgacgacgccttgatcctcaacctctcgtcggctgccaagatcgaacggatcgtcgacaaggtcaagtctctctcgcgcgagcgctttgcgcccgaggatttttcgttccagtggtttcgctccatcagtcgcgttgaacgaacgacagataacaacccctctgccgcaactaccgccgcggcaacgacgaccgttcactcctccgcctcctcttctgccgccgctgccgcttcgtccgaggccggcggcacgcgcgtaccctgcgtcgaccgttggcccttctttcccttccgcgcgctgctcgtcaccggcacggcgggcgccggcaagacttccagcatccaggtgctggcggccaatctagattgcgtgatcaccggtaccacggtgatcgccgcgcagaacctcagcgcgatcctcaaccgcactcgctcggcgcaggtcaagaccatctaccgcgtcttcggtttcgtcagcaagcacgtgccgctggctgatagcgccgttagccacgagacgctggaacgctaccgcgtgtgcgagccgcacgaggagaccaccatccagcgcctgcagatcaacgatctgctcgcctactggccggtcatcgccgacatcgtggacaaatgcttaaatatgtgggagcgcaaggccgcttcggcctccgccgcggccgcggccgccgcctgcgaggacctctcggagctgtgcgagagcaatatcatcgtcatcgacgagtgcggccttatgctgcgctacatgctgcaggtggtggtgtttttttactacttttacaacgccctgggcgacacgcgactttaccgcgaacgccgcgtgccctgcatcatctgcgtcggttcgcccacgcagaccgaggcgctggagagccgctacgaccactacacgcaaaacaagagcgtgcgcaagggcgttgacgtgctctcggcgctgattcagaacgaggtgctcatcaactactgcgacatcgccgacaactgggtcatgtttattcacaacaagcgttgcaccgacctggactttggcgacctgctcaagtacatggagttcggtatcccgctcaaggaggagcacgtggcctacgtggaccgcttcgtgcggccgcccagctccatccgcaacccctcgtacgccgccgagatgacgcggctttttctctcgcacgtcgaggtgcaggcttacttcaagcggctgcacgagcagatccgcctgagcgagcgccaccgtctcttcgatctgcccgtctactgcgtggtcaacaaccgcgcgtaccaggagctctgcgagctggccgacccgctgggcgactcgccgcagcccgtcgagctctggttccgccagaacttggcgcgcatcattaactactcgcagtttgtcgaccacaacctctccagcgagatcaccaaggaggcgctgcgccccgcggccgacgtcgttgccaccaacaactcctccgtccaggctcacggagggggaggatctgtcatcgggagcaccggcggcaacgacgagacggcgtttttccaggacgatgataccaccaccgcgcccgatagccgtgagacgctgctcaccttgcgcattacctacatcaagggcagttcggtgggagtcaactctaaggtgcgggcctgtgttatcggataccagggcacggtcgaacgtttcgtggacatcttgcaaaaggacacgtttatcgaacgcacgccctgcgagcaggcggcctacgcctactcgttagtttcgggcctgctcttctcggccatgtactacttctacgtgtcgccctacacgaccgaggagatgttgcgtgagctggcgcgcgttgagctgcccgacgtgagttcgctctgcgccgctgccgccgccacggccgccgctcccgcttggagcgggggagagaatccgataaataatcacgtcgacgcggattcttctcagggcggccagagcgtgccggtatctcaacggatggaacatggccaagaggaaacccacgacatcccctgcctgtccagccaccatgacgactcggacgccatcacggacgccgaactcatggatcacaccagtctgtacgcggatcccttttttctcaaatacgtcaagccacctagcctggcgctgctttctttcgaggagacggtgcacatgtacactaccttccgcgacatttttctcaagcgctaccagctcatgcagcgtctcacgggcggtcgcttcgccacgttgccgctcgttacctacaatcgccgtaacgtggtgttcaaggccaactgtcagatcagctcgcaaaccggctccttcgtgggcatgctttcgcatgtgtcgccggcgcagacgtacacgctcgagggctacaccagcgacaacgtgctcagtctgcccagtgaccgccaccgcatccaccccgaggtggtgcagcgcggtctttcgcggctggtactacgcgatgcgctcgggttcctctttgtgctcgacgttaacgtctcgcgcttcgtcgagtcggcgcagggcaagagtctgcacgtgtgcaccaccgtggactacggcctcacttcgcgcacggccatgaccatcgccaagagtcagggcctgtcgctcgagaaggtggccgtggactttggggaccatcccaagaacctcaagatgagccacatctacgtggccatgtcgcgagtcacggaccccgagcacctcatgatgaacgttaacccgttgcgactgccctatgagaagaacaccgctatcaccccctatatctgtcgcgcgctcaaagacaaacgcaccacgcttattttttgacacaacaccgtgtaagcaaaacgtgactttattgagcagggtaaaaaccacgtacaagaaccacgttgtctatccccccaaaaaaaaacacaccgtcagggaacacatcgcctatagatagcggcactttacataaaaccaccgtacctgcatcacggtggctcgatacactggaaattcaataaaaaccaccgtgtccacgttacggtacttgccgggtcagcgtccttctcttgagatttctgttcgcaaacttatccgtttccccggtccgcggtgtctcctcgcgaggctgacagtctacgagtggtatctacaagagaaagaaacccgggtgggagcgacgccgtcgctgggtatcaaccccgcggctgaccgtcgtccggtaaaggaacaacccgtcgtcgcaagccgggttcgaccaagagaaaaaaacccgggtgcggggggagacgggtcgtcctttggtcgttcgcggacggcgtacatgccgcgtgggtcagtcgacggcgtcgctccgtgcggtcggtcatcattctgcttcacatatatgggttgtttgtgttttttttataatgaatacgcactcatcctatccgtgactgcgcgtgtggcagagaggatgccttataacatgtattttgaaaaattgccaacagctataatttctctcatgtagcagaatagagaccttttgtcgtctttttgtttgtcattacttgttttccagggaattagagagagggaaccgcgcctccggcggcggtgcccgcggaccccggccccttctcgcgtgcgcggtgtgactggttgagcgaatgagcagctaggcttggtggtgctccgcgtgcgggggagaagacgattaacaacaaaaaataagtggaagtggccggtgggtctttgtccgcgtgcgcgcccatccgtcgccgggaccgagcagaaagtgatgtggtggtacattgattttttccttgacaggaaagaaaaaaaagagttttgttttcctatgtgagaggagaaaggtatgtgaggagatgttcgatgatcgtatgttacagttatgctgtaaggaagcttttatcgtgcgtcctgtttttcatttgatgtatatgacacaattgaaacctatcgataggcgtatatcgaggattcatcaattcttagaatcgtcgtctttttggctaattggactttgcccatgttggttgtcattcgtggcctgaggtcatcgtcgtccacgacgacgtgtctatagcgtgcggtgtgatcattgtgtcgagccagagaaagcgcgcctcgcacgacgtttgcggatcggctcgcgggtgtgtggaattcctaagaacataatcagctggtcgtctttctttgatgtgttgttgtcgtcgaggtcttgcttcgttttcttttttctttttagtcgatggaacttttcttcggtacgggttcttgttatggaagcttgtgttttcgaacatgaattcgaaaaaataaaaaggcctatcttcgtttcaaaaaaaggacagatatcaatcttcttaacttatatcatggtaaattcagaatcctatggtgtcttattatctctaaagtagtcaacattatggtctaacttgtatttccctgacgagatatatatgatccttataacctggctactatcatgaacaacaatatccttacttacagtcatcttcgtgagttaatgaagtataatatcggtcatctatcaacttatctgctatgtaacgtacccttttaggtattttgcgtttcttaacgagtgtacccgcctgtgtgaggcgaaactctgagaagtctaccgagtcgagttacaagtcactaaaacacttacacgagttatctatactaaaatcactatctatgttgtttgcttacctaattattatcctacatgacgaagctacctcccaacgtaaggtagggggagaggagacagaacaataaaaagtaactaatgtttcttagaacttacccgctaaggacttaccaaactatattcaccaaaaaacaacagctacgtgtttcatttgttttaatctaccgaagtaaaaaaaaaaaagatgattagctatccagaacctacttacttcttaatgttttaactaaggatgcctatgggattggaaaaaaaatcacagcaacttgctactaatcagttgacagcgaagagactcataacaaagatttctgggtaatacggttataataatgcttatggactaaaggatacttggaaaaaaagaacgggctatgactatagagattcgtcgagatattaaacttcaaataggcggctatcattcatggttgtggtgactatatcgtggagaaaaaatgtgatcgttagttagctaggtgagacttacagctatccatccgtctagtttttcgttgtaatgatgatagtacgtctatggtggtgatcgattttggttaacaatttgttcgtttaaaggcttaatgtacttatgctacatgatgtattattctttgattcatcgttcctcctaagggggtgtatgtatgtatgtactagtcgtatagtgttcctaacatcatgattattcagactatggcttcatctatcgtgtctaaagttcacttattctactattactatatatatgcactactatgtaactaggatatggtcctataaggtgtcttctatcacggtggcttgtttatcgcttggcggttacgagcaagagttcatcacggaccagccgtgaggcagggcacacgcgggtcggcggcgatgatgtcccccgcgaaggggacaacaaaaacaagacaagaggccgccggccgcggccacggacgcgtagcggttacacaatgtttggttgagcgttttgtttcatcgtcgtggtggtggttttgttgttctctgtatatatcgtgtggtggctttatcgtcatcattattatcatcattcttgtttccatcatcacgatgagttttctccgttttcctctcctccagtggtagtcgtgtatcatcatcaatcatcgtagtgacgtcgttgctgctgctgctcttgccttcatggcggtatttctcttcctcccccctaaccccatattaactcgtgagtgtgatggttagagtggctgcttgtttttttttcttttctctttggaacaacaaaagaggataaagatggtcggtgaatgtattattattattatcatcattatgatacggtcgcggtcttcttctccgatgacgaaacctgcgcacatcgaagaaaagacgagcgcgcgaaccgatagccgtccgtctgggacgaaggagaagatgatggggagaggaggagagccccagaagccagagcgagaagggagacgacagacatacgtcgtcaccgtcctctggaggaggcacggcggcgctgtttgttgtttggatgcttgattatatcctgttctatggggtagattattatcaataggcttggttttcaaaggtcagcctgtgtattgtcgtgtcttttttttcgttctcatgatcgcggagaccacacagacgtgcgcgtctcccaatggctaggcgttctttttaggtagtaattttttgatcttttttttttcttaacaagtctggcttgatttcttttatctatgatcgattcttctttttctcgggggttgcatcttccgtgaaagtaaagtgacactactctaaatggtaaccatattatctgttgattaggagaaaaaataattttttcgcacgaaatcgatcctaagtgaggtgatttacttgctatcacacgaaatgattatcttttgctgctaacgtactgaattttttaacagaattgcttctccgtaactatttccgcagattcagacagattgtcaaaaaaaaatacggcacagaaatagtgggtctgtggcttttggttcgtgtacattcgcgtttgcgtgtcgagatttctacggtatgtttattcttcctgcgatgatgtagggtccttggtgtaagtaggatttcgagtatctctcttagagcgaacaaaataatcaaaaaacaacagctaggaaatcgagggttactctacgataaagtgtctctacaaagtgaagaatgttacgttgtggtggaataataagactcgcgtgatcgatgagtgatcgagagcggctcgaaccttctttaagagctttgtttagtgcaactttaaattacaaggagtagaaagctgaaatgaatctatgaaggtgctattctttgaatatcttactttgtacgcttcacattcgttatttggatagagagttgtctagagaaaatctgtgattctctatgagtgttatttttattatccttttggggactacgatttttcttcttgttctacataccactactactcgtaatcacatacatggacgaaaaaaaaattcgtcaggcagtagataccagattctccgacgttacggcgtctttttttcttttgagagagtatctgctgagattgtccgtggtgtatctagtcgctatttttgttgttactagtagttttgcacacagtttattcagtataatttttcttcttgccatgatcaattgagcccaccaccttttttttttagagaggaggaatttcgtcttgatctccagccggagacaacggcggcggtggtggtggcgggagagatttcaaggcaatgaaaaaaaaaatttcgttttgccatcaagtggtgacgataacccgtcagattgataattggttcctacagaaactattctaaccgcggaagaaagaaattgaaaaaaaaaattgacaaaaacatcataacataaaggaccacctacctgggacgcgcagttgggcggcggactggggcggcatgctgcggcgatgctgtcggtgatggtctcttcctctctggtcctgatcgtcttttttctaggcgcttccgaggaggcgaagccggcgacgacgacgacgacgataaagaatacaaagccgcggtgtcgtccggaggattacgcgaccagattgcaagatctccgcgtcacctttcatcgagtaaaacctacgttggtaggtcacgtaggtacggtttattgcgacggtctttcttttccgcgtgtcgggtgacgtagttttcctcttgtagcaacgtgaggacgactactccgtgtggctcgacggtacggtggtcaaaggctgttggggatgcagcgtcatggactggttgttgaggcggtatctggagatcgtgttccccgcaggcgaccacgtctatcctggacttaagacggaattgcatagtatgcgctcgacgctagaatccatctacaaagacatgcggcaatgcgtaagtgtctctgtggcggcgctgtccgcgcagaggtaacaacgtgttcatagcacggtgttttacttttgtcgggctcccagcctctgttaggttgcggagataagtccgtgattagtcggctgtctcaggaggcggaaaggaaatcggataacggcacgcggaaaggtctcagcgagttggacacgttgtttagccgtctcgaagagtatctgcactcgagaaagtagcgttgcgatttgcagtccgctccggtgtcgttcacccagttactttaataaacgtactgtttaaccacgttgcgtcgtgacgttgtttgtgggtgttgctaggcgggctggaaagatgatgtataaatagagtctgcgacggggttcggcgctctgccggctgcggcggcactcgctccacggcctccgacgagcgttgcgctcgcgctttgcgccgccgcgtcatggatctgcctactaccgtcgtgcgaaaatactggacttttacgaatcctaaccgcatcctgcatcagagcgtcaatcagactttcgacgtgcgccagttcgtctttgacaacgcccgtctggtcaactgcgtggacggcgatggcaaggtgctgcaccttaacaagggctggctctgcgctaccattatgcagcacggcgaggcttcggccggcgccaagacgcagcagggcttcatgtccattgacattacgggcgacggggaacttcaggagcacctctttgtacgcggcggtatcgtctttaacaaatccgtctcctcggtggtgggctccagcggacccaatgagagcgcgctgctcactatgatttccgagaacggtaatttgcaagtgacttacgtgcggcattacctgaaaaaccacggcgaatcctccagcggaggcggtggttgcggtgccgcgtctaccgcctccgccgtctgcgtgtcctcgctgggtggcagcggcgggactcgcgacggcccttctgcggaggaacagcaacggcgaaggcaggaacagcgtcacgaagaacggcgcaaaaaatcgtcctcgtctgccggtggtggtggaggcggcggcactggtggtggcggtggcggcggcgggagcggcggtcagcactcctcggactccgccaacggactgctgcgggatccccggttgatgaaccggcagaaggagcggcggccgcctccctcctccgagaacgacggtgagtcccggccctcctcgcgtcacggtgctttccgagtggactcgtgagccccccgtagcgcacgagcgagcaggcgagcggtgttggtgcgctggtggttgtgtggatgataaccatgtgctttttcgtgcgctatgtgtcgtcccgtctgtaggctctcctcccctccgggaggcgaagagacaaaagaccaccgcacagcacgaaggccatggcggcggcggcaagaacgagacggagcagcagtccggtggtgctggcggtggtggtggcggcggcagcggccgcatgtcgctgccgctggacacgtctgaagcggtggcctttctcaattactcgtcctcatcctccgcggtctcttcttcctccaacaaccaccaccaccatcatcaccaccataacgccgtgacggacgtggccgccggcaccgacggtgcgttacttctacccattgagcgcggagcggtggtttcgtcgccgtcgtcgacgtcgccgtcgtcacttctttcgctccctcgacccagcagcgcccacagcgcgggcgagacggtgcaggagtccgaggcggcggcgacggcggcggctgcggggttaatgatgatgaggaggatgaggagggctccggctgaggcggcggaggcaccaccgcagtcggaggaggagaatgattccaccactccagtctctaactgccgtgttcctccgaattcgcaggaatccgcggcgcctcagcctcctcgcagtccgcgttttgatgacattatacagtcattgaccaaaatgctcaatgattgtaaggagaaaagattgtgcgatctccccctggtttccagcagactcttgccagagacgtcgggcgggactgtcgtcgtcaaccacagcagcgtcgcgaggaccgccgcagctgtctccacagccggcgttggccccccagcagccgcatgtccgccactcgtcaccaccggtgttgtaccctcaggttccgtcgccggtgtcgcgcccgttgccgccgcagtcgaaacaccagctgctcctccccggcccgtgtgtgaaatcaagccctacgtggtaaaccccgttgtcgccaccgccgcggctgccagtaactcttcctcgtcttcttcggctccactgccgccgccgccaccaccgccgggcggacgtcggggtcgggcccggaacaatacccgaggaggcggcggtggtggcggtggtagaaacagccggcggcaggccgcatcgtcgtcgtcctcctcctctcggagatcgcgacggagaaacaaccgccacgaggacgaggacaacgatcctctgctccggttgtcgcaagtcgccggcagcggccgccggcgagggccctcgttcctcgaggacggactcgaaattatcgatcccagcgaggaggctgcgatcgccgccgcctcgatcgcggcgtttttcgacgattaaaaaaccgagccgagaccggaaaaattatgaaacaggacgcgcttggacatttgggtttccacccctttcggtgtgtgtctatatatattgtggtcactgattttttttttacaataaagagatagacatcacagttcaccatcttgtctccccggtgtgtctattatcatcaatcacccacagagtcgccagtccatggtctctcggtaatgcgtgtccagatacgcgttggccagtataaagtggtcgttgcccacgaaggcgcgggtggtgttgcgcggcgacgggtggcaggacttaagtaccaagtgccgccgtcggtcgatcaggtactcgcaggtgtgcgcgtcggcgccccacagcatgaacaccagatgctcccggcgctctgacagcctccggatcacatggttactcagcgtctgccagcctaagtgacggtgagatccaggctgtccgtgcaccacggtgaacacggtgttgagcagcagcacgccgcgtcgcgcccaggcgtccaggcaacccgaggccggacgctgaaacccgtccaccgtacgcgccagttcgcgaaacacgttgttgagggagggcggcggcggtcggcccgccagcgtgccgaaggccaggccgctggcgctgccgtcgcagtacgggtcctggcccacgatcaccacgcgcacctgctcgggcggacacagatagctccagcggtgtacgtgctcgggtgccgggtacaccatctcgagttgccgcgcgccttccaccgccgccaccgtgtcgcgcagcagcaccgtgtcgtggtcgggcaagctgaggaagcggatccagtcggcgctcagacaaaacacgcgagcctgctcgtcgggggttaacagagagcctttattatcagcaatgttagcgagcatccactgcttgagggccatagcgcgagtgagccggcaggttgacgcgcgtctgcttcagctcgggcggcagtccggcgtagtatttatctaggtggcgtagcagcggcgggtccagctggtgacgcaggcagaattccttcaccgcgttgtacaggccgtaaaagagcgtgatgccctcgggcgcggcagcggtgctcacgggcagacgcacggcgcggttggtacgcgtggcttcgttgcgtatggccaccaccacgttaaagagagacggtggcaccagctcgaagcctaacacgtgttccgtgaagatgctgcgcccgtatgacagtcgcgtgaggtcgtagccgcggcacaggtcgtccacgcacgtgtacacggccggcgagccatcgccgcactcgctgtagccgcgcattaccgtcatccagcgcggcgctgtgtccgagcttaacagcgtcagcagggcccgcaattgatccggattgttgtacagcagggccagagtgtccaggaaagcatcgtccaacagcacggagttggcggcctccggcgtaacgggacggtaacggataagttgcgatagcgggccatcgcgcccggtaacattcaccaacgggcgcagccaactttcatacttgtcaccctgaaacacctcacccaacaggcatcggcgcgttagttcggggcactccgcggggactttctcggcggcggtaggagcgacgctgacggcggctgaggaaacaatggacagcagaaggcaacaccacagcagtatcaccggtccaggtgagaaagagaagccgcaatccgggcggcggcacatcaagtctgcggcacgatgagagtgtgacggtaaggagccagttggcgccgaaagttggcactcaggtcttcgatccctaaaacgttatatattgcatccagcaggtgagccaggctaaacggattcacgtaccaggtttggttacccgcgacgatgacggccagaccgtgggcgctacagttggagaggttcctgggtacgaaggtaactgagtcgatgtcgcgccacggggggaatgagacagacgactggcgcacgctgtaatcacaactgtgattgacgtattgtagcgtgtaatttaggttgcactcagcctcgaagtagagggggaaccacagttcgtcgtactcgtcgtcgtcctccagttctggctcttcttcatccaccgcaatgtctacgctgctttgagattcctcttcgtacaggatgattgacaggttatggctacaaaggtcctgggcgggaggacgcgtgggagcgcgggtggtggtaatgttttccagatcaaaagttggagtgtagtcggatgttacatccccgttgttggaggtggtagaagttgcggccggtgtcgcggtggtaagtatggatacagaaggggagggggaagtagcgttcgtaccgatggttgtggtattattattccctgtgtttcttgttccagaaaccgttgacgttgagatgggaatcgacgtggtgctggacgtcagattgctgaccgaggaaaccgtggtgggagtggtgacggtgttactcgtggttgaagtgacgttaggggaggtagtagtggtaccggtggtggcgacggtagtgtttgtcgtggcggcggcagcggtggtaccggtaacggtggtcgcgttggtttccaccgcttcacacagtaagcaaaagcacagagccaggaaaagcaaccagccccgccatcgccgccgccgcttcatgaggtgggcaggcgaaagctggtgaattcgttgtacagcggcaagtggggcgccgcgatcgaagggtacgtcaacaagctgacgttgatattaaatacgtctggctgcttttctacgatggaagcgcacagggttacggcgtcaaacaggtctttcttggtggcgcccgagacccacatctggtatacacccgtctcgtggtacgaagtagagcgcggcaccaccggacggatgcagtccagaacgcggttgggatcttggtgaaagaatttgaacgtggctacggcctgtggcgtgtgcggcatcgtctgcgtgatgagctgctggcccgctaacacggtgacgttgtgcaacttgagcagggcactcttgagggcctggaaagcgttgccgcacgaggcgctgatctgcagctgcacggccgtggagtcgtgcagccgcatgagacgtgacacctcttcgaagacgtacttatacttactggcaaagagtggcgcgtatcgacagtcggccggcaaaatgtaggtggcgttgccgccgttggtagccacggcgggcgcagcggccgcggaggccggcgtaaacagcgtcagcggccggtggtggctggtaaggtcgatcatgggcggcgtggtgaccgtggcggtggcgggcatgacggggtttgcggcgacgggcactccggccacagcggcggccgcggcggccacggcggcgctggccgagcccacacccgccggcagtcctccgctacccatgacgccgccgggcagagcgtcgcccagacagacttccacagtggcgggcgcgctctcggcggtcagtacggtttgccgatcgacctcgcgacgaaagctggtgaggaactcactatgatccatggccgcagggcccgagatcccgggattctgcgggtgctgaccgagtgcgggccgagttatatggaagacgattagcttggagcggagttttgcgtccctagctgacctgcggatcagcgacgtaccatagggatagactgtgagcggcggccgcaacggcggggtcggccgccgttcgtcgtcacggggcggcgcgagggaggaggaggtggtgggtacgatcttgacgtggttgacgtcctgcccgtccgggggaatacgcaaaaaaacccgtcgcggcgctaccacgatggtgcgatgggtctttctcttgttggccggggccagggacttgcagatgcgtgtggagccgtagacgatctggacgtggtcctgggagaacatgaccatcgccgccaacgctcagcggggggacgtattgggaacacagaggatgagggaaaactccgtagaagtcagcgaaataaagacaacacagcagccactcctctcgtctcgggccctaccactgcttgaagtagggcaccgggtgtttcttttcctcaacgggctcctccagtctcttataggaccagtcccgccggcgcgccagcatgtaggtcacgtacaaaagaataatcaccatgaacaccaggaaagccagcacgccgtaggccagcagccggtcctcgaacagcgggtcgctcttgataaacacgtaggtggtggtaaaacttcggcccgcgatctgaacgtggagacgcacgacagtatacgtgccgttgaggtagaagacaaactcgcgtaaccgttgtccgttatacgtcacgttactaatattccacggcggaatgagctggttgccctgatgcagatgcacggtgctgttggggtgatagaggctgctaccgttgagcaagcagtgttcgtgttcctgaagcagcacgcggacccgcatcgtggtagcgttcaagcgagtcccgtacacggcgtagatgggataggtgaaaaggtcccaagtggcgttgtgatggcggccccagctgaagaaagagcacgtgtactcagtggtctcctgcggcctgagtcccgagataagcagctcttgagcagtagcgttgtaggagagatgtagttttcctgtggaaaaaattaatgagttgtttattttgttagcaggttggcgagggaggaaggagaacaaaacagaaaggtacgtgttacttacctttatcgttggagggaaaagcgctaagataccccacctgagtgaagggacccttgcagtctgtccgtgcataacaagtaactgataaaatgtctggatttttggtattattcaacaggattactttgcaggtggcgtttagagacacttggtcgtagctgtagctggcttcgcaattcacagtatacaggtgcccctctttctgcgtcgtggctatcacggaggtggaggcggacgaggtagaggtttgtaccgtggtggtgacagcagaagtgacgttgttagaggtacttattgacgtagtagacgtgacggtggtattactaggggaagtgacggcgcttgtggtgctacttttcactctcgggtgcatgtcgcccaagagcgcaactacgagcgcgatcgccagcacggaacacatgttgccgtgtgacgagacggcgtgtggacgagctatatgtggcaggaggtcgcgtcacctcttgtgacgcctaaacgtccagctccagataaaagaggcgttaataatgaagaccacaaaaaccacttgcgtcagtatgacaatcataaaggctcggtgattgctacgcctaaagtacgcgggattatccaccagttcatcctgctgaacaaagtggatgattgacgtgctggtgttaccggccgtcgtattgatcatggattttactaagaaagttttggcaccaaaagtcccgttagagccccagcaggtaacgctgccgttcacataggctcccggtgcccctgtcagcatgcgtttcagttcatgagtataatttttcctatcgttatacatatcatcactgtagttgactttgctggtgagaaactgtgtgttctgtggaatactgatcatcatccccgaggccaaaaagggcgaatcgcaagctgtagtgttacagaaaatagtcaggttagtgtcattatgctcatacatataagccacgctaacctggggctcataccacccaatcgcaaccgccagcacgtcccatctcccgacatttatcaccgccaccactaacaacgtcacccccgcacggtacatagttaccctctcgacgtcgccggctgtcaatgacgtgcctgcgtcagtggctatgatttatagcttttggacacaaccgcaacggatctgtcgtaatctaccttccacagggccgccgcgacgatgctgaacgacaggatcagacagacggcgtataggagtcctaggtcggcgtcgacgcggcaagtgcggatgtctcgcagggtgggtagatgggcgatgcacaactctttctccccccgcacgtacatcccatctcgtatcagcagccgtagcgtagcattaatggtcagcggggtaaccaaagaaatcacatagggatgtgtacaggaagtacagtgacgggtatccgtgagatgtaagtcatcacccttctcactgttatcatgaaagaccaggactcgggtaagacgacccgatgaatactggatctcccaccacagtctttggtccaacaccgagagggcacaagagattctaagtctccctgggttgggggagcagatgtaagccccgtgtgtgcccctcgccatcagaaccatacacatgagggggaaaaggacaagtatccgggaccacccgcacccccacatcacgagaccagagacggagatgtataaaaaaaagctacttttattaaacagcattctcaccacacgttaatactgtcacggggaatcactatgtacaagagtccatgtctctttccagtttttcacttactgagacttgttcctcaggtcctggatggctgcctcgatggctaggctcagggtgtccaggtcttcgggaggggtctcggtgggctgctcaaactgccccacgtcgtaggccttcgcggccgtctcgtagataggcagcatgaacccaccctggttggtggagaagatgcgcaccatgacctgtttgggaaacttttgcatcaggggcaggcacaggttgagagcgcccaacaggtccacgggggtggcagcgtggatgatcatgttgcggtaatcggaagaacgggggcataattggtgggtgtgcaattctttgaggctccacgcggccttgacgccttcgttacaagcatcggccgtgcgctgcgccacttcgggtgggtgtgtcacaggcatggtgtgctccatgagaaagggagtggagagggccaggttgcacatggtgcccaggcgacaccgcaccgcatccacctcactcttcacctcatgattgcgggtgtagatgatctggatgcccttgttgttcacctgcatggttttgcaagctttgatggcctcatctaacacctggtgcatactgggaatcatgaagggcaggttcttgtattcaagagagcgattggtgttgcggaacatgcggctcacctcgtcaatcttgacgcgaccccgccgagtctgcacgttgggtgtgcagaagggggtgttcttatctttcatgatattgcgcaccttctcgttgtccaactcggagatgcgtttgctcttcttcttgcggggtccggtgctcgccccgccgctgctctgatggccgcagctcagcagagaggaggaggccgcgccaccaaaaccgccgcgcccatggtggctcgaggtcacggatgctcctccgccactgctgcatttcatctcctcggactcactctccgagtccgaagccgaactgcaggaggaggaagacgaagaggaactatcttcatcgggccggcccaagggatcgggaagaggagggtggttcatctgggagagcgggtgcgtgggagaggtcactcgcggcgtgccgctgccggtggaaggggaagacgcggtagcaccgcgggtttcgacttcttcaccctgttcttcctcgctatcagagatcacgatacagccggcggtatcgataatcttgttgcggtactggatggtaaagtcgggctcgggcttgatgtcttcctgtttgatgaggaggggcagcatgataggcgcgggaggcacgggcggtttaataatcaccttgaaaggacgcgtggttttgcgcggtttcttacgcgggctgagctcgggagtagcggatgccccggggagaggagtgttagtaaccgcgacgctggtgggggtcggcttgttaagaggggcgctgctaacgctgcaagagtgggttgtcagcgtgtggccggtgctactggaatcgataccggcatgattgacagcctgggcgaggatgtcacctgatggtgataagaagacacgggagacttagtacggtttcacaggcgtaacacgtttattgagtaggattacagagtataacatagagtataatatagagtatacaatagtgacgtgggatccataacagtaactgatatatatacaatagtttactggtcagccttgcttctagtcaccatagggtgggtgctcttgcctccagaggtggtgggttcctcagcaccatcctcttcttcctctgaggcaacttcccctatctcagacactggctcagacttgacagacacagtgtcctcccgctcctcctgagcaccctccccctgttcctcatcactctgctcactttcttcctgatcactgttctcagccacaatcactgaggacagagggatagtggcgggtacaggggactctgggggtgacaccagagaatcagaggagctagcaccagcggtggccaaagtgtaggctgcaatagcatcttcctcatctgactcctcagcgatggcccgtaggtcatccacactaggagagcagactctcagaggatcggcccccagaatgtactgggcaaagaccttcatgcagatctcctcaatgcggcgcttcatgacattgataacctcaggcttggttatcagaggccgcttggccagcatcacactagtctcctctaagatatagcagcacagcacccgacaaaactcacttaagagagagatggacccgtacatggtcatcatgcaagcgtcactggtgaccttgtactcattacacatggtttccacacatgtagtgaggatatccataaatatgtgatcaatgtgcgtgagcaccttgtctctctcctcatccaaaatcttaaagattttctgggcataagctataatctcatcaggggagcactgaggcaagttctgcaatgccgccatggcctgactgcagccattggtggtcttagggaaggctgagttcttggtaaagaactctatattcctgtagcacatataaatcatttttctcttaagttcatccttcttagcacgggccttagccttcagtgcaccccctaacttgttagcggcgcccttggtcacatcatgcagctccttaatacaagccatccacatctcccgcttatcctcgggtacaatgtagttctcatacatgctctgcatagttagcccaatacacttcatctcctcgaaaggctcatgaaccttatctaagatatctaaggcattctgcaaacatccccccatcatattaaaggcgccagtgaatttctcttccgtctgggtatattttttcagcatgtgctccttgattctatgccgcaccatgtccactcgaaccttaatctgtttgactgtagaggaggataacaacacatataagtatccgtcctcctgactcatttatcgctatctcgatgccccgctcacatgcaagagttaatcttcactctatctgacatacacaagtaaatccacgtcccatgcaggttagtatatatcacatacatgtcaacagacttaccgagttctgccaggacatctttttcggggttctcgttgcaatcctcggtcacttgttcaaaggttttgagagattcttcggccaattctgggaacagcgggtctcccaggctcagctgactgttaacctccttccttaacatagtctgcaggaacgtcgtggccttggtcacgggtgtctcgggcctaaacacatgataaacaaagtcataagcacatgggtcacatacaggaaatatgtatataacattaaagatataactttttattaaaaaaaggggaacacaagtcccgacacgtaccgtggcaccttggaggaagggccctcgtcaggattatcagggtccatctttctcttggcagaggactccatcgtgtcaaggacggtgactgcagaaaagacccatggaaaggaacagtctgttagtctgtcagctattatgtctggtggcgcgcgcggcagcaacgagtactgctcagactacactgccctccaccgttaacagcaccgcaacaggagttacctctgactctcaacagaacacaactcagctgcctgcttcttctgctgctgctgccttaaatcttccatctgcgtcagcggtgcaagcccattccccgagctcattttcagacacataccctaccgccacggccttgtgcggcacactggtggtggtgggcatcgtgctgtgcctaagtctggcctccactgttaggagcaaggagctgccgagcgaccatgagccgctggaggcatgggagcagggctcggatgtagaagctccaccgctaccggagaagagcccatgtccggaacacgtacccgagattcgcgtggagatcccacgctatgtttaataaaaactgcgggcactggggacggtggtgttgtatatgtgaatttgtaaataataaatgagaccccatcctgtaaaaatacagagtccgtgtcagtctctgaaggacagagtattggcatatagccaataaagatagttgtggcaaagagccatgttatggattagtaatggaaagtatcgtcaccaataggggagtggtcaataatggtcaataacccacacctataggctaagctataccatcacctatagcataaggaagcgggggtgtatagaccccaagccaaaaacagtatagcatgcataagaagccaagggggtgggcctatagagtctataggcggtacttacgtcactcttggcacggggaatccgcgttccaatgcaccgttcccggccgcggaggctggatcggtcccggtgtcttctatggaggtcaaaacagcgtggatggcgtctccaggcgatctgacggttcactaaacgagctctgcttatatagacctcccatcgtacacgcctaccgcccatttgcgtcaatggggcggagttattacgacattttggaaagtcccgttgaatttggtgccaaaacaaactcccattgacgtcaatggggtggagacttggaaatccccgtgagtcaaaccgctatccacgcccattgatgtactgccaaaaccgcatcaccatggtaatagcgatgactaatacgtagatgtactgccaagtaggaaagtcccgtaaggtcatgtactgggcataatgccaggcgggccatttaccgtcattgacgtcaatagggggcgtacttggcatatgatacacttgatgtactgccaagtgggcagtttaccgtaaatactcctcccattgacgtcaatggaaagtccctattggcgttactatgggaacatacgtcattattgacgtcaatgggcgggggtcgttgggcggtcagccaggcgggccatttaccgtaagttatgtaacgcggaactccatatatgggctatgaactaatgaccccgtaattgattactattaataactagtcaataatcaatgtcaccatggcggtcatattggacatgagccaatataaatgtacatattatgatatggatacaacgtatgcaatggccattagccaatattgatttatgctatataaccaatgactaatatggctaatggccaatattgattcaatgtatatatcgatatggattggccatgtgccaacttgatgtcgcctctatcggcgatatggcctcatatcgtctgtcacctatatcgaaactgcgatatttgcgacacacagaatcgcccaggtcgccaaagtcgtctatcgccatcccccgtaaacgatataagcgctatcgccagatatcgcgtatgcccaaaaatcacttttggaaaaatggcgatatcagttacacagagactcacatcggcgacattttcaatatgccatattttcaaatatcgatttttccaatatcgccatctctatcggcgataaacaccactatcgcgcgacatgaatttagtcggcgacagaaatctcaaaacgcgtatttcggacaaacacacattttattattcactgcagcatatagcccattttagcgcggcacacatccagccgtttgtgtttcttaacgctctccaggtactgatccaggcccacgatccgggttatcttgtcgtattccaggttgatccatcgatagggaacgctgccagcggcgcccagcaggtactgcgccttgtcgttcactttgccgcagcgtattcgcccgtcagcttcgaggtataacctacaacacggaagggaaggggggtacaaaacgtgaaattagactttttttttaatgatgttttgtccctctctgtcttactctcccataggctgtaaggccctcgaggaagagacttacggattgtagttgcagctcgtcagtttgttgtgtacgacctggcgtgtcaatgaatgggtcatggtggtgatgatcccgcgaatctcagccgttttctcgggactgtagcagacttcgccgtccggacaccgcagcctgtggattcatgaaaatctactctggcattcccgaggatcgtcgatggaacatggctatcagaaacgtcgagagacagatccagacgcaccacagaacgcagacaatcatgaaaatacgtacgcgacggtgaagcgattgcacattttgaaatcgtaacagcgttccggcgggtggttgacgtttatgaattcgcaacattcttctgcgcgtacccgcggcacgcggctgtgacccagtagcaaccacaacgtcgtcaagaacggcgtcaggtctttgggactcatgacgcgcggttttcaaaattccctgcgcgcgcgacgggctcaaacgatgagattgggatgggtgcagaaggtgtaagtctggttattggcctcggtgaacgtcaatcgcacctgaaaagacacgctgtagtcccggaagacgtgggcccagctctccagtttcatcacacacatctgataacgtgtgccatcgttgacgacgaagcgtagcagcttggtctgcttgggcaccatgtgcgctccaaaaatcttggcgtcttccacgctgatctgcacgtttccgtcgctcggtttcgaagccgttcggggcatccgttggaggatggtctggttgcgaccgctcagataccagatcacctttttcacccaggtggagcttttctccaccaaggtctggccttcccggttgtacagcagatacagggtctcgttgcgacactcgggacccgttgatacccgctggaaccccgagaattgcgagggggaccgtgggggcgagggatagagaaaaggacagtaaaacgtcgccgcgtcatgcggtttggaatacgtcagtttagaccatggcggggacggattctggttcgccgttagcgtcgaccacgaagacgccagacagggcgttgcccaaaccgcgcacagaagcaggcagtgaaagtagtgacgaagcagaagccgcagcatattatttcccgtgacgcaggctagttggcaaagagccgcacgctgaactcgaggctccgggcgtgcggcgccagcgaaccggcggcgttgaacgtggtccttttgttggtgccgccgcgacggttctgacgtctaaagtcgctgatgagcaacgacacctcggtcacgttgattctgcaagcacaggttccgaacgtcatttcacaccccatgcggttacctacccgttacccgttcgcccttaccttcccgttgtcatacacctttagcgcgtaccctcacctcttgagcacgtcaaagttgtccaagccgtggctcgcatcgtagtggtagttcaacgtgaggtccacgagctgttccacatacttgtaacgggtttggtcgggcagcgcgcgagagcacgcgtcccagtaatgcggtactcggtaataatcgtttttttctgcggtctcccgctggcactgacccagcaccacggcgcacagacaaacagacagccacacccgatacagccgcatgttgcagactgagaaagagagctttattatgagacatcatacacatagtataggcgaggtaatggggcggggaaagagttggaaccgaaagacaaaaaaaaaagcctagtcgtactcgggatctctgagcgagacggattgcgtagcaactttcattagtttgggaatctgccagctggtgctgttggaaggttcttccatttccgaggcggtcagttcatcgtacaccgagacgtagtacctgatggggtcctcctcattgtccgagaggtgagattcgatggtcaaaggcgagcctctcccataattgggattcacgaacgacgtgtccaagttgccatcctttctgaaatagatgacgttctcaggatcatgtttcatgcgctcgcgggccgcggacgcctcctcctcctcgtcccagtcccgagtttccaaccgctgataagggctcgaggaacaaaatccggcggggatctgagaacctcgtcgggaaccgctgccaaacgggctgctgccgccactatcgtccgtgtcgtccaacaggttgacggcctcttcgtcggcgaaacgaaagcggcccgggtgcttgcaacacgaggagtaaactaccgcgatgagtaccgctatgaagctgaaaatggaggtgcctgtcacaatgtagaagaggatagccagcactttcatgatttcgtcattgcgcgcgtcgtgaacggaagattcgcgggcggtggtcatgttggtttcggttgtaggttcgctactcgtagtgctctcgacggtatttctgctgctggtgctagtagggacgtttgtgctgctggtcatatttgtagcgtcgctgaagtccatgtgaagcagcaacccgaacgcgaccaggaccaggaatgttgcgcgaaggagaccccgcggggccggcattcttgagacgtggcgacgtggatttcttgttatgtccgcgaacgacgtgtgacgaggacgtggtttccgcaagcctctaccgacgccgcgacaccaggtaggttatgaaaacgcgagcccatatcgccgccatcattgtaatcagcaatgtgttgaggtactgcacgatgaatctgtctagtgacaccagccaaccctctgcttttgcgggcaagcgcgctttcggtgacagggtgtatcgtacgtagccgcgggtcaggcgcgcgttgtagcggtacacgcagaaatctatccacaggccaacgcccggctgtagcttcggatggtggataatagcgcggtgacgtacgccgcggggctttagaatctccacctgtaaggccatctcctccaggtagtgggtctgactgcgacgcagcgtccagttcatgtaaaagtcggtctcgccgtgtccggccacgaagaggctgcttactaaatcgggcgccagagctaggtcaggcgtatcaaattccactgccaggcgacctgattctaacggttccacgatccgggagagcgtttctagatatagagcaaagcgtaccacgtctacctgcggtgtaaaaaactgttgtgggcgttcaccgtcgttgaccacgtaggccacgtagaggccaacattttccaccacgggttctagctgcaggcggcacgtaaagcttagaaacgacggctgtacggtttggttcccgtgaagctgaagcgtcacttccttgccggggctcaccgtgctgtaacgtcgcaccgagtcggtcatctgctccagatcggtagaccagaaaggcgtgcaatgcatactgtcccagtcgcgacacacagcccagcctagctcggtgaagggtcgacgcacacccgaaaaagtgtgcttgaagaccagggggtcgcctcggtagctcagtagccgaacatgcacatagtcgcggctagcgttgacagacggcccgtggagggccagtaggacgagcgtgaacagcaagcgcaacatgctgcgcgggttaggaaatgcggcgtgccggccaccgcccgactcataaacgctaccagcatgacgtctcagatcacacaagtgacgaggagcgtaccgcaaatcactagggaaaaggccagcagagcccgatagtcttgctcttcgcgaacgatctcgtccggttcctcgcagtcttcgtggtccacagaagatgaggagcaggattcttcgttaatctctgccaggatactagtgctataccacaccagagcgctcagcgtgcccagggctaccgcacggtaaaatagggacatgatcaccagcgcagtctaaagtagtggtaattaagtttcttggcgtatttccagagaaaggctttgtaggccgtagggactggccaggcaccgaactcaatattggtagacactacgtcgtaaatgcgttgttcctcatctaagattaaccgaaaaaatagccggttgatgtgacggcgcacggcttgcgcgttaggattgagacacttggtgcccttgtcctttaaaatagccagcacttcctgacgattgcagctttcgctcgctgcgattggcttaagcagttgagttccgactggcagggtattcaacagaatttggttgttgcaacggcagcgcctgtcgtaatcttctagttctaaaacatggacggctaggggacatatggtaagtaacatatatgcgattaatgacaggtatcgtaccgataacagattgatatgcgagtttgaaaccggatggtgcaaccatgttagtaccatattaaacacatactgtaatattttgttttaacgaacttgtctgtttgaaaacatacattaaatattatcctctaacacctatcaaggttatatttattcgtctcggttctggtgatttcgttatgttaacattataccacctattatcgttgcgtttgtctaaccattttgagaagaggtgatcgggcgataaacatactccatgtccaggcggcttccttccgtctggatacaataaatgttcatttttatcgcatccgggccctctgggatcgcgatgaagccaataattacccaatataattttattaggcggccattttctatgaagacatctgcagcgtaattctgttccattcacctcataatgatacacatatgctaaaaaaataatcaacgcaccaaaaattaatcgcattataattttattatctacgtcactaccagtaattcgtaatatccggtattcccggaaaatcactcaaaactgcgtccatgacacatcaattcccgataagtacccccctttgaaatcggatccccccacataccaatcaatcacacaacacacaggtttaaaaatcgatcacacgtcaattaggtttcaaaatcgatactgtttattatcaggaatctagactaattctacaatgacagctctgaatttctctcttgtctttcttgtcaggttctcatcatcagtcatcacttccacccatcgaggagtcatcgtcgctccaaaatcctttggggtcgctagttggaaaagtctctgacacgatccaggcaccccgcacccagtccgactgatctagcttgcggagcatctcaacaggcatgagctgcagggccacggctgtcacggcactgtatcgatgtaacactagggactttctttgcgatgtagccatcaacacggcgtatgccccatagttcgcgtgatacgacgcatgatgggttaaacgttcccatccggcagtgccgtctcgggtccgtgcacacaacagctgcacagcgttatgatgcttaaaattaaccataacgctgggactactgatgaaggagtagtaatgagccaggacgccgtacatcgaaggcaacaagaaagagtgacagcacgatagcaccgggctcttatgtaggcgacagcttatttttcctgacgtcggcaaaaagtacctaaattccccacagatattcagacacggttccgtaaagtgcttctttttttagtgcaggaattggaaaaaataataaaaaatatgaacagctcatctgtaattatctgtgtgacttcatcgtaccgtgatgtaaaaacaacaacaggaagcttacagggtgcggtagaaaaatttgccgattgtgcaacactgttggcatctctcactccgataggcggctataagatagagaattaaaagtatgatacccacaagaaagatgaagagggacaaccaggctagagtatgacgaccgcttttcctttgtttgacggttacatgtgcggtatgattttgctgtcgttgcttgtgatgttggacacctggagtggaaaacgacgtatgattcttagatgcgcatatggtgttattagtggaagtgcagttacgaaccgtgatctgagtgtcgttacattgagtacaattagtacagttgtaaagccctgtgagataagtaccgtttgggcacagtgtacacgttatgccactattctctgtacacacttttgtaactttttgtcctgatccgcatggcgggcaacattgattacccagcttcacctcatcgggcttacacattttacttcccccaagctgtagtaaaaacataccgaagcagatgagcatcaccagaggcttcatgcctcctaccggaagaataaaaataactcatagggccgaacggtgtcatcctctccgcggtttgtaatacgagattgcaaacgtaaataaatgacataacttcactaacacgcatactacaaagtccacctacgacgctgaaagttcttccaggacagaacaggatagtcagccatcttcacagtctacctcttaggccgtatccaggagcataggtaatcagtttccagccacagtacagcgagcccaggaaaccgcacacggtccctgccgggaacacgtaccaccacatcgattcgtcgtgccgtagaaccgtagagttttccgaacttttatacacgccggtggcgttagggccgtgtgtgctgctgtgattggaggttttgtgagctaggtaacagctgtgatttcacctgtcgccaacactgacagcgattacccaggtggagcacaatcacatagctgatggacgttggttgatccgttgattcccatggacattttaacggcgacagtacagctcccgttaaacattagaataatagacgttagtggataacagcatgttattcgcccaagtgtgatcgtggttatacactttcttgttttttgctcatatgctgtaaggtgttcgaggatcgtggggagtatatgtgttgaatcggaatcatgtttactgaccgcgccatacttcgtatacgaacctaaccggcgtaaagtgttttccgatatataaactggcgcctattgtggctgtagcgcccataggtatggcgtatacccacggtgatgttgtgttattcgttttttgtgataaaacgtagcttatgtttaacgtgtgttccgtcacgttatgtgtgtcgttaaaagacggcgcctgtacagtatggctttgagttgtatcttgaattgttattgcatctggaggtgttgtgtacagagtggttgttgcgtgttgaggtgttgttacgttttgaggcacagttgcggtgtacacgggctccaaggtgtagttacggagtctttctatgcaggtagtgttgagatatttttgaatgctggttatgttcgattctgtgaggttaaagtgtgtactatttatgacggtgtaatttagacggtcttgccatcccgaggatattagtgttaggtaattcgtgttgttcacgtttgcttgatatgtataggtaggtgtactgtttgtgaggtcgcaagtgtgattttcttgcagagattttatccatcttgtgtgaaaatattgagatacgcgatgaatgttttcgctatctatattataaagcgtttcagtgtcacctaggggttgtttgttgtaacttttattttggaccctgggtgtgaaccatgattccaatgtttgtatagtaaggtgtcctactaataaagacgaactgattcctaccgtaatgttataccgcacacccagggtgccgtttacaaacacggaaatgtttccgttacaaaccacgttggcagatgaattagattccaggtggtaacgataggataatgaccgttcgctcccaacggatgacacaaagtatccgaataaccaacacgcccattcaatccgcatattttaatcacactattcacacctcacacactgcattttttaacatcttatttttttattttatgcgtgttctcacctcttcatctttttaacaccggggtaactatcgtaagtcggtaggcgtcgatagccctcaccacctcgtcgtccccttcccggcgtggggcaccagcgtccacagcactgcaggtaacacaggtagcataggaaacatacggtgaaaatactccaaaatcccaaaaatgccgcgattccccgagtggcccagggagacatcccggtgtctatgtcggccggcggtgctggcgtcaccggtaaaaatttcggcgggtgtggctgcgaacggtagcagtcgccggggagccggtaacgctgtatcactgtccaacagcggtcgggttcctcgtccggacatgcgggtttccagcaatcctcggcgtcggcgcgtccgatatagaagtagttgcgctgaaaaccgcggtacatcccgcagtcgtgattccgtagacgccagggcgtcggcgaccagatctggtctcccagcgagtagcgacctaacgccggcgtgcagcaaggttcgtcgggccggctgagcgtctccagttgcgtgagaattacgaagcgttgcatgatgaggccgtggctgtagttgcgcagcacgcattcgtacatgccggccgtgtccgtcgatacgttgaaagtcagcgagaatatttggccgagatgcaattgcgagaaattccaagtggcgtacggcaggcggtactggagtccgttcatcagccgatggcctttgacggcgtccaggatgagctcgtcgctgccgtcgtgggaacgacagaaacgtgcgcgaatggagaccatgggccaggagtgtgtcatgaccgtgcaggggatggtaacttgctctccctcggcgaccaacaccggcgccggcgacgtggtctcataattctcggcccacatcttttcggcaatgtcagcggtggcgaaggggaacgaagaggaagaatattcgaggagtcgcgggcagctcaacagcacccagaacagccacggcagagttcggagcgactcccggcggcacatgatgattctttccttccctttttcgcagagacgctgcgcgcctgctcctgctccgtgtgtcggccgctcaaacgtcgggccggcgtggtggtgaccaccgtgcgacgcagcttctcgcccgggatgcccgcgactgagcgtccggtttttttgcaggtcttttttgctgcctcctcctcgccgtcgccgtcgcggccgacgtggtggaccagcaccgcgcaggaactctcgcgtcgccggcggtacgcgacctgtctcattgctacctcggatgtttaagaaggaacgttcatctgcgtcacagggtctgatgaagctgccaagagtcgtggctgtggcgcagcgcgttctgtacggcgcgtttcaccgctttctgcatggccgctaccacgtcgggcgggagcggctccggcggaagctcgatgagcagttgctgcgagtctcggcgctcggcgtccgccgtttcgtcggacgtggcgtagaaaaccgaggtggtcgcccagtcgtccacgctgtcgacggcctctgtcagtgccgggttgtcaaaaccgccatcggacgcgggtgataaaagaacgtacgatgacacgctgttagtacgattctcgtcgtcgctctgggaacgacgtgatggacgacggtagatgacctcgtcttgccacgcgtcgaagcgatcgcagcagcgctggatccaagcgcagcgaagcagcttacggaacacgtcgttgttccaaaagtagagcataaagagaaagaaaagtagcgtaacgatgaagccgaaaacgacgagggtcggcagggcactaccgccgctgccgttttttgtgtcgtgcgggtgcacggtggtagtggcgttagtctgagctggggtcatgacaagtctgaagagatgagagcgtgggtgctcatcagggacagttgaggtctctccctaccgaagccttagcctctacggtgttttatgatcaacgtgtctacgaacgtcattgtgaaagtgacgtctcaggctttccgaaaccgcgtcagattcaacgtgggtttcggtttagcctgcgtcaccgaggcggaggtggaaatgagccgtcctgtgggggagtgtacgaccctgtagtgcccatgggtaacgtcgcgtcggaagaagtgaatgcggcattggtgtacgcgtgggttgttttgctctctgactcggaggagttgccgcagcagctgcagattttacgtactagccaaaagcagcaaaagcagcaggtaaataagagaaggagtccagataatgtccagccgctagcggcaaacagcgcaagttgcgcgactgtccaattactaccaccaaaactctcaacacattgaatcgacgctgaggttggtgttgcagtgctgttgctactagtggatgaagacgaagtagattgactggaattagagctggtacctgtagtggtttcacttgccgatgcggcaagtgcaaataaaactaatatccacagcatgttcgttactatataattgatatacgaacccgtttgtcgtaacaatcagcgttatatacgctgtatcggcatcgttttaccggaaagtttatcgtaatgtaacccgcgttgtgtacattcgtactgaaagggaacccccggtgatgtgcacattatactctttcattctggggtttcccaatgacgtaaaaatttccactatacaataaaattacggaatcatgtgaaaagtgtgctttttattaacagagcagagggtttacagtagatatatgtttgccagggccactgttttctaacaccgatcaccgccaccattaccacccgttgaactccacacccgggagccgcctgatcgccagggactcctcaccgtccatcgtccgaacaagctcccgccaccgatgctgccaccatcaccgagagaaagaaccgcttgctgcagatacgcttgggctcgcctccgtgcggacgccgtttcgtgcagacgctgagtagatcgagcagagaatgtcaaaacgacattaccgcgatccgctcccctcttttttctttttctcattcacgtgtattcttgatgataatgtaccatggctacggtggtgaactgcgtcgcggatcccgtcacgggtttcaacagatcgacgtcggtcagcggcgccgtcaccgccatgtccggcggaggcacgctgtttctctggttagcgacgtggaccgacgacgaagacgatgaacccgcgcggcggtctgttatccgcgacgacgcgtagctgcactgggaagacacttcctcccaacggaccaagatctcatcgggccgttcggagaaacggtatcgtctgtccgactcccgccgtacggcgccgaggcccagcgacgacaggtccgcgaaccggcgctcgtattccccgtacagctcgcaacagcggatcagccagcggtagctcaaaaacatgcgcaccagtttgaaggtgtcgtgccaatggtaagctagatagcagagaatggccacgatcagcacgagcatcacgccgatgatgggtaacccgacgttcagcggcagatcgtccatggtgaccgtcctctgtccggatctacgtcccagtctctctcttttgtacagcactcgcgcgggaacggccccctcaaccctcttacgtagcgggagatacggcgttctcccgcgggccacttacttgcacggtcgcttgaacggcggcttggactgccacatgcaccgcatccatccatttcggcagcagcgcgttcgacgatgtcgtacgagtcgcggatgatgttaccccgccagcacctccgccggcaaccgcgtcgtcgttgctatcgtcgccggtttcgggcgatgacagcgccggcggcgcgggtctcgtctcgtccaccatttccaccgtgtcgaagcgacagccgctgccgtagtacatagctccgttcaacggccggcgggccgggtcgccgagttccgggtcgggcacatccatggctcgccgtctccttctttgccgctcgtggtgccgacggcacttctcgggataatgacagccgcaaaatagatcgtggagcatgtctcgccaactgtcctggtgataatatcttaagtacgcgatgagcgcgccgatggccataatcataagcgtaagcaaaacggcacagataacgtgaaacaccgcggtcatccaagtcgggcggcgtcggggacgcggtgggtcggtttctcttacgccggcgtcactcagccaccacacccgtagccgacattcccagaatcggtgaatgcgactcaaggcctttcgacgccgccatttatttccaacgtccaagtcccacgtcatttctggcatctccacgcccttgactgacatactctctttctctctcttagctgcggtgaaaaagagggaaggcgtgtgctgctatacaactgtacaacggacgcgctcgctctttcggtctcaggtcatctgcatcgactcggcgtccttcatgacgctctgcaccgccttttccaacagttcctcgatgtccgaccatcgaggaggcggggctaactcggaaaccgacacgataggcagcgtggtcggctccgttggtgtgcggggtcggggacagggacacgagagtcccaccttcgagagattctccagcccgacggtgcgcggcagtctcggattccgcggcggcttttgcggcgtcggcgttttcgggaagggcctgggcgtcaccggcggtgtccagccgaccggcttgggtttcgtgggcggcggtgttttcttggtgagcggcgtgctcaggttcttacgcggcgcgggtatcggcgtcgggggcctgtgcgacgacagccgcgtggtgggggcccggaccggcggcgtaggcggccgcttcttgcgcccgggcggcggaggtggcttccaggatggtggcggctgatgcagcaccgtgtcgacgctggtcgaggacgacaaagagctcgacgaggaacaatgcgacggagatcggccgatgctggttggcgttcccggagtggatacgtcggggatctcgaaccgcgccggaggaaactcgggtttatctatcggcagaccatcctctcctatgtagagcgacgtacaccgcggcacctgcggcgtcggcgggtgggtggccacccgcatgagccccagttccagatccagcggctcgacgacgtcttctttcggattgcgatagcagcacgcgcaggcaccacgcttatcagaagcagcacccgggagccggcctcgcgacgaagtctcgtcggatcgcttgcggcctcggcgctgggtaaataaggaaatggccaggaccagggaagccagtccggtaccgccgaggagcccgacgccgagccacagccacaccatgatcttctctcctgcttggaatctcaaactccgtgtcgggaagggccggtgtacggacatttatgccttggatttctggaaacgtcattttttggcaaggaatgtgtttattgtccaaacactgaggaaggagatgtgggccaagtcggaaaattccttatcacaccgggggcgggttacgttccggtctgatgctgctgctgttgttgtagagccgcggccacggccgtctgcacggcagcttgtaccgcctcggccacgccgggtggcatctgcggcatggcggggggaggcgcgtcgggcggaccgccgggcatcgccgtcggctgtgacggtggttgtgaactcaccgtcggctcgcacggaggtttgttcttcggtctacccctcggtttgtctttcgccctacctttcttcggtttgggttccgatgtcggtgttggcggctgcggtgggatgacgggctggtgggactcctccgacggcggggggacgaacaccgtcggcgccgaaaccgggggactctcgactatctcgcagatcaccctgtcaggatcgtcgccgtgcccgggacgccgtcgatgaccgtattggaccatgtcgtaaatcatcgtctccttgtaacacgctgaacagcagcggctgcaggggcccgagatgcatttacagctgcacttacagctgcagctgcagtagcgcacccatcggcaagttaaaatgtcgattatggaatctttgaaaaattcccggtagcggatgaggtacgcgcagaggaaaatcatgaaaacggaacagacgaccacagccgcgatgccaggtccagaaaaaatattcgctgatgaacccgccaaacaccaaattcccaaggccgcgcatatcatccagatcacaatgatcgcggggacgccccattggcattggcacgaaggatcttgcacatcgcaacccatcgctactgcgttctcccacaaacgccatcgcactatttatccctacagcggctgccgagtcacgtccgccggcgcccatcggccgcggcgatctcctagtaacactcgtccgacacttccaccatctccagctcggccggcggttcggcatcctccaccagcggcgtcgtctcatctttgccgcagcagcggacgcacaccttctccaggcagaacgccaccagctgccgccgaacgtaccacaggtacacgtgcagacctgcgaacaggactacggaggtcatgaccaccacgacgcacacgggaatccaaggatcgagattgtcgctggaactcatggctatcgccaccgacgtgcccgcgtctgtctcaccgccgctcgcccgatgtcgcacggcttgttatacgctagcccgtcgccgcctcggggcacggtgccctcctacccacgtaacttcctccgtgacttaaagtcgcgtgtggtagatctcctgctccgtggacgaaccgttcggcaggatagcggttaaggattcggtgctaaggccgtgtcgccaacgtcgaatgctacgttgcaatagcttcgacggacggccatcctccctctcatcgcaataataaaacaccagcagcgcacacgacgcgatcacggtgacccccatgactagacccacgcagatagccagccccgctagcgtatccagcgccatcccgttcgctcccgtcgtcgtctcctgaacaaagcaactccgcagtccccgttttcaaccgttttcaaccgtttttgtttccttctccgcgactagatgttaacgcccgcggtctttccggccgtgctctacctcctggcgcttgtcgtctgggttgagatgttctgcctcgtcgccgtagccgtcgtcgagcgcgagatcgcctgggcgctgctgctgcggatgctggtcgttggcttgatggtggaagtcggcgccgccgccgcttggaccttcgtgcgttgcctcgcctaccagcgctcctttcccgtgcttacagccttcccctgaaacccgcgtcaatcgactgtcccgaaaacgccggcgttaacacaggaaaaaaaaaccacgcaggaaccgcgtaggaaccacgcggaacatgggacactatctggaaatcctgttgaacgtcatcgtcttcactctgctgctcggcgtcatggtcagcatcgccgcctggtacttcacgtgaaccaccgtcgtcccggtttaaaaaccatcatcgacggccgttataaagccacccggacacgtgccgcggcacttgcctacggcgctgctccagggaaactcctcttccttctgctcttcctccttcaccgcagggaccgtctccctcgaccagggacccgccgaagcaaccgccggaacaacctggaggaggcgcggcatgacggcacccaagtgtgttacgaccactacttatctggtcaagaccaaggaacagccctggtggcccgacaacgccatcaggagatggtggatcagcgttgccatcgtcatcttcatcggagtctgtctggtggccctgatgtactttacgcagcagcaggcacgcaacgggagcggcagcggctagataagtctctggcggctacagctccaagcgccgtagccggcccgcctgccgatcgcgacgtcgtggaccatcgaacagagactcacgcgtacgagaccccgaggtacgccacgcggtgcctaacgcggtataccacacccgtacggtctgcagtgcggcgtacaacgtgtggaaaacgcgttgcgtcgcagagtcagccacgtccccgtcttgtcgctccccaatcggctcccgcacaccccccgcggcacccagagggcgggtgagccaagtattcttaaggccgttctctgttccatatcccataaattgtttattccggagctcgttggcgcggaaatagccggataaggggagcaacaaccgtcggcgaaagccgtcccgctcattcagtccgggtttcgcgtctagtcggaggtgtgaccgttggccaacggaacggcgtttcacgatcaaaatcgtatcgggtagtgtaggagacgtcggcggtgcagaatgcgactcgcggcgtagctcgccgtcgctatgcggctcgtcgccgtgtggcgcggcctggccggctgtctgcgcccagatctgttggccttttgggtcctctggctgctgctgcgtgtgtgctttggcagacgcggtggcaatttgcggtctgcggtaagtgaggatatcgccgagcaagcgcatttgcggcacgtgggcggcacgcgtgttattgttcgttcgttgccagatagcaagtgctgtcgacagcagacgttgtgggcggttggtgtatttttgcgggttgcggtgaaagtcggcagccggcgtcttgtgaagtatcttaaccatctgtgttgctttttgcagcgtccagaaaagcgacgcgactttggggatggcctcgtgctcaccttcgcggagagcgccgccggacctgctcgtcagcagcgagctacgcagacggaatatctggaggagagttacgtgtgtcacaggggagcgcgggtctccggcggtaacgacggcggtatcgtcgacacgtgtgcggcctgctgtgctctgcggaaaagcgccggtctcggagaccgtggacgaaaaagagaacgcagcagctaccgctggcggcggcgtcgttaatgctgccgttgatgatcgacgttgtgagtactcggaaacagcggtgaggcagaagctcggttctccagggaacgaccgtcgatgcgtggtaggcgcagcaggtgaggttggggcggacaacgtgttgcggatcgtggcgagaacgtcgtcctccccttcttcaccgccccacccaccctcggttggtgtttctttttccttgtgttctgcagatagttccacggacagcgacggcaagtccataagcaccggtgtgcaagtggtggagcacgacgaagatatcaccgcgccgcagagtttgtggtgcacggcgttcaaggaagccctgtgggatgtggccctgctggaagtgccgcgttgggtgtggcagggctggaagaggtggcgcaacagcgagtccgggcgtcgatggagtgctgggtctgcgtcggcttccagcttgtctgacttggcgggcgaggccgtgggagaattggtgggctcgctcgtcgcgtacgtcatcctcgaacggctgtggttggcggcccgaggctgggtgtgcgaaacgggtgtgcaagccgaggaggccatggcgcgacggcgacagcgcatgctgtggcggatgttctctcgtggaggcgacggcgaatgcagcacacggtgtgcgatggagatggcgtgcgaggaagaaagcgccgtgttgtgagccgacggcgcgggacgcgggccggcgcagcgcgtgggccacgtgtggtggcaggcggcgtcgtccgcttgcggccgtcgccgcgccgcacagacgcaaacacatgtcgccgtcaagagaaacagtctgagcatagccgtctgcagcggtccgcgtgtagaagcggggggagaacgacgttaataaagaatagcggcggtgccgatagggcgaccgctgaagcgagctgcgtgtgcgtgcctgttttgttccccgtcgccgccgaaaagctacgcgcggcccccgtccctagccttgagcgcgccacagcacgccgcaaactcggcgtcgcgcttacgtcccgcaaacccccctcagcctcgtcccgccaaccaataccgtggcacgcagtgccatagcgccgcgcgtcaaggcgcttacacccccctcagcccggtcccgcaccggcgtcggtctgggtgtggcgggggtgcggctgggtgggtgtgtgccgggtgcggctgggtgtggcgggtgtgtcgcgggtgtgtcggctggctgtgtggcgggcgcgtgccgggtgtgtcgcgggcgtgtgccgggtgtgtcgcgggtgtgtcaggggtgtgtcggcggggtgtgcgcgcggccagatggaagcagtgtgccccggggcccgcgatccccccccccgccccggcgcgggcgcttcttctgcgtgtgtcctcgacgcgggtctgtgcgcctgcctgccggtcccggcagactgggctgcggcttcctcgttttttttttccgcctgtggccgtccccggggacttcctcttttccgcgtccgatcttcgcgtccccagggagtcgcgccgccgtcccctcgggaccgcttcctcttttccccggggactcaaagacacgcaagacagacgcgcgactgaaagagacgcaagacacacgcgcgtctgggtttcgccgtgcgcgccgcacggcgcttttattcgccgtcgccgtcccccgccaccgccaacttcccaaattcccacatttcacccccccgatgaaaacacccccccgcccctcggggacccagcacacggcccggaatggaggtcaggcgtccacctaggtgtgcgcgcgctcggcggcccgttgttggtggcttgtcgcgcatcttctttcggttttttcacggccttccagactgcgcggcggcaaggcggcgccagcaagcgccgtgcacgtcgctgcctataaaagccaggtgcgtgtcgcccgcggcacacgggcgacggaggcgtccgcgtgtgtaaacggcgtggtcgctgacgcgggtttgcttcctatatatacagagtggacgtcggaggcgtccggcggccatggcccagcgcaacggcatgtcgccgcgccccccgcccctcggtcgcggccgcggagccggagggccttcgggggttggttcctctcgttcttcttctttggaagcgacgtcaacagcggggactagtacgagtactgcgggtacggcgacgccggcccacgccgtccaccgggtagaaccccgcgggccgccgggcgcccctccgggtagcggcaacaacagcaccttttggcacggcccggagcgcttgctgctgtctcagattccggtggagcgccaggcgctgacggagctggaataccaggccatgggcgccgtgtggcgcgccgcgtttttggccaacagcacgggccgcgccatgcgcaagtggtcgcagcgcgacgcgggcacgctgctgccgctcggacggccgtacggattctacgcgcgagtgacgccgcgcagccagatgaacggcgtgggcgccacggacctgcgtcagctgtcgccgcgggacgcgtggatcgtgctggtggcgaccgtggtgcacgaggtggaccccgcggccgacccgacggtgggcgacaaggccggccatcccgagggtctgtgcgcgcaggacggactgtacctggcgctgggcgccgggttccgcgtgttcgtgtacgacctggcgaacaacacgctgatcctggcggcgcgcgacgcggacgagtggtttcggcacggcgcgggcgaggtggtgcgcctgtaccgctgcaaccggctgggcgtgggcaccccgcgcgcgacgctgctgcctcagccggcgcttcgccagacgttgctgcgcgccgaggaggcgacggcgctcggacgggagctgcgccggcggtgggccggcacgacggtggcgctgcagacgccgggcaggcgactgcagccgatggtgctgctgggcgcgtggcaggagctggcgcagtacgagccgttcgcgtcggcgccgcaccccgcgtcgctgctgacggccgtgcgtcggcacctgaaccagcgtctgtgctgcggctggctggcgctgggcgcggtgctgccgtcgcggtggctgcgctgcgcggcagggccggcgacagggacgacggcggggacgacgacgacgatgacggcggggacgacggcgatggcgacggggacgacgttgctgccgggggcgagcggcacggagacggaggccgccggcggggacgcgccgtgcgcgatggcgggagccgtggggtctgctgtgactttacctccgcagccgtacggcgccgccggcgggagcgcgatttgcgtgccaaacgcggacgcgcacgcggtggtcggaacggatgcggcagcggcagcagcggcggcgccgacggtgatggtgggtccgacggcgatggcgggtccggcggcgtcggggaccgtgccgcgcgccatgctggtggtggtgctggacgagctgggcgccgtgttcgggtactgcccgctggacgggcacgtgtacccgctggcggcggagctgtcgcactttctgcgcgcgggcgtgttgggcgcgctggcgctggggcgcgagtcggcgcccgccgccgaggccgcgcggcggctgctgcccgagctggaccgcgagcagtgggagcggccgcgctgggacgcgctgcacctgcacccgcgcgccgcgctgtgggcgcgcgagccgcacgggcagtgggagttcatgtttcgcgaacaacgcggtgaccccataaatgatcccgtcgcatttcgtctttcggacgctcgaactctcggtctcgacctcaccaccgtcatgacagagcgtcaaagtcaattgcccgaaaagtatatcggtttctatcagattaggaaacctccttggctcatggaacaacctccacccccatctcgccaaaccaaaccggacgctgcaactctgcccccaccgctcagtgctcaggcaagcgtcagccacgcactccgatacgatgacgagttgtggcgcccgctcagtacagttcacgaccacaaagcctggttggatctcgacgaatcacactgggtcctcggagacagccgacccgacgatataaggcaacgcagactgctgaaggccactcaacgacgaggcgccgaaatcgacagacccatgcctgtcgtgcccgaagaatgttacgaccaacggttcactaccgaaggccaccaggtcatcccgttgtgcgcgtccgaacccgaggatgacgacgaagatcctacctacgacgaattgccgtcgcgcccaccccagaaacataagccgccagacaaacctccgcgcttatgcaaaactggccccggcccacctccgctgccgccaaagcaacggcacggttccaccgacggaaaagtttctgcgccccgacagtcggagcatcataaaagacagacccgaccgccaaggccgccaccgcccaaattcggggatagaaccgcggcccatctctcgcaaaatatgcgagacatgtacctcgatatgtgtacatcttcggcccacaggccacggccgccagcacctccgcggccgaaaaaatgtcaaacacacgcccctcaccacgttcatcattgaaagtctctccagtccatatgttgtcaggacgtgctgtcgttctccgcttgctgcgaagcccgttcttccgagtcgtgtcgctgcgtccagcgtcgcgcccaagatgggaatttgggtctcttcacgcgtagcctcctccaccacggctgctgatcgccgtcactaaggaccgacacggaggatgacgaggagcttctccccgactccgcggtccgcgaccggctacgtagcgcgtgtccctgccagtctccgcagttacaccacacgtcgtgagcagcgtgcacctgctgccgccactgggcctcggcgtgctcgggccacccgccggagcccggtctgagctccgacgcaggatgcgcgtactcaacgtgcgccttccagtccatacagcaacaccataggtcgtgcgagtcgtcggctacccgccgccaggccagttcccgcatgggaaggctggacacgccgaccgagaggtcaccgagcccggacgccatctcttcttcctctccgtcgctgtcattaagcagccaggtcacctcctccgctccgcggtccgccggtctcgacggaccgcgccgccgtcggcaacacggaaaacagtacgccagcccgagccgctaaggccgcatgcccctgccgcccaactgaacacgcatatcccgctcaactgcgttttgccacccctgccagtgctcccgctcgagcaccaccccgcatctcccaacctttttccaataaacgaaaccgacatgacacacgtaatgggtactcgtggctagatttattgaaataaaccgcgatcccgggcgtctcagcacacgaaaaaccgcatccacatcatagacaagttacagtccacagtcacatacacgataaacaataccaacagggtaatgtttatggagtaaaacactattgtccaggccacatgcgtgtatgacttccgcaccatcccgtactgcatgttccacatgtacgcgctagacgtgtaatccactcgcagttcggggacgcaacgcagccagatcacatccccttgcagtaccagacgcagggctagcgtctcgaagatcggcatcacatctaagttccgcacgttccactttaacgactccccgggaacgaactccacgtcgtcggcgtgtacgtacaggttctctcccacgccgccataatcggccttcggatcgaagacgaaccgactcatgttgcccacgatgctcccccgagcaaacaacttgccgttgtcaatgtagcaccggttgtcctcgatttgaaaccagggatgcttggccgtggacttccagggccggagcgcgtcttccccggctttagtgattccatcgggcaggcggatcaagggacccatggaggtccaaagacccacccaggctttccagagattgttcatggtgaaacagcgtgtggactgtacgctctttcccaatttatatcccagagtagtgacgtgagcccagccacctcccagattcctgacgttttggttgtctttcctgccaattcctcccgtaaacttatgattatcctagcccattcccgataaaaatacacggagacagtagatagagttacgaataaaccggtttatttattcaagtgtctcaggagattattgaacgagcgtggataccacgccgtcgtcagttcatggtggcattgagcagccatagcaccagagtcccggcgcccggtatcagacacgctgacctaccgggcgccttcgagtccgtaccccgcggcctgggtgttagagtccgtaccttgcagcccaggtaggtttcaggtaccagctggttcgtacctgttaaataaatcgcagacgggcgctcacccctacggtcaggagcacaagaacaaccagagagaacagatatacgagcagggttctgaacagcagaccccaattgtcgtctctcatgcttcgctgaaggtaccagttgatggtctgagagctatagtccatcctcacctgaggaacacacgcggcatatttcttggggtctccccacctcgtagacaacgtgatgtccaccatatccacggtgtgcgtcaccgggtgcccaccgatgttccactcgaaataggctccgcgctcatcatggtggtactgctcaccggacacctgcagtctgtccatgtaagattgagagacgatacccacgttcacaaagtgtttctcggtgaagttgcccgacatcctccccttgaagtacagcatgcccatatggaaccagcattggttctcctccactcgaaagtgggccgatctgatctccgataccaccacatccaggggccggggcaccgagtccgcgagtctcaggaacaagacggccaggatcgcgagcaccaacaccggcttcatggctccgaaggtccgctgctcggctccgctcaccgctccggtctggctgcagcagtgcttcgctgagaagtagcgtgtggactgaacggtgtttttgaatatatagcgtttcttggtgacgttgtttcccctacgtagtaggcaactacgtgccaaaagaggcgttacggtactttccgtactgggatttccaaaccgggactttccacacggcggtttcaacaccgggacttttcacacggtgatttcggcaccgggactttccgcacggcggtttcgccaccgctgacgttctcatcgccgcccacgtcaacggtggcgacaccgtactttcccatgcggtttataaacgtcaagagtcacgtcagtcgcccacccccattacacggcgatatcccgatagggcatgaggggacccgggtgtcgcgacatgtcgacgacaggtgcggattagtggtcgtgtcgcgacatggacgtgcagggggatgtctgtcgcgatagagttgatgtgacagcccgctacacctctctgtcgcgacatgcatacacaacgggccggcttgtcggcgattgtcgcgacatatcgttatcagttagcgaccggagttgtctatcgcgacatatcgtcgactatcgcgacagaaaaaataccgttcgtagagaatgccgtgttgaaggaacgcgcttttattgagacgataaaacagcatcaggagccacaacgtcgaatcccacgtccagtcgattcgtatgttatgctgcacagcaatgctagaataacaaccagcagggtaatcccgcaacataaatacaaagtcacagcgaagaatccgtgtcgttctatcaagcgaaacgcgttccaaacggccccgtcacagacgcagttattcataagcgttaacaaccggtggctaggatgaatatccaaatcacagggcagtagccgacggactcgttgacaggtcagcctaccctcaaggttcctatcgttcggacgggatttgtgcgttttaggcctctttttcgccgcctgcaagcattggtgcgcaaagtcctcacccagctgtttccagctatcatctgcatctgtgcagtcccctgtatcgttgtaacaaacgggtctgtgcgacttcgttctcggaacacaagcttgttgtcgcggagacagagagagaagggttttcgggtcacgcgaagaccgctcaccgggggtcggcaacgcacacatcaacagaaaaccgagacgaatcaagagatccatagtgaaggagtgatatcgacgtgcttacgaaacggcgattatatatgttctcaacaataccgccctacgttgtatgatgtaacgtgtgacgtgagtctgatccaacactgaacgctttcgtcgtgtttttcatgcagcttttacagaccatgacaagcctgacgagagcgttcatcggggcatgaagtacgcattacacaaactccatatatttgttacgatagaatacggaacggaggaggctttcgccacacctatcctgaaagcgttgcattctttatgataggtgtgacgatgtctttaccattcccacggctgctttgcgtgatgatgacattcatcatgtatttccattcacacataccttttgtgcatacggtttatatatgaccatccacgcttataacgaacctaacagtttattagcccttgacaggataggtcaaaagattatatgtaggttttccggtaaaccgaattgtgatatttctctgcaggaaatagaacagcctggtacctataaaacggacaatgcagtactgtagcagcgtaaccaagtaggtccacatgaacacgtacaaaattatggtaagccatcgtttttcataccacagcctgtagctgtcgtacatgaatgaggacggtcgaggaacccagggtagttgtaattgggggcgacattcgtactgtccagaagacaattgcacgggtttcagtgagatgagtactttagcgatgtcggcgggggcgctacgtttcaccgtgacggtgagaacttgaccgtcgttttgtatttcatgaggcacgttatacaagccactggtatcatgaaggatgacctctgatgcgatgtgaggattaaattgtccctcaaaccgccaaacgctggtcatgtttccaccgtcaattacgcagctgacggtgtgagataccacgatgttggacttaggtttgggggctaattgcctttttacaaattcccttctgtattgcaggtcctgctgccactgcttttccgtgcggaaagtcgccatgtcttccacacgtgtggcgacgatagacgccaccaaggtagctaccagaagcagctggatccgcatggcattaccgtatgtcaattagaaagttgagcggacacggttatcgttcctggcggatataagtatataaacgcgagttagcctttcccgtccgttttgtacacccgttccccacacaaatgacgaatacgacctttttttttataaaaataaaccacgtgtattatataaaaacatttacatagaaaagagacacactctagattaattaagggccggccgcatcagcttgatatcgaattcctgcagatctgctagataacttcgtataatgtatgctatacgaagttatgcggccacggatgcatgtttaaactcgacagcgacacacttgcatcggatgcagcccggttaacgtgccggcacggcctgggtaaccaggtattttgtccacataaccgtgcgcaaaatgttgtggataagcaggacacagcagcaatccacagcaggcatacaaccgcacaccgaggttactccgttctacaggttacgacgacatgtcaatacttgcccttgacaggcattgatggaatcgtagtctcacgctgatagtctgatcgacaatacaagtgggaccgtggtcccagaccgataatcagaccgacaacacgagtgggatcgtggtcccagactaataatcagaccgacgatacgagtgggaccgtggtcccagactaataatcagaccgacgatacgagtgggaccgtggttccagactaataatcagaccgacgatacgagtgggaccgtggtcccagactaataatcagaccgacgatacgagtgggaccatggtcccagactaataatcagaccgacgatacgagtgggaccgtggtcccagtctgattatcagaccgacgatacgagtgggaccgtggtcccagactaataatcagaccgacgatacgagtgggaccgtggtcccagactaataatcagaccgacgatacgagtgggaccgtggtcccagtctgattatcagaccgacgatacaagtggaacagtgggcccagagagaatattcaggccagttatgctttctggcctgtaacaaaggacattaagtaaagacagataaacgtagactaaaacgtggtcgcatcagggtgctggcttttcaagttccttaagaatggcctcaattttctctatacactcagttggaacacgagacctgtccaggttaagcaccattttatcgcccttatacaatactgtcgctccaggagcaaactgatgtcgtgagcttaaactagttcttgatgcagatgacgttttaagcacagaagttaaaagagtgataacttcttcagcttcaaatatcaccccagcttttttctgctcatgaaggttagatgcctgctgcttaagtaattcctctttatctgtaaaggctttttgaagtgcatcacctgaccgggcagatagttcaccggggtgagaaaaaagagcaacaactgatttaggcaatttggcggtgttgatacagcgggtaataatcttacgtgaaatattttccgcatcagccagcgcagaaatatttccagcaaattcattctgcaatcggcttgcataacgctgaccacgttcataagcacttgttgggcgataatcgttacccaatctggataatgcagccatctgctcatcatccagctcgccaaccagaacacgataatcactttcggtaagtgcagcagctttacgacggcgactcccatcggcaatttctatgacaccagatactcttcgaccgaacgccggtgtctgttgaccagtcagtagaaaagaagggatgagatcatccagtgcgtcctcagtaagcagctcctggtcacgttcattacctgaccatacccgagaggtcttctcaacactatcaccccggagcacttcaagagtaaacttcacatcccgaccacatacaggcaaagtaatggcattaccgcgagccattactcctacgcgcgcaattaacgaatccaccatcggggcagctggtgtcgataacgaagtatcttcaaccggttgagtattgagcgtatgttttggaataacaggcgcacgcttcattatctaatctcccagcgtggtttaatcagacgatcgaaaatttcattgcagacaggttcccaaatagaaagagcatttctccaggcaccagttgaagagcgttgatcaatggcctgttcaaaaacagttctcatccggatctgacctttaccaacttcatccgtttcacgtacaacattttttagaaccatgcttccccaggcatcccgaatttgctcctccatccacggggactgagagccattactattgctgtatttggtaagcaaaatacgtacatcaggctcgaaccctttaagatcaacgttcttgagcagatcacgaagcatatcgaaaaactgcagtgcggaggtgtagtcaaacaactcagcaggcgtgggaacaatcagcacatcagcagcacatacgacattaatcgtgccgatacccaggttaggcgcgctgtcaataactatgacatcatagtcatgagcaacagtttcaatggccagtcggagcatcaggtgtggatcggtgggcagtttaccttcatcaaatttgcccattaactcagtttcaatacggtgcagagccagacaggaaggaataatgtcaagccccggccagcaagtgggctttattgcataagtgacatcgtccttttccccaagatagaaaggcaggagagtgtcttctgcatgaatatgaagatctggtacccatccgtgatacattgaggctgttccctgggggtcgttaccttccacgagcaaaacacgtagccccttcagagccagatcctgagcaagatgaacagaaactgaggttttgtaaacgccacctttatgggcagcaaccccgatcaccggtggaaatacgtcttcagcacgtcgcaatcgcgtaccaaacacatcacgcatatgattaatttgttcaattgtataaccaacacgttgctcaacccgtcctcgaatttccatatccgggtgcggtagtcgccctgctttctcggcatctctgatagcctgagaagaaaccccaactaaatccgctgcttcacctattctccagcgccgggttattttcctcgcttccgggctgtcatcattaaactgtgcaatggcgatagccttcgtcatttcatgaccagcgtttatgcactggttaagtgtttccatgagtttcattctgaacatcctttaatcattgctttgcgtttttttattaaatcttgcaatttactgcaaagcaacaacaaaatcgcaaagtcatcaaaaaaccgcaaagttgtttaaaataagagcaacactacaaaaggagataagaagagcacatacctcagtcacttattatcactagcgctcgccgcagccgtgtaaccgagcatagcgagcgaactggcgaggaagcaaagaagaactgttctgtcagatagctcttacgctcagcgcaagaagaaatatccaccgtgggaaaaactccaggtagaggtacacacgcggatagccaattcagagtaataaactgtgataatcaaccctcatcaatgatgacgaactaacccccgatatcaggtcacatgacgaagggaaagagaaggaaatcaactgtgacaaactgccctcaaatttggcttccttaaaaattacagttcaaaaagtatgagaaaatccatgcaggctgaaggaaacagcaaaactgtgacaaattaccctcagtaggtcagaacaaatgtgacgaaccaccctcaaatctgtgacagataaccctcagactatcctgtcgtcatggaagtgatatcgcggaaggaaaatacgatatgagtcgtctggcggcctttctttttctcaatgtatgagaggcgcattggagttctgctgttgatctcattaacacagacctgcaggaagcggcggcggaagtcaggcatacgctggtaactttgaggcagctggtaacgctctatgatccagtcgattttcagagagacgatgcctgagccatccggcttacgatactgacacagggattcgtataaacgcatgggcatacggattggtgatttctttttgtttcactaagccgaaactgcgtaaaccggttctgtaaccccgataaagaagggaaatgagatatgggttgatatgtacactgtaaagccctctggatggactgtgcgcacgtttgataaaccaaggaaaagattcatagcctttttcatcgccggcatcctcttcagggcgataaaaaaccacttccttccccgcgaaactcttcaatgcctgccgtatatccttactggcttccgcagaggtcaatccgaatatttcagcatatttagcaacatggatctcgcagataccgtcatgttcctgtagggtgccatcagattttctgatctggtcaacgaacagatacagcatacgtttttgatcccgggagagactatatgccgcctcagtgaggtcgtttgactggacgattcgcgggctatttttacgtttcttgtgattgataaccgctgtttccgccatgacagatccatgtgaagtgtgacaagtttttagattgtcacactaaataaaaaagagtcaataagcagggataactttgtgaaaaaacagcttcttctgagggcaatttgtcacagggttaagggcaatttgtcacagacaggactgtcatttgagggtgatttgtcacactgaaagggcaatttgtcacaacaccttctctagaaccagcatggataaaggcctacaaggcgctctaaaaaagaagatctaaaaactataaaaaaaataattataaaaatatccccgtggataagtggataaccccaagggaagttttttcaggcatcgtgtgtaagcagaatatataagtgctgttccctggtgcttcctcgctcactcgagggcttcgccctgtcgctcgactgcggcgagcactactggctgtaaaaggacagaccacatcatggttctgtgttcattaggttgttctgtccattgctgacataatccgctccacttcaacgtaacaccgcacgaagatttctattgttcctgaaggcatattcaaatcgttttcgttaccgcttgcaggcatcatgacagaacactacttcctataaacgctacacaggctcctgagattaataatgcggatctctacgataatgggagattttcccgactgtttcgttcgcttctcagtggataacagccagcttctctgtttaacagacaaaaacagcatatccactcagttccacatttccatataaaggccaaggcatttattctcaggataattgtttcagcatcgcaaccgcatcagactccggcatcgcaaactgcacccggtgccgggcagccacatccagcgcaaaaaccttcgtgtagacttccgttgaactgatggacttatgtcccatcaggctttgcagaactttcagcggtataccggcatacagcatgtgcatcgcataggaatggcggaacgtatgtggtgtgaccggaacagagaacgtcacaccgtcagcagcagcggcggcaaccgcctccccaatccaggtcctgaccgttctgtccgtcacttcccagatccgcgctttctctgtccttcctgtgcgacggttacgccgctccatgagcttatcgcgaataaatacctgtgacggaagatcacttcgcagaataaataaatcctggtgtccctgttgataccgggaagccctgggccaacttttggcgaaaatgagacgttgatcggcacgtaagaggttccaactttcaccataatgaaataagatcactaccgggcgtattttttgagttatcgagattttcaggagctaaggaagctaaaatggagaaaaaaatcactggatataccaccgttgatatatcccaatggcatcgtaaagaacattttgaggcatttcagtcagttgctcaatgtacctataaccagaccgttcagctggatattacggcctttttaaagaccgtaaagaaaaataagcacaagttttatccggcctttattcacattcttgcccgcctgatgaatgctcatccggaattccgtatggcaatgaaagacggtgagctggtgatatgggatagtgttcacccttgttacaccgttttccatgagcaaactgaaacgttttcatcgctctggagtgaataccacgacgatttccggcagtttctacacatatattcgcaagatgtggcgtgttacggtgaaaacctggcctatttccctaaagggtttattgagaatatgtttttcgtctcagccaatccctgggtgagtttcaccagttttgatttaaacgtggccaatatggacaacttcttcgcccccgttttcaccatgggcaaatattatacgcaaggcgacaaggtgctgatgccgctggcgattcaggttcatcatgccgtttgtgatggcttccatgtcggcagaatgcttaatgaattacaacagtactgcgatgagtggcagggcggggcgtaatttttttaaggcagttattggtgcccttaaacgcctggttgctacgcctgaataagtgataataagcggatgaatggcagaaattcgatgataagctgtcaaacatgagaattggtcgacggcccgggtcgacagttagggtgtggaaagtccccaggctccccagcaggcagaagtatgcaaagcatgcatctcaattagtcagcaaccaggtgtggaaagtccccaggctccccagcaggcagaagtatgcaaagcatgcatctcaattagtcagcaaccatagtcccgcccctaactccgcccatcccgcccctaactccgcccagttccgcccattctccgccccatggctgactaattttttttatttatgcagaggccgaggccgcctcggcctctgagctattccagaagtagtgaggatcgatccaccggtctcgaggaagatgtccaatttactgaccgtacaccaaaatttgcctgcattaccggtcgatgcaacgagtgatgaggttcgcaagaacctgatggacatgttcagggatcgccaggcgttttctgagcatacctggaaaatgcttctgtccgtttgccggtcgtgggcggcatggtgcaagttgaataaccggaaatggtttcccgcagaacctgaagatgttcgcgattatcttctatatcttcaggcgcgcggtctggcagtaaaaactatccagcaacatttgggccagctaaacatgcttcatcgtcggtccgggctgccacgaccaagtgacagcaatgctgtttcactggttatgcggcggatccgaaaagaaaacgttgatgccggtgaacgtgcaaaacaggctctagcgttcgaacgcactgatttcgaccaggttcgttcactcatggaaaatagcgatcgctgccaggatatacgtaatctggcatttctggggattgcttataacaccctgttacgtatagccgaaattgccaggatcagggttaaagatgtaagtatcaaggttacaagacaggtttaaggagaccaatagaaactgggcttgtcgagacagagaagactcttgcgtttctgataggcacctattggtcttactgacatccactttgcctttctctccacagatctcacgtactgacggtgggagaatgttaatccatattggcagaacgaaaacgctggttagcaccgcaggtgtagagaaggcacttagcctgggggtaactaaactggtcgagcgatggatttccgtctctggtgtagctgatgatccgaataactacctgttttgccgggtcagaaaaaatggtgttgccgcgccatctgccaccagccagctatcaactcgcgccctggaagggatttttgaagcaactcatcgattgatttacggcgctaaggatgactctggtcagagatacctggcctggtctggacacagtgcccgtgtcggagccgcgcgagatatggcccgcgctggagtttcaataccggagatcatgcaagctggtggctggaccaatgtaaatattgtcatgaactatatccgtaacctggatagtgaaacaggggcaatggtgcgcctgctggaagatggcgattagcggccgcgactctagatcataatcagccataccacatttgtagaggttttacttgctttaaaaaacctcccacacctccccctgaacctgaaacataaaatgaatgcaattgttgttgttaacttgtttattgcagcttataatggttacaaataaagcaatagcatcacaaatttcacaaataaagcatttttttcactgcattctagttgtggtttgtccaaactcatcaatgtatcttaagcttataacttcgtataatgtatgctatacgaagttatggatcaacataaggacttttcacacttttggggtacacaggcgtgccaccgcagataataagcgctggatacacggtacacagtcctggccagcacgtatcccaacagcagcaccatcgccatctgtatggcgatcacgaccccgagctctaagtgtctgtattcatagtgtagtcgtcgcaggttatccactgaattcccgtagctgaaataacgtatatggtaccgaggctggcaccacatgggtttgcatttggagcacggcaccaaatgcagagtgagatggtccaagtccgtgggcacccactggcgcaaacggaatacggcttcggtggtctccacgaggcactccggggcttgcagacggccccactttcgtccgtgacggcccgaccagccgacccgagccactatccctttctcgggatagaacgtaccctgtacacgccatacagcgtccaacacgccgtctttgacgacgcagctggcctgatagctggacacgttgttaagcggcggaaagcgaaactgacgtgccggcggagccacatagttcggttcaccgtgttgtcgcggttcgtcctccctatagtaatagtagtcgtcgtcctcataggggttgccggcgtgagccagcgttacccaacagcagcccaggccgacgaggaggcgcagccaccgcctcatggcggcttcgccagtcaatcgtctttagcctcttcttcccgtgaggtccttccggtggcgcggtgccgacctcggacccagggacgtatccacctcaggtacacacagtaggctacctggacaccgaagctgaacaaggctacatgtttcacaaactgcaccagtaccacatagaggaatgtcaggtagcgtctctccgcaaacagccgttccaagtctgagggcgttacccgcagcggcaaccagggcagcctggacgccggccggcaatggagcacgctccggttacaggcactgcaggggtaaacggttaacatcacgtaagagagtcgagcgtccacctgtgggagctcagtttcgtaacgtagagccccgtcattttccagctggggtgcgccgaccttgaaatgggtcgcgctccgttcgttaccccaggtgccgtaggctctcggggccgtatcggagaagttgccgtgcacaagccaggcggccacgagtaccccgtgctggacgtaacattcggacacggaactggagacacggtagccggacacgtccccaaacccgcgagggtactggggcagacggacggacttgctatttgacaacggacagatacgagacgacgaggacgcagacgactcgtcgctggaccacgacaaccggagcgactccttggagcggctcgagagtacacttactgcgatcagacaccagtgccagaagaaggaacaggtggacggggaccacaggatcatagccgccggcaccgcggccggccgcaggaagccgcccggcgcgtcgtctgtgtgcgggagccgaaacaccgtgcctctttatatcgtcccgacgtgacgcgagtattacgtgtcaggggaaaaccccgtcatgacgaacgtgattcgtaagtgacgcggggtgctgacggggttcggctcgagaagtgacggagcgcctcacgtcagtatgatgtccgatccgcgtcagccccgacgtggttatggtcaccgaaacccacgtttatatggacgttgagaacagcgcctgaccacatgattcatcataccatttctcggaatcgggcccatgccgggaaagcacattccttttcagtaaacaacaatgacatcataacaaatcattttattcgcgaggtggataataaccgcatatcaggaggagggatcgggtgatgacgcaggccccgcaaaacagtccgaaataaatttttagtatcgccccgtagtcgcctagataccagaggtacgtcaagttcatcaaaacgcccatcggcgtcccggaatcgtataccgggcacacgaagcgttcataacaatcccgggaggcgagtgttagggtagcagaatagtttcggggtcggtttccttccggcgacgacagctccgtgggcagcagaatgtagagcgcctcggtagccgtcgcggtgccttccacgaggatgggctgccggtgcctttcgtgattttctccgtcgtgtagccaagccgaggcccgcaaagtcttaggcgaggggaattgtccatagactttcaccgcacccttcagtacatggttctgaataacacagccgcacgtgaagtaggtcggttctctcgtctcctccgtggctgccgccaccactcccagccaccacaacaggcaggtcgcgagagggttccggaggcttccccggcgtagcatggtttcgggttaaagcaaaaagtctggtgagtcgtttccgagcgactcgagatgcactccgcttcagtctatatatcaccactggtccgaaaacatccagggaaaatgtcggtgcagccaacctttcacatacagcccccaaaacacttgaatcactgccaccatcatcagcgtatactgcgccgacttaatcgtgagcgcgtagtacgccattagacggcgatcttcgaacaatagtcgttcgatgtcctctaacgagctccacagaggaacccaaggcacgaggcaccggggttcgcactctacataataagtttggcattggtggcagggggaaaagtagaacaacacgagttttgtgcgttggggaacacgatagtcccggagccagtagcgttttgcgacgaggctttcggagacgtcctccaccggcgtcggcactcgatccgcgtagccctccagcgtctggtagtacacccggggtgtcggcgtgggcacggacaggttcccgcgcagggtccacagagcctccagtcgaccgcccgatcggagcacgcagcgcgcctcggaatactctactcggtactccgaaacatcgggcagaggcggtaacggctccgtctccaccaagggcggaggttcatcgaaaagagtcaaggataattcaggcatactacctgcgaccggggcccagagggctaggataagcattacaagattcattctgtcttacaagggaaggctgttcccctgtctagactcaaaagctgtaaggctgtcttatagcatgtagtcttgcacgtcacggggaacagggtggtgatctagtgacgtcgggagaacacggtgttttagggtgcgggggacaaaggacagtacgacagattaggtgatagaaacgtttttttttatttatgaaaaagccagtgtgccgtgcggcctagggccccggcgtagtttggataccagatgggggccgtcaggggtactaccacgagcagaaacataataacttggtccatgtatagcagcatagcggtgcgtagcaggtcgccgtccgtgtagcaatttgacggtgagcgataaagcaccgttaatgtgtcgcggataagcacgatcttgaggccgtagatgaagctcacagtcagtgctaaaatgatgcgttggtatggttcccaggactgcacggcgatgaagagccagagtatgggaagcatgaagcttagcaaacagaggatggctaaccgtcgttgcatgttccaggccatgagccaggctaggcccgtacaccagacgcagagcatggatgacaggacataggcctggattaccacggtgcgatcgaaacacagcccgatggtggacacggatatcgtagtgagggtggtatataccatgaccagcatcagggtcccgggtaggcgccgacgttccagccagtacgcgtggcaacgcagagcgcagggtagcagtgtgctccagaagggcagtgtatcgcgcaggtagggggtcgtcacgcgccacggtatgagcatgaaaaggatggtagtggctatggtggcgctggtctggaacacgacggtgccgtagagacgtaccatccagagaaagtgttgaacgctccgcagggtgtcttcatctttggtgattacggtgactcgacggatcggcggtggtgacggcggcgacacgggtgggggtttctctttcttatggccgagtggctcgccttggtgaaactggatctgtaccatgacgggtgctcgacgaacagtcgtcggggctttaggtacccggcaagttttatagagaaagggggacgatgggtggtggctacgagccaccgccaccttcgcaatacgaggatctgaaggcggcaaagacggtcgtccagggcaggtgccagaggttgggactgagcacgatcagcgtgattttaaacatggtcaccagtcctacgtagatcagcagcgagccacgtaacgtctgagcagccggcagttcgtcgcggatgtaacgcgtgccgtagaaagtcacggtcatcataaggaagacgatggcgccgtagccgtagagtagaatacgctgatgatggaacacggtctggtcgccgataacccagagcgtgatgaaaaaaacgctggtgagcacccgtgtgcatatgagctcccaacgcttagcgcgaaagctgtccccaaccatgacagcgccggtgcaagctatccacagcgtgaggaccagtgtgtagtcgatgaggatggcgggcaggtcggagcaccaggtgtagaaaaccgtggtaacggagaggaggcctacgtagcccatggtcaataccacgtcgtcggggtgcctttcgccctgtatcaagaccaaacaccagagaagggagggggcaaaaaccagcagcagaggggaagattcatgttgacatatgttgtgggaatcggggatgcccagccaaatcattccgcagaaagccgtactgatggcgatgtgaaagaccactagggcgtagacccggacgaggacagcaaaacggcgcagccacataaggccgtggtgcagctgcaggagagaagcccattgcggcgaatgtagcgacggcagcggcgggtccatgaggcgggtgatgcacccgagtgaacgggtgagcgtctcggtggagtcttcttataaaccagcggagctcaggcagtcttgctctggagcgtcgcagtggtggtgttgaggatgacgctgagcgtgccgttgtcaatccggtaatgatgataggtgccaagcttggccaggtagctgaacatttggtcccagcgtgccgaccacaccacgggcgtgagcatcaggagtgtggtgtgataaatgagtgtttcggtggcgtaaagtatcagcgagctgcggatgatgtggctcacgggcattttggtggcgatgtagcgcacgtcttggaaaagaacggccaggatgcagcccacgaacacggtatagagacacagcagagtcttatgcaaccaggtgtaagtagaagccaggacgctgaccatcaccgtcaaaagtgtggaggtaaaaagcgcgtcacgccacacggagctgagacggtgctcccaagccacgccgttgcaggccacgaacaacgtccacgttaagatgaggctggaaacgccaatgggcgctgtggcgcacaggttgagcccggcggtggtgaacgacagaagcgccacatacagcgcaaacaccaggccgttgctggggtgtctatgatcggtaagctccagcgcgcccagaaccaacaccggtgtgcagctaagcaataacggcgaaggatcgtcgcggcactcgtagcccagcgaggggtaacccagccaaaccagcgcgctaatgagcacgctaaaagcggtttccagcgtcagcaatccgtagacacgcatgacgatcgcggtccgccgtagccaacacaccgcatcttcggaagctgtggacgctgtttccgaataccgggaggagatcgtgcttccctcttccaaggatcggaaagtagcgtccgtcgtttccgcagacgcggcttccctggtacgctccgtttccgacgacgcggtttcccgctgcgtggaaactgtctccatgtcgggaccgcagcgcccggcggcgtatccgcaaggtctcgaagctacagcttgtcagaggaaaagtaggtttgcaaaaaggtgcgcagggtcatgattctcagcaccatcagcagagtgaaaaccaggctgagaaacaccttgacggccgccaaaagcgcgcgttccagcggcgtctcgtagcgtacagccagggccgcttcgtggaaatgcgagacggctagacaggtaatgagcacgctgaaggacaagacgatcttaaagcaccaggaccaaccacgcctcaagatgaccaccacgattgccgtgaaggtcaacgtgatcaaagcatggatgaccacgatctgacggcggacggtacgttcgggagccaacaacgctacgccggtgcagctgagaaaggccagtaaggtgaacaacgcggccgagatgaccaacgtaccgtccaggcagagacatatcacgatcaacggcggcacgtgaagcagcgtgtaaaagagcagaacgccgatattgctgggatgcgatgtttcgtaacagtgaatgaagatcaccgacgtgacgggtatgataaagacgaggctgggcgaggactccgtgagacacagacgggaatggtgaaaccacgtcgcgggcgccgcgtagcagaaggcgctcaacaacgcggtcaagccggccagctgccaacccacggcgccataggtgtgcagcgccacgcggcaacagtcgacccaagccagactgcgggtcgccagccgggtctcttggatcccggggggcacgtagatgaccgtgccatcggtgggtacctgaaaccctttttctcttctcatggtgcgctgcgttctctggaaacggctgctctgtccgaaaaccagttccgaacgaaaatctagggcgagagggtggacaacggcgtcgacgacgaagcatgggacaggtcgttcggcgttaacgtcatcgcgtcggacgacggtagttctaagagacgtagatcgctcagcaggtcctgacagttgcggattcgcaagatcagaaaaaaaagggaaatgaacgtaataaagagctgtagcgacgtatgcgctacatcgcgtggcataagaacgtgacggacgaaaaggacctgctgcgaaaagtggccggcaaagataaggcccaccgtgctgtagaagcccaaaagcagccgcaggggccaagtccagggccgcgtaaagacgatgagaacgttaaccagaaagaccacgacccagacgccgttgatgagggtaaattgatcggacagggtgcagttgtcgcgacagatgaagactacttccgcgcagagcaaggtgatgaccaatgtgagcacaaacgacgtcaacacctcgcggggctcctggcaggcacacgtgacacctagcgccgggatgtgcgccaggaggccggcgagtaatagcaccagctgtcggaacggacgacggcagcgcgggtgccggtttcgctgagcgagaaccggtcgctcataacggaaatacacgaagagcgcggaggccacaggcaccaggaggagcacctcgggcgcccagacgacgtgacaaggaaagcctggacgcgacttaagagtcgctgtagggaagaccagagagaagctacccaagacggccaccgccgcggagatttggaagaggagcaagccggcgattcggacgacaacctcgaagcgatgcacccagcccagcacggccaccacggccgcttcatcatagtcgtcgttgttgccgctgtcgaacagccgccgaaacacgatctgtcgctgggtcgcggtgggaaagcgcagacccatgacagccggaggctatatgaccgcgcgtctaaggcgcgagatccgtggggggacttttagatgtttgggcggcccgcggttctaacaggcttgattggtggagacggccggcgcggcgggtgggggaaacgacgagtttttccgttacgccatggttcgcgtgaggtttctctgtacctcccgcaaaaggtcacagcccgaaatggaggccgcgttggtggccccggtggcgcgtgacgataaccaggtcatccaagtgatgagtttgtctaatgagtcctcggtggtgaagaggataagaatgagcaggtacaagtacaccaggttctcatagagacacaaggtgagcaggtcggcctcggaccacgcgatctcaaacaggcgtgtggtgtcaaagaccgtaacgaccagcatgaagctgagcgccatggcgtaatagcccaaaaaaagtttgtgccccaacggtacgggctgcaggtaaagtgcgatcaagaacgcgataacgccgatcacaaacagcgtgacgatgacctgccatcgacggcgattatggccggctagacccgtgacgcagctgcagaggctaaaaagcacgcaagccaagaggcccgagaaggtcaccagcgtagaggaggagcaggcgctggccacgatcaccgaaagcgtcgtgagcacgctataaatggtgagcaggcccgggctcggcggcgacgtaaacgatccttcatcgcgtttgccatgcagcagggccaaacagatggtgggcaccatcaaactcaagggcggcataaagccggtgcaacagagaaagacggtgcctttaagatgcggaaaagccagcaccaggcccagacagagcaagaaggtgcaggtgccctgcacggccacggtgctgtagacccgcatacaaagtaaaaagcgacgtacgtcgttcgtcgagacggaggaaatcataatgactccgcgcgagggtcgcgggggtgggggcgcccaggccgtcccggtggcctctgagttcggagacatgacggcggtggctatcaaaaggcgcgtatgagaaaccgtttatagagtgtaatagaatcaccgtcattcccacacggcgttcccccataaagtcacgtcacactcgagtaagcgtgaaaaagctttattattgaataaaaaacacgagtacaacaccgagttgcggtgtcctgtctactgggtgggggaggtttatcgtctgtctctagagggaaggtggggaacgtctaagcgagcgggagcgtgtcatctcccccatctttttacaacaagctgaggagactcacgccgtcgatgcgtccgccgtgtttctcggcgtactgctgcacccagacgtggccgctaaagatggcgacgctcatgtttaggagactcatgacgatggtgtacaacacgacgctgacacagacgctgtttttagacagcgttccacgctggtagatgagatccagggtctcgtaaataagcacggccgaagcggcggtcaccaccaggacgtagagtccgctgtagatcttgctgacccacagcacgggcgaaaagtaaagcaataggtaaaagacgatgacggaccagccgtagccaatcccgatgactttccagcgcgtgggattgttgccggccaggtaggtgagaccgctgcagagaacgaaaaagaccatcaccagggcaaacgacagaccgatgacgcgcctttctccgcaaaagcccgtgcacacggtgatgccggtgttgatcagcaggcatgccaccgtgagatgagcaaaattggtggtgtgtgggcgaaactcggcgaaaccgcgtagcatggccagcgtggacacgggcacgatggaggacagggctggcactatgccgttggcgcactgtccctgcacatcggggaaggcgagccaagccagcaggcagaccgtgagggtacaagccagctgccacacgagcccgtgatagacctccatgagcagcttgaagcgtttcaaccactggaagagctgctgttcggccaccagcgcgtggctgcgatggagcggcacgatggtgaccgtcggcgactcatggtgttcggaaaccgaggcggtgtcgcccatgctgccgcttacgaccgctgtcggtctaaggtaggcgtcgatgaaacagtccgtcttatcagcacccggttaccgcggatttgattgacgtcacgagtgtggtcaaaccgtggcggcaccctgtatccgacccgtcgtcatgggctccacaaccagagcctcagaagatggtacatgccgatgaataaagccacattttcgacatagaggcgtagcgagggctgaaaactctccgggaaagaactctgacaggtgatcagggacagatcgtgaattagcatcagcgtcaccgtcaacagcgtcgtcgcgtgtaaaccgagaaagaacggggtcgcggcccgcagcagccaaagtcccagcgccgtagcgcagagcagagacaggaccgacggtagccacagccgccggagagacgcgccaggatcgcaacccaaaagcgaggcccccaggcagccgagatctaccgccagggcgagaagagccgcgccgagaaaggcctgcggcgacggctggcacatcagcaaggtcagaaaggctagcgcgtgcggcaggcagtaagccaacaggagtgggagtttgcggggacaacggtcgatagacggaccgcgtagcagcaggaacaggcagccgacgggcacgacgaggctgagatgagaaagcggcggtgggtcgtcgtcccgtccccgctcgcatagctcggccaccggtggcggcatgagccaccagctgagcacgctgagggcgacggtggcggtaagctggaaggcgacgaggacggaggcgcgcagccataccgccagcctctctaagtaggggactacctcctcgacggtccattctagcgggacgacatgaagcatggcgacaagcgcggctgctgtgaaaatgagcgcggttttataggcattaggacttcccgatcgtactggcggctgtcaaagtcccgttgtccaaagacgcgccgtccgaaagactaatccaacggggacccgagagcatgagcaacaacgtgagaaagatggccatgctgtccaggtagagacagacggcatgacggatgcactggttaggtgggcagaaaaagatgaccatgagactgtcgtaggccagaatacccaaaaagaagctgatggagaaggcgcacaacgtcaccactatcttctgcagccagtcggcgtcgcttagcagagcgagcgtgaggaacgaaagcagcatcaccacgtagacgcagctgatgcatttccaacgacgtcggtcacggccacctagaaacgccagccccgtaaaggagataaacaacgccagggtcatcacgtaggaacctactagtacgcggctttcagagcacatttggaagatggccgccgtcaggctgttggccaacagatagatgaaaagcaccgtggcgttactagggtgctcgttgcccaaagtgtacgtgatgaacatgcagacgatgggcacgagcacggtgagaaagaagctgtagttctcgacgcaaaagttgcggttttgtgggaaccccaaccaaaaaacgcttcccaagccgaagctgaaagccaactgaaagatgaagatggcgtacacacgcagccatacggtgaactttttgaaccactcgagagcctccatgcgggagagcagcagcgcgttagcctcctgcgcctgcatggtggcgacggtctcggcacaaagccgctgcggcgcacctacccttctcttatacacaagcgagcgagtggggcacggtgacgtggtcacgccgcggacacgtcgattaggagacgaactggggcgacgccgctgctgtggcagcgaccgtcgtagcgaccgtcgtctgagcagtgtgggcgctgccgggctcggagggcatgaagtagagcacggagacaaagaggtacatgaggtccatgtacaagcagagcgcgcccgggatataactctcatactcgatgtcgtgcaggatgtcctgcgtatcgcacaccaccgaggtcacgatgacggccaaaccggctatcatcaccaggatctcacttaccgcctcgggaaaaagagaaaatacggcgaacagtaagagaatcagcgtggatgcgcccgtcaatagggaacgctgtaattccacgtcgcgggcaaacagatacgtagcgagcgtaaggaaacaaaatagcgttactgtggccaccatggcataaatgactgaacgatgactaaaatggaagcctgacgccgtgacagccacgctggtaagcaacgtgtacgtcagtaagatccatacgtttttgggaaagttgggctcggcccaacgcaacagacctaggcacacgatggagatcattaagcaagacagcgtcagacgcacgctggaaaagagctgctccagccggtgcggcaacaccagccagcaaaaggcgcagacgctcataaggatgaggcattgcacccagataaggatgtagatgcgcagcaggaagaccgaccgggctatctggacctgaccgcggagcgacatggcggcaacgccggcggttatcgccgagattcgtctaaatacacgaagcgaactagaaaacgcacacacgttatttgcaaaaagaaagcagctgccggcttattattttattaaaaatttatctgtgcagaatcataagtttatgatgaataaaaacggggaaagggaatctgcttttagggacccgggtctggtccgtcgtctcccatctggtcgggttcggggatggggacctgtttcagcgtgtgtccgcgggcgtgcatggcttttgctcgccggccgcgctgtaaccaggcctctttctctgtggtcggcgagtcttccgacgggtagggagtctgggagtccatcgcttcaggcccaccgctcgttccctcgaccgtcgtgtcgtcctcgttttcgctattacacggggtttctggagtatcgcctatacggttggcgattctccgggggtggccgctctcgtcctcgtcgctgctatcgccgcccggtaattcgacgccgcattcgttgtacggagcgcggcacatgggcggcggaaagaacttgggcatgcgaaagcagcgttgtccatccacggtctgcgtggtttcatcattatcctcccataatcccccctgtagcgccggcagcgtttcgacgctgtgagaggggaaggcccagttctggttgtcttgcagcgcgcccgtgggcagtaggtccgtgcggccccaggcgctgctgttgttgggtaccttgtcagtgccgcgagtaggtcgcagaaaccagtccagagcgctctctagctgcgagcgtgtgatggtgcccagtgcgccgtgccagcgcagcacgtctcttttcagcgtgtggtgacagacgggcagctcctccaaccgacactcgccgcgcaatccgcggtcgaagcggcagagaccacgcaatttaagcagaccgcacttgagaaacatgtgaaaattatcggcaatgcgatacaggtctgagtcctcgatcttgtgtaggtagaccacgccaaacttgtcgagcagcaccaggccgctgggcacaaaaggcccgtaggccaggtaatagcccacgaggccgacgacgtaccactcgcagcacaagcgttgacgaataaagttcagaagatcgcgaaagtccgcggccggcatgtggtcaaaaggccggcaggcgcgcaggccctcgatggagcccagcatgagcaacggctccacctcggtgcgacccggcgtgcggatgaccaggttgagaccgctcatttcgcgggccgtcttggccacggccgcagcgtcagtggggtcggtgcagaggaatttttgcacatgatagcgcggttcggtggtggcgaacggcgtttgtgggtgccgatacacatattcgcaccagagtaggccgttcttggaaaaggctttgatatcactggccacctcgtagagcccgtcggtctcccagtcgtagacgtagacggtgccgtaatgacttagcatgagcacgcagggcagttcctgcgcctgcttggtgtttcgtgttagatcgctgtcgggtggacgcacggctagtacaccgacggcttccagggtgtcatcgcagcagagatagtcggcggccagagaacgtgcgtaaatctgcgggatggcggcctgttcgcgcatcactaggaaccagttggcggggttgcgcagtgctacggtggttccttggtggcgctgcacgtaggttctcagcgccggaggatcgtactggcgcagatagaggccttgcagcatcgataacgtcttttgaaagacggtgtttctaaattggaaaacgccgtagtcgcagcggatagcatcttcgcagcgctcgtcgcgctgtcggagataggtgccccaggcttcggcggcggctttggtgagtagggacatgccggcggagccgtctcgacagcgagtcggataaagcgcgctgcgcgaaagcttaatataggagcagcgtcagacgaatcgcggctggtggcccggggggtgggacgcgccgcctacacaaaatgctcccgaaaatcgaaactcttgacccactccggagacaaatccgtattcagattgatgcgtcgcgcttccacttcggcttccgaaacctcggcctccgtccggtaggcgttaacaatacgctgacccaggtgccaacgctctttctctgccaaacgccgttgctcaaaccactcgtctacgtccttgaggtcaaagacagtgtcctcctcaaggtcaaagcctaggtcttcccactcgtcgtcatcgctctcgtggccggcggccatacgcgcggcaaccgcgtcttcccctcctcttctttcaacgttgggtaccacgttgttttcttcgggttccatgggttctgcgccactatcgtcatcgtcctctccctgctcctcatcgtccgccaaggcgtcgtggatcacctccaggttctgattgtcgggtacgacgtggttatcttcgtcgtcgtcgcgtggcatgggcggcggccgacggcggacgaccggcatggcgcggccgtcgtttccttcgtcttcctcttcaccgtctcccaaggaacgcggtcgacgacgttccgcgaagtcgccgcggaccacgcgcgcctgccaaatggtaaacgcgtcccaaccgtcccagttattgagcatttcggcgcgaaaacggtcgcctcgacagagccagcgaaactgccgcgcgtagtcgcggtctacgccgctgtcgaacatggtaaagtgcagacgcgccgcctcgcccatgtgtacgcagcctccattgcgttccagcctggccgcgcgccgcagaccgtgttcgtagcggcgacgcacgtacaccttcatgaggccggcgcgaaaaagttcctctaggctgtcggccagacggtagatttcaccggctagacgctgcaggggcggcgagcggtccagatgcgacttgacaatcaccacgtaaaaacgacagaaacggtcgaagatgatgaggaaggacgtgtcaaagaaaccaccggcgcggtaggagcccacggcgcctagcaggtaccagcggcaacgcagttgcagcgtgacgtacatttcgcactcggccaagcgggcggctggcgctacctcgaagggccagcaatccgtcaagcagccgaaactggtcaggagtttcaacgttttggcatggcgcccaggtgtgtgaaagttcacgtcgcgtccgtggtgttcgccaacgcaggcggccaacgcgtcggcgtcatgagcgtgacgcagcagcatcgctaccacgtcgtgcggtacccgcgtagcaaacggcgtctgtggctgacggtatacggcttcggtgtacatcataccgtaacgtgccagctcgtccagatgacgcgcgcacagcagcagaatctcttgcgagggttcgtagatgtagaggcgcgtaccgccccccatgcagagcaccagctccgtctcttcgtagtgatcttccaccatgatcacgcacttgcctagcacgataaggcgttcggggcaacaaatcacgtcgtccagcagttggtcgcgcagctccggcatggtgctgccaggccgcacctgcaggaaccagttgtgcggaatgccgagcgacaacacctggtcgacgtggttacggacccagtcgcgaagcacgtcggcgctgtactggcactcaaagatgccctgaaagtcgctcatgacccgcagaaaagtttcgtagcgcgtgtggcaatagaggaattcatcgtttcgcgtgaacgtgggagctccgtcttcccaacgtgtacgccacatgtcaaaagaggccgccagctagacaccccagaaaagaagcagagaaagagagttctttgtgcgacacgttttattccgcgtcctccgctcgacgctcaaatctggatgtactcgcgcacacccgtcaggctctttaagggaaaagggtccgagtacgtcactaaccgcgactgatgcaccagggcggtaatcacccgctctgcgccctcgcgcgtcgacgaacgcgtcgtcaccaggcagtgcagccgcgggcccgtatcgtcctgatgaccagcggcctcgcgctcggctgcttccacaccgacaatgtcgggatccaacacgtagctctgcgagttggtgtcgtagcggtgtaacaccaacgtgttggggtccagacgctcccacgcgccctcgtgcgggtcaaaacgctccgttaaacagagccagtcatactgctgctgcagaatacgccgctcgcgctcgcgtcgctcatcgggcaacgcagcgtcttcgttgaagagaatgtcccgcttgtggtctacggcacgctcgtggtggtgcgggcacagatgacggtgttccatacgcgtctgacgctgacgctcgcgttcgaagcgccggtgtcgaaagaccattttcagcaaccccatgcggaaaaactccgtgatggtgttggcaacgcgccgcacatagtggttggggtcgtccatctggatggcgtacacggcaccgaaccagtccagcagtaccagcacttcggccacaaagttgcgtcccggtcgcggacgtcccgtcacgcctagcacataccacggcgtggccagattagcacggacagcccaccaccaacgacggctctccacctcggtgagcgcacagaagggccaaatgcggtgtaactgctgcaccgttttcatcagccgcataatcaccgtaccgtaacccggtgtatgcaacttcacgtcgcaacccaggattcgttcggccgtggcgtacgagccctcgggcgtggtgtcattgagaaacaaaacatgcatggtacgcgcgcccttagggtatcgtcgcggaacaggtaccgtcattctccgcagagtggtgtgaatcacgtcgcgatacgcaatctccgaacgcgacacaccgtaacgtgccagttcatccaagttgtgcgatactaacaccatgtacttttcacgagtgtcgtaggcgtagacgcgagaaaagcgacccataaaaaccacgtacggggtagccaccatgccatcatggtgatcgcgacgtggctcgggcaacaaaataacagcgtatcccaacggcgtcagcggctcgcggcaacagatgagctttgacgccgcctgtctggcggcggtaatgatcccgtcctccgtacgtaacatcacatgccagcccttggggggacccaaggacagacaacgtccctcgttacgatgaacgtaacgcgtgatttccattggctccaggcaaaagaacagttccttaaaatcccgcaacacttgtcggtataacgccatgggatcctcggccgccacaggcagcgcggggagctccggcggcacaactgcagcgccgtcagggccagaacccgcagccggatccatcattacgcgacactctcagccggacaaccggcgtcactgacagaagccgagccaaatacagagaaagcaacgctacaccgtcaccccgctcccaagcgccgcggaaagtgctccgatttttcaccgtcgttcgcgacgttgatttgcctcggtctgagaaccgacctagcgttcggaccggtgcgcagaaacagccggcggtccgagccactgagcggttcacagccccggccgccgatagttaccggagagacgttcgagctgcaggtacatcggcgctccccgcttcgccaccccgcgcccgccccagtttatactctccgacgccccgtccaacgcgcctgtggagggccaatcggaccgcgggagctctccaagtggatgacaggcacagccgggtgcccgaccgtgaagagccctcatccacctgaacagaccgctaaccgaaggaccccgagtcgcgtccgtcggtcccgacgtccgtcgccatctggctccctgctgttggctacctctcggatttcaaaaaagagcacgtgccgatgacggtgcacaggaaagagccaaagtgtcacggcgtctttttttatttgtattcctttcctgttttgtactcgtaaactgttgacgttgtttttacatccaaaagggcaagtaagaaacaggatgaggcatggtaggtttgggcgtggggcggccctccagcacggcggcccgggccgcccggcgggtgagcacccggcgttgcgccgtatctatcttgtgtttcttctgtgtctttttcctatcttgttccgcgacggcctctttcatcacgttcagcatgcgttcctcgacgccctccagggatcctggggaggagggagtcctagtgaggcttccaatgttgttttgtggattttcggtttcctcttcttggtcgtcatcgtcggacgtgtcgtcttcctcttgatcctcttcttcgtccgagtagtagacgcatagtccctggttcatcaggctgggattcatcaggttctgacggggaatccgctgttgtagacgtttaaccgcccgttccaggcgagagctcatgccgcaccagacgctgtaacgccgcacgggcccgtagcgggctgtttgttcgcgtacatgatcgttgagctcttgccaatattgtttggcacactccagatcggaggtttgtggatagtcgggtcggatccgcggatcccaactgacatcggcggtgccagagacttcgtccagactgttacgcatagagcaccagtcgggtcggacgataaacctgtccttgcggattaaccatttataacgtagttcgtgatggcgtgtagaggcccgtacacgctccacggtcccaaagcggtcccagaagggaaagttttcgtgggggcagcgacccggcacttccaaacgttcggcgtcgtccacggcgtagtggaaacgccggccggcctggtaaattttgagcagacccacggttaacaacatatccacgctgtcagccaaccgccagatctcgcgccgagatacgtcaaaatagaaaaattcgcaggctcggtcgaccaggatcacgaaatcggcgtgaaaaacgccggagggtagcgactcgcccaccacacccattatcatggtttcacagcataagcggtccacaaagaacttcaacaggtcgttgaattgctccgtctccatacagatgaagggccagacgcctttgaggttctcggcctggccgcagagcagcaacggacgcgtcatctcgcctggagtgcgcagaggcacgcattcgccgcgataacgacaggtcacacgctgcagttcgctgatgctgttgtcgtgcaggcgaaggtcgcagataatatgatccggttgcgtggttagcagcggcgtgcgcatttgctcgccgtagatggcctcgcagtgcaatagcccgtgtcgtgcaaaatcgtccagactgtgcgccaggtagtaaagcaccccgcgatcgcggtctagacaccacacggtttcgtaacgtcctagcagaagcaccagacgggcctggctaggtggctcaatttcctctacatacacgaaaaagtcgtcatcgtccgagtcctcgtcctcagaagaggaccgcggcccgtgtactctgggcaacacggtggtagagaactgcaggacgcccagagactcgagcgactcttcgcagcagatgagctgaccccagggcgtttctggcccgtcggtgacagccgcgctgccaaagatgtcctcaaactctacaaaatctagacgccatccgggtggcgctgaaacgggaaggctaatgttcatatcagcatagctacgaactaagtggcggatgtcctgccgcaagtcttggcagagaatgagctttcgtaaacccttgagggtcctccgaacaacggccccagacgcgtagcgataggactggcgcatggtgccgcggcgtggagcggcacttggcagcctattttatggagtttcttcagtgacgtggcttgttcacgtcgttcgtgggctgcggttggcagctccggtctgtaaaccacccgaaaagactgacatcgacgtcaaagacccacgtaatttggaacatgtgcgaccgcaaagtgcgtcagaataacacgtggctttaggacataaaaagtaccgtgaggtccagacgtggtttttgtgattgacacttacaccaggtaagccaagggacggtgaaactgtatgtgaggaacctgggtgcttagacgactaacgtgtaatgctttttacaggactgttcgacaggtgatagtacctgtaaggtgatgaccacctctacaaataatcaaaccttaacacaggtgagcaacatgacaaaccacaccttaaacagcaccgaaatttatcagttgttcgagtacactcggctcggagtatggttgatgtgcatcgtgggcacgtttctgaacgtgctggtgattaccaccatcctgtactaccgtcgtaagaaaaaatctccgagcgatacttacatctgcaacctggctgtagccgatctgttgattgtcgtcggcctgccgttttttctagaatatgccaagcatcaccccaaactcagccgagaggtggtttgttcgggactcaatgcttgtttctacatctgtctttttgccggcgtttgttttctcatcaacctgtcgatggatcgctactgcgtcatcgtctggggtgtagaattgaaccgcgtccgaaataacaagcgggctacctgttgggtggtgattttttggatactagccgtgcttatggggatgccacattacctgatgtacagccataccaacaacgagtgtgttggtgaattcgctaacgagacttcgggttggttccccgtgtttttgaataccaaagttaacatttgcggctacctggcgcccattgcgctgatggcgtacacgtacaaccgtatggtgcggtttatcattaactacgttggtaaatggcacatgcagacgctccacgttcttttggttgtggttgtgtcttttgccagtttttggtttcctttcaacctggcgctatttttagaatccatccgtcttctggcgggagtgtacaatgacacacttcaaaacgttattatcttctgtctatacgtcggtcagtttttggcctacgttcgcgcttgtctgaatcctgggatctacatcctagtaggcactcaaatgaggaaggacatgtggacaaccctaagggtattcgcctgttgctgcgtgaagcaggagataccttaccaggacattgatattgagctacaaaaggacatacaaagaagggccaaaaacaccaaacgtacccattatgacagaaaacatgcacctatggagtccggggaggaggaatttctgttgtaattcgatcctctctcacgcgtccgccgcacatctatttttgctaattgcacgtttcttcgtggtcacgtcggctcgaagaggttggtgtgaaaacgtcatctcgccgacgtggtgaaccgctcatatagaccaaaccggacgctgcctcagtctctcggtgcgtggaccagacggcgtccatgcaccgagggcagaactggtgctaccatgacgccgacgacgacgaccgcggaactcacgacggagtttgactacgatgaagccgcgactccttgtgttttcaccgacgtgcttaatcagtcaaagccggtcacgttgtttctgtacggcgttgtctttatcttcggttccatcggcaactttttggtgatcttcaccatcacctggcgacgtcggattcaatgctccggcgatgtttactttatcaacctcgcggccgccgatttgcttttcgtttgtacactacctctgtggatgcaatacctcctagatcacaactccctagccagcgtgccgtgtacgttactcactgcctgtttctacgtggctatgtttgccagtttgtgttttattacggagattgcactcgatcgctactacgctattgtttacatgagatatcggcctgtaaaacaggcctgccttttcagtattttttggtggatctttgccgtgatcatcgccattccacactttatggtggtgaccaaaaaaaacaatcaatgtatgaccgactacgactacttagaggtcagttacccgatcatcctcaacgtagaactcatgctcggtgctttcgtgatcccgctcagtgtcatcagctactgctactaccgcatttccagaatcgttgcggtgtctcagtcacgccacaaaggtcgcattgtacgggtacttatagcggtcgtgcttgtctttatcatcttttggctgccgtaccacctgacgctgtttgtggacacgttgaaactgctcaaatggatctccagcagctgcgagttcgaaaaatcactcaagcgcgcgctcatcttgaccgagtcactcgccttttgtcactgttgtctcaatccgctgctgtacgtcttcgtgggcaccaagtttcggcaagaactgcactgtctgctggccgagtttcgccagcgactcttttcccgcgatgtatcctggtaccacagcatgagcttttcgcgtcggagctcgccgagccgaagagagacgtcttccgacacgctgtccgacgaggtgtgtcgcgtctcacaaattataccgtaataaaaaagcgctacctcggccttttcatacaaaccccgtgtccgccccttttttccccgtgcccgatatacacgatattaaacccacgaccatttccgttcgattagcgaaccggaaaagtttatggggaaaaagacgtaggaaaggatcatgtagaaaaaacatgcggtgtttccgatggtggctctacagtgggtggtggtggctcacgtttggatgtgctcggaccgtgacggtgggtttcgtcgcgcccacggtccgggcacaatcaaccgtggtccgctctgagccggctccgccgtcggaaacccgacgagacaacaatgacacgtcttacttcagcggcacctctttccattcttccgtgtcccctgccacctcagtggaccgtcaatttcgacggaccacgtacgaccgttgggacggtcgacgttggctgcgcacccgctacgggaacgccagcgcctgcgtgacgggcacccaatggagcaccaacttttttttctctcagtgtgagcactaccctagtttcgtgaaactcaacggggtgcagcgctggacacctgttcggagacctatgggcgaggttgcctactacgggggttgttgtatggtgggcgggggtaatcgtgcgtatgtgatactcgtgagcggttacgggaccgccagctacggcaacgctttacgcgtggattttgggcgcggcaactgcacggcgccgaaacgcacctaccctcggcgcctggaactgcacgatggccgcacagaccctagccgttgcgatccctaccaagtgtatttctacggtctgcagtgtcctgagcaactggttatcaccgcccacggcggcgtgggtatgcgccgctgtcctaccggctctcgtcccaccccgtcccggccccaccggcatgacttggagaacgagctacatggtctgtgtgtggatcttctggtgtgcgtccttttattagctctgctgctgttggagctcgttcccatggaagccgtgcgtcacccgctgcttttctggcgacgcgtggcgttatcgtcgtccacttccaaggtggaccgcgccgtcaagctgtgtcttcggcgcatgctgggtctgccgccgccaccgtcagtcgcaccacctggggaaaagaaggagctaccggctcaggcggccttgtcgccgccactgaccacctggtcactaccgccgtttccgtccacgcggatacctgacagtccgccgccaccgtaccagcttcgtcacgccacgtcactagtgacggtacccacgttgctgttatatacgtcatccgacatcggtgacacagcttcagaaacaacgtgtgtggcgcacgctacttatggggaacccccggagcccgctcgatcgacggctacggttcaggaatgtaccgttcttaccgctccaaattgcggcatcgtcaacaacgacggcgcggtctctgaaggccaagaccatggagatgcggttcaccatagcctggatgtggtttcccagtgtgctgctgatactggggttgttgacgcctccgagtaacggctgcactgttgatgtcggacgaaacatgtccattcgagaacagtgccgccttcgaaacggtgcgacgttctccaagggagacatcgaaggtaacttcagtgggcccgtcgtcgtggagttggactacgaagacatcgatattactggcgaacggcagcgacttcggttccacctcagcggactcgggtgtcctacaagggagaaaataagaaaagataatgaaagcgacgtcaacggtggaattcgctgggctctatatatacaaaccggcgacgccaagtacggtattcgtaatcagcatttgagtatacggttaatgtatcctggggaaaaaaatacacaacagctgttgggttctgatttcagttgcgaacgtcaccggagaccgtccacgccgttgggaaagaacgccgaagtgcctcccgcgacccgcacgtcttctacatacagcgtcctcagcgcttttgtagtgtggatcggatccggcctcaatatcatctggtggaccggcatcgtgcttctggcggtggacgctctcggacttggcgagcgttggctgaggttagcactgtcccaccgggacaaacatcacgcatcgcgaaccgcggcgctccagtgtcaacgcgacatgttacttcggcaacgtcgacgggctcggcggctgcatgccgtttctgaaggcaaactgcaggaagagaagaaacgacagtctgctctggtctggaacgttgaggcgcgaccctttccgtccacacatcagctgattgtgctgccccctcctgtagcgtcagctcctcctgcagttccctcgcagccccccgagtattcgtctgtgtttccgcctgtataaaaataaagagacgggaggctgatcgcggccttcagcgtctcatttgtctttactctcgagtgcggtcggtgtctcgtcggtgagacgaggccgccgcccgacaagttcgatctcatgtcgctcttggagcgcgaagagagttggcgtcgcgtagtcgactactcgcacaacctgtggtgtacgtgcggtaactggcagagccacgttgagattcaggacgaagagcccaactgcgagcagccggagcccgcacactggctggaatacgtggcggtccagtggcaggcccgggttcgcgattctcacgatcgctggtgtctctgcaacgcctggcgtgatcacgctttgcgcggccgttggggtacggcgtattcctcgggttcctcggcctcttcctccggtttcgtcgcggagagcaagttcacctggtggaaacgactgcgccacagtacccggcgctggttgtttcgccgccggcgagctcgatacactccatctaactgtggggaaagtagcactagcagcggccagagtagcggtgacgagagtaactgcagtctacgcacccacggcgtgtacacacggggtgaacaacactaatcgataagtcgcgtgtaggcgactggctacatcaaccggatatctgcggggatttaaaaagacgacccgttgtcatccggcttagagcaaaccgtccttttatcatcttccgtcgccatggctatgtacacatccgaatccgaacgcgactggcgtcgtgtaatccacgactcgcacggcctgtggtgcgactgcggcgactggcgagagcacctctattgtgtgtacgacagccattttcagcgacgacccacgacccgagccgaacggagggccgccaattggcggcgacagatgcggcggttacaccgtctgtggtgtttttgtcaggactggaagtgtcacgcgttatacgccgagtgggacggcaaagaatccgacgacgagtcgtcggcgtcttcctcgggcgaagcgccagagcaacaggtccccgcttggaagaccgtgcgggccttctcgcgggcctaccaccaccgcattaaccggggtctgcggggcacgcccccaccgcgcaacttgccgggatacgagcacgcctccgagggctggcggttttgcagtcgacgggaacggcgagaggacgatcttcgcacgcgggctgagccggaccgcgtggtgttccagttagggggagtacctcctcgtcgtcaccgagaaacttacgtgtaagaacacggcgtgacaataaacaacatagcgtaaatccccgtgtgatgtgtgtgattgacgttcgggaaacatgtccccatcatcagcgtcacaactgacgtgggttggtcactgacgtgcaggatgttgcgcgagtcagagaatcgcataagaacggggtggtgagcgggttcccacaggagtctctggcgcaaaagcaccatgagcctcaggttccccgagagggcgggttacgagaaactgggataccgcccgcatgccaaacgcgtgcgggtgcatgacccgttgggattgacgcggtttatcatgaggcaactcatgatgtacccgctggtgttgccgttcacctttccgttttacgtgccgcggtcctagcacgtcagtggtgatgctgataattgcaacatggcccatgacgaacccgcttgggacgaacgtcaataccacgtcaaaccaccgtgacttggctgaacgttgaaacataaagccaaagcgccgtcggcacttggcttcagagcagcgcctcggggcgatgcgacggcgatgaacttagagcaactcatcaacgtccttggtctgctcgtctggattgccgctcgtgctgtcagccgcgttggtccgcatggctccggactcgtttatcgtgagcttcatgatttctacgggtatctgcagctggaccttctgggaccagtggtggcggggaatcgctcagtccggacctggaaagagcaggcggaccgagccagagggaccttcgttcggcgttcaggccttaatactagctacatcttacctgtcggcggcctgtctgggggctccggtaccttacccgtcggcctgtatcgtcccgaagaagaggtgttcctcctcttgaaccgctgccatgggccactgtcaacgccgaaaaatgcttgtctggctgaggtcggtgtcgctaatgccacttttttgtctcgcttcaatgtcggtgattttcacggagcgtcatgggaaaacggtaccgctcccgatggagagcccggggtatgctgaaattcctcttaagattccgtaaacgacgttgtccagtcgttgtgccgcgattcgtacggttcatcgtctacgtcgttttgttcaccgtcgctgtgcaacgcgtgaaacaagagcgtgatgcgcaccttcggcggtatgaagaacggttacggaaaaaccgcgcacggcgtcggcagtcttttccgtgacttggggcgatgggtccgagctgcggtatgggtcacggcggcgtgtgttttattgacgaagatgccgatgtgtgactaaaaacgtcccagccctagagcgatgtgtttcaataaaaattatgtcgtatcatagtatgcgtgtcctggtttttcatttttggatgtatttgtgacataaaaggcgatagaatgtggggacgaaacatatccagatacacagttttgttattcgaacaaaacccgtgtgatgcagaaaacagtactgcaggatgaaagtcccatgggggggggggggcagacagtagtcgtttttgccgctgggcgtacgctatgcttgtatttatgactataatatgtgcactcgtgtgtcgatgttcctattgggaagggtgtcaatgtaggaggtataaagaatggtgggatgcggagaggcatcgctagacacaggttgatcgctgtgctagccccacctgatcagcgtcatgggtaaagcggtgattaagcgtgaaaacaccgtaagggggggggggcagacaggaagcttggtggcagtggccgttagatgcattacgtgtctgtattggtacatttgcaaaccgtcgggtgtggcggtatagtttagcgatgattatattatgtatgtgccgtatagaatggcctaaaacattgtaacacgaaacgttacaatgatgggaaagatgccgataaaaaacacataaaaggcatatacacgaattactagttacacgtttgtctatgtgcgagtttaaggacgcttgtataatgcgtatgacggcaaacggccgcggaaacgatggggggggggggtagtaactgtattaattatacgtcttgcagtacacggtattgtgtgctggtgcgcgtattacgacacgaacggcatagcgctataaccgggtgtatggtatttatatgtgcgtctagcatccttgcgagattctgaaagtcttcttgtaagcgtaattaaaacggtgtatgttctgcgtaaagtgcattcaaacaacgtaacagtatgggatgaatgccaataaataacatataaaagcgagaagtatacatataagggttgctagacacaggtttgtttctgtgctagcccaatggcacttgtacaatccatgcaagcaaaaaaaggatgcgaaaccaacatcgtggggtggggggggggtaaaagcaatgttaatcattggtctcgcggtgcaagttgctgcgttttacgtgtattgttacacgggttgcgtatcggtataatcggatgtgtgttactcattcgtggcgttgttatagtattgtgaaaaagaattctcgtaagcatgttgacaactgcaaaataaaaccattttattgagcattgtaatggtagtgtgtcgctacattagaaaacgtgacgcgtcgcatgtcgcggcacaatctggcagcggggtcggggtagggtacggtgggaggcatgtacacagatggaacaaaagcagaagtaacgtgagacggagcatatagtccagtatccagcggttcctgagtagcaccacccatcaactgaatgccctcatgagtaaaagtctgcgggcggcagcccttggggaccgttggcatgggacgatcgatctccaaaccacagcgtaacacggttttcttccaacgtcgttgatacacgtcgtttttacggttactccccagaacccagaaagtctcgtccaagtcgtaccaggagtcttccccagggagacgtggcggtttccaatcctcatcgtcccgtcgcaaagcacgtcccaaactggcttggggagtcaacggtggttctgtgggtcgggtgtagcgcgagtgttttccgttcatgagcgattcgtcctccttgcctttaggctttttggcctttttgtgtatcatctggccgccggcctccataaccaccgtggccaagtccagtcccagagcttgagcgtcggcgcggcgtcgggcgtcttgcaggtagtcttccacatttgcacagatggccgggtgtttggtggctagggtgaggacctcagcctcgccgcggcccggacgtagcaaaaaagctaactgcccgtgcggctcgcgcgcccacagcgcggcgcgcgggtgcaggtgcagcgcgtcccagcgcggccgctcccactgctcgcggtccagctcgggcagcagccgccgcgcggcctcggcggcgggcgccgactcgcgccccagcgccagcgcgcccaacacgcccgcgcgcagaaagtgcgacagctccgccgccagcgggtacacgtgcccgtccagcgggcagtacccgaacacggcgcccagctcgtccagcaccaccaccagcatggcgcgcggcacggtccccgacgccgccggacccgccatcgccgtcggacccaccatcaccgtcggcgccgccgctgctgccgctgccgcatccgttccgaccaccgcgtgcgcgtccgcgtttggcacgcaaatcgcgctcccgccggcggcgccgtacggctgcggaggtaaagtcacagcagaccccacggctcccgccatcgcgcacggcgcgtccccgccggcggcctccgtctccgtgccgctcgcccccggcagcaacgtcgtccccgtcgccatcgccgtcgtccccgccgtcatcgtcgtcgtcgtccccgccgtcgtccctgtcgccggccctgccgcgcagcgcagccaccgcgacggcagcaccgcgcccagcgccagccagccgcagcacagacgctggttcaggtgccgacgcacggccgtcagcagcgacgcggggtgcggcgccgacgcgaacggctcgtactgcgccagctcctgccacgcgcccagcagcaccatcggctgcagtcgcctgcccggcgtctgcagcgccaccgtcgtgccggcccaccgccggcgcagctcccgtccgagcgccgtcgcctcctcggcgcgcagcaacgtctggcgaagcgccggctgaggcagcagcgtcgcgcgcggggtgcccacgcccagccggttgcagcggtacaggcgcaccacctcgcccgcgccgtgccgaaaccactcgtccgcgtcgcgcgccgccaggatcagcgtgttgttcgccaggtcgtacacgaacacgcggaacccggcgcccagcgccaggtacagtccgtcctgcgcgcacagaccctcgggatggccggccttgtcgcccaccgtcgggtcggccgcggggtccacctcgtgcaccacggtcgccaccagcacgatccacgcgtcccgcggcgacagctgacgcaggtccgtggcgcccacgccgttcatctggctgcgcggcgtcactcgcgcgtagaatccgtacggccgtccgagcggcagcagcgtgcccgcgtcgcgctgcgaccacttgcgcatggcgcggcccgtgctgttggccaaaaacgcggcgcgccacacggcgcccatggcctggtattccagctccgtcagcgcctggcgctccaccggaatctgagacagcagcaagcgctccgggccgtgccaaaaggtgctgttgttgccgctacccggaggggcgcccggcggcccgcggggttctacccggtggacggcgtgggccggcgtcgccgtacccgcagtactcgtactagtccccgctgttgacgtcgcttccaaagaagaagaacgagaggaaccaacccccgaaggccctccggctccgcggccgcgaccgaggggcggggggcgcggcgacatgccgttgcgctgggccatggccgccggacgcctccgacgtccactctgtatatataggaagcaaacccgcgtcagcgaccacgccgtttacacacgcggacgcctccgtcgcccgtgtgccgcgggcgacacgcacctggcttttataggcagcgacgtgcacggcgcttgctggcgccgccttgccgccgcgcagtctggaaggccgtgaaaaaaccgaaagaagatgcgcgacaagccaccaacaacgggccgccgagcgcgcgcacacctaggtggacgcctgacctccattccgggccgtgtgctgggtccccgaggggcgggggggtgttttcatcgggggggtgaaatgtgggaatttgggaagttggcggtggcgggggacggcgacggcgaataaaagcgccgtgcggcgcgcacggcgaaacccagacgcgcgtgtgtcttgcgtctctttcagtcgcgcgtctgtcttgcgtgtctttgagtccccggggaaaagaggaagcggtcccgaggggacggcggcgcgactccctggggacgcgaagatcggacgcggaaaagaggaagtccccggggacggccacaggcggaaaaaaaaaacgaggaagccgcagcccagtctgccgggaccggcaggcaggcgcacagacccgcgtcgaggacacacgcagaagaagcgcccgcgccggggcggggggggggatcgcgggccccggggcacactgcttccatctggccgcgcgcacaccccgccgacacacccctgacacacccgcgacacacccggcacacgcccgcgacacacccggcacgcgcccgccacacagccagccgacacacccgcgacacacccgccacacccagccgcacccggcacacacccacccagccgcacccccgccacacccagaccgacgccggtgcgggaccgggctccattccgggccgtgtgctgggtccccgaggggcgggggggtgttttcatcgggggggtgaaatgtgggaatttgggaagttggcggtggcgggggacggcgacggcgaataaaagcgccgtgcggcgcgcacggcgaaacccagacgcgcgtgtgtcttgcgtctctttcagtcgcgcgtctgtcttgcgtgtctttgagtccccggggaaaagaggaagcggtcccgaggggacggcggcgcgactccctggggacgcgaagatcggacgcggaaaagaggaagtccccggggacggccacaggcggaaaaaaaaaacgaggaagccgcagcccagtctgccgggaccggcaggcaggcgcacagacccgcgtcgaggacacacgcagaagaagcgcccgcgccggggcggggggggggatcgcgggccccggggcacactgcttccatctggccgcgcgcacaccccgccgacacacccctgacacacccgcgacacacccggcacacgcccgcgacacacccggcacgcgcccgccacacagccagccgacacacccgcgacacacccgccacacccagccgcacccggcacacacccacccagccgcacccccgccacacccagaccgacgccggtgcgggaccgggctccattccgggccgtgtgctgggtccccgaggggcgggggggtgttttcatcgggggggtgaaatgtgggaatttgggaagttggcggtggcgggggacggcgacggcgaataaaagcgccgtgcggcgcgcacggcgaaacccagacgcgcgtgtgtcttgcgtctctttcagtcgcgcgtctgtcttgcgtgtctttgagtccccggggaaaagaggaagcggtcccgaggggacggcggcgcgactccctggggacgcgaagatcggacgcggaaaagaggaagtccccggggacggccacaggcggaaaaaaaaaacgaggaagccgcagcccagtctgccgggaccggcaggcaggcgcacagacccgcgtcgaggacacacgcagaagaagcgcccgcgccggggcggggggggggatcgcgggccccggggcacactgcttccatctggccgcgcgcacaccccgccgacacacccctgacacacccgcgacacacccggcacacgcccgcgacacacccggcacgcgcccgccacacagccagccgacacacccgcgacacacccgccacacccagccgcacccggcacacacccacccagccgcacccccgccacacccagaccgacgccggtgcgggaccgggctgaggggggtgtaagcgccttgacgcgcggcgctatggcactgcgtgccacggtattggttggcgggacgaggctgaggggggtttgcgggacgtaagcgcgacgccgagtttgcggcgtgctgtggcgcgctcaaggctagggacgggggccgcgcgtagcttttcggcggcgacggggaacaaaacaggcacgcacacgcagctcgcttcagcggtcgccctatcggcaccgccgctattctttattaacgtcgttctccccccgcttctacacgcggaccgctgcagacggctatgctcagactgtttctcttgacggcgacatgtgtttgcgtctgtgcggcgcggcgacggccgcaagcggacgacgccgcctgccaccacacgtggcccacgcgctgcgccggcccgcgtcccgcgccgtcggctcacaacacggcgctttcttcctcgcacgccatctccatcgcacaccgtgtgctgcattcgccgtcgcctccacgagagaacatccgccacagcatgcgctgtcgccgtcgcgccatggcctcctcggcttgcacacccgtttcgcacacccagcctcgggccgccaaccacagccgttcgaggatgacgtacgcgacgagcgagcccaccaattctcccacggcctcgcccgccaagtcagac

SEQ ID NO: 2 - RNA, 21 nt, synthetic construct
  misc_feature 1..21: note = siRNA
  source 1..21: mol_type = other RNA
gctacaagctggagaatgatt

SEQ ID NO: 3 - RNA, 21 nt, synthetic construct
  misc_feature 1..21: note = siRNA
  source 1..21: mol_type = other RNA
tcattctccagcttgtagctt

SEQ ID NO: 4 - protein, 498 aa, synthetic construct
  REGION 1..498: note = HIVgag
MAARASILSGGKLDAWEKIRLRPGGKKKYTLKHLVWASRELDRFALNPSLLETTEGCQQIMNQLQPAVKTGTEEIKSLFNTVATLYCVHQRIDVKDTKEALDKIEEIQNKSKQKTQQAAADTGDSSKVSQNYPIIQNAQGQMIHQNLSPRTLNAWVKVIEEKAFSPEVIPMFSALSEGATPQDLNVMLNIVGGHQAAMQMLKDTINEEAAEWDRLHPVQAGPIPPGQIREPRGSDIAGTTSTPQEQLQWMTGNPPIPVGNIYKRWIILGLNKIVRMYSPVSILDIKQGPKEPFRDYVDRFFKALRAEQATQDVKGWMTETLLVQNANPDCKSILKALGSGATLEEMMTACQGVGGPGHKARVLAEAMSQAQQTNIMMQRGNFRGQKRIKCFNCGKEGHLARNCRAPRKKGCWKCGKEGHQMKDCTERQANFLGKIWPSSKGRPGNFPQSRPEPTAPPAELFGMGEGIASLPKQEQKDREQVPPLVSLKSLFGNDPLSQ

SEQ ID NO: 5 - protein, 498 aa, synthetic construct
  REGION 1..498: note = #3D6 p4
MAARASILSGGKLDAWEKIRLRPGGKKKYRLKHLVWASRELDRFALNPSLLETTEGCQQIMNQLQPAVKTGTEEIKSLFNTVATLYCVHQRIDVKDTKEALDKIEEIQNKSKQKTQQAAADTGDSSKVSQNYPIIQNAQGQMIHQNLSPRTLNAWVKVIEEKAFSPEVIPMFSALSEGATPQDLNVMLNIVGGHQAAMQMLKDTINEEAAEWDRLHPVQAGPIPPGQIREPRGSDIAGTTSTPQEQLQWMTGNPPIPVGNIYKRWIILGLNKIVRMYSPVSILDIKQGPKEPFRDYVDRFFKALRAEQATQDVKGWMTETLLVQNANPDCKSILKALGSGATLEEMMTACQGVGGPGHKARVLAEAMSQAQQTNIMMQRGNFRGQKRIKCFNCGKEGHLARNCRAPRKKGCWKCGKEGHQMKDCTERQANFLGKIWPSSKGRPGNFPQSRPEPTAPPAELFGMGEGIASLPKQEQKDREQVPPLVSLKSLFGNDPLSQ

SEQ ID NO: 6 - protein, 498 aa, synthetic construct; identical to SEQ ID NO: 5
  REGION 1..498: note = #3D6 p5

SEQ ID NO: 7 - protein, 498 aa, synthetic construct; identical to SEQ ID NO: 5
  REGION 1..498: note = #3D6 p6